European Patent Specification EP 3 292 142 B1, published March 20, 2024. Title: ONCOLYTIC ADENOVIRUSES WITH MUTATIONS IN ALTERED IMMUNODOMINANT ADENOVIRUS EPITOPES AND THEIR USE IN CANCER TREATMENT. Applicant: VCN Biosciences ALEMANY, RAMON HOYOS, RAUL GIL BAZAN, MIRIAM. The sequence listing filed with the application follows.

SEQUENCE LISTING (38 sequences)

SEQ ID NO: 1 - DNA, 36124 bp, Artificial Sequence
  ICOVIR15K (nt1-36124)
taattaccctgttatccctacatcatcaataatataccttattttggattgaagccaatatgataatgagggggtggagtttgtgacgtggcgcggggcgtgggaacggggcgggtgacgtagtagtgtggcggaagtgtgatgttgcaagtgtggcggaacacatgtaagcgacggatgtggcaaaagtgacgtttttggtgtgcgccggtgtacacaggaagtgacaattttcgcgcggttttaggcggatgttgtagtaaatttgggcgtaaccgagtaagatttggccattttcgcgggaaaactgaataagaggaagtgaaatctgaataattttgtgttactcatagcgcgtaatatttgtctagggccgcggggactttgaccgtttacgtggagactcgcccaggtgtttttctcaggtgttttccgcgtactcggcggctcgtggctctttcgcggcaaaaaggatttggcgcgtaaaagtggttcgaagtactcggcggctcgtggctctttcgcggcaaaaaggatttggcgcgtaaaagtggttcgaagtacgtcgaccacaaaccccgcccagcgtcttgtcattggcgtcgacgctgtacggggtcaaagttggcgttttattattatagtcagctgacgtgtagtgtatttatacccggtgagttcctcaagaggccactcttgagtgccagcgagtagagttttctcctccgagccgctccgacaccgggactgaaaatgagacatattatctgccacggaggtgttattaccgaagaaatggccgccagtcttttggaccagctgatcgaagaggtactggctgataatcttccacctcctagccattttgaaccacctacccttcacgaactgtatgatttagacgtgacggcccccgaagatcccaacgaggaggcggtttcgcagatttttcccgactctgtaatgttggcggtgcaggaagggattgacttactcacttttccgccggcgcccggttctccggagccgcctcacctttcccggcagcccgagcagccggagcagagagccttgggtccggtttctatgccaaaccttgtaccggaggtgatcgatccacccagtgacgacgaggatgaagagggtgaggagtttgtgttagattatgtggagcaccccgggcacggttgcaggtcttgtcattatcaccggaggaatacgggggacccagatattatgtgttcgctttgctatatgaggacctgtggcatgtttgtctacagtaagtgaaaattatgggcagtgggtgatagagtggtgggtttggtgtggtaattttttttttaatttttacagttttgtggtttaaagaattttgtattgtgatttttttaaaaggtcctgtgtctgaacctgagcctgagcccgagccagaaccggagcctgcaagacctacccgccgtcctaaaatggcgcctgctatcctgagacgcccgacatcacctgtgtccagagaatgcaatagtagtacggatagctgtgactccggtccttctaacacacctcctgagatacacccggtggtcccgctgtgccccattaaaccagttgccgtgagagttggtgggcgtcgccaggctgtggaatgtatcgaggacttgcttaacgagcctgggcaacctttggacttgagctgtaaacgccccaggccataaggtgtaaacctgtgattgcgtgtgtggttaacgcctttgtttgctgaatgagttgatgtaagtttaataaagggtgagataatgtttaacttgcatggcgtgttaaatggggcggggcttaaagggtatataatgcgccgtgggctaatcttggttacatctgacctcatggaggcttgggagtgtttggaagatttttctgctgtgcgtaacttgctggaacagagctctaacagtacctcttggttttggaggtttctgtggggctcatcccaggcaaagttagtctgcagaattaaggaggattacaagtgggaatttgaagagcttttgaaatcctgtggtgagctgtttgattctttgaatctgggtcaccaggcgcttttccaagagaaggtcatcaagactttggatttttccacaccggggcgcgctgcggctgctgttgcttttttgagttttataaaggataaatggagcgaagaaacccatctgagcggggggtacctgctggattttctggccatgcatctgtggagagcggttgtgagacacaagaatcgcctgctactgttgtcttccgtccgcccggcgataataccgacggaggagcagcagcagcagcaggaggaagccaggcggcggcggcaggagcagagcccatggaacccgagagccggcctggaccctcgggaatgaatgttgtacaggtggctgaactgtatccagaactgagacgcattttgacaattacagaggatgggcaggggctaaagggggtaaagagggagcggggggcttgtgaggctacagaggaggctaggaatctagcttttagcttaatgaccagacaccgtcctgagtgtattacttttcaacagatcaaggataattgcgctaatgagcttgatctgctggcgcagaagtattccatagagcagctgaccacttactggctgcagccaggggatgattttgaggaggctattagggtatatgcaaaggtggcacttaggccagattgcaagtacaagatcagcaaacttgtaaatatcaggaattgttgctacatttctgggaacggggccgaggtggagatagatacggaggatagggtggcctttagatgtagcatgataaatatgtggccgggggtgcttggcatggacggggtggttattatgaatgtaaggtttactggccccaattttagcggtacggttttcctggccaataccaaccttatcctacacggtgtaagcttctatgggtttaacaatacctgtgtggaagcctggaccgatgtaagggttcggggctgtgccttttactgctgctggaagggggtggtgtgtcgccccaaaagcagggcttcaattaagaaatgcctctttgaaaggtgtaccttgggtatcctgtctgagggtaactccagggtgcgccacaatgtggcctccgactgtggttgcttcatgctagtgaaaagcgtggctgtgattaagcataacatggtatgtggcaactgcgaggacagggcctctcagatgctgacctgctcggacggcaactgtcacctgctgaagaccattcacgtagccagccactctcgcaaggcctggccagtgtttgagcataacatactgacccgctgttccttgcatttgggtaacaggaggggggtgttcctaccttaccaatgcaatttgagtcacactaagatattgcttgagcccgagagcatgtccaaggtgaacctgaacggggtgtttgacatgaccatgaagatctggaaggtgctgaggtacgatgagacccgcaccaggtgcagaccctgcgagtgtggcggtaaacatattaggaaccagcctgtgatgctggatgtgaccgaggagctgaggcccgatcacttggtgctggcctgcacccgcgctgagtttggctctagcgatgaagatacagattgaggtactgaaatgtgtgggcgtggcttaagggtgggaaagaatatataaggtgggggtcttatgtagttttgtatctgttttgcagcagccgccgccgccatgagcaccaactcgtttgatggaagcattgtgagctcatatttgacaacgcgcatgcccccatgggccggggtgcgtcagaatgtgatgggctccagcattgatggtcgccccgtcctgcccgcaaactctactaccttgacctacgagaccgtgtctggaacgccgttggagactgcagcctccgccgccgcttcagccgctgcagccaccgcccgcgggattgtgactgactttgctttcctgagcccgcttgcaagcagtgcagcttcccgttcatccgcccgcgatgacaagttgacggctcttttggcacaattggattctttgacccgggaacttaatgtcgtttctcagcagctgttggatctgcgccagcaggtttctgccctgaaggcttcctcccctcccaatgcggtttaaaacataaataaaaaaccagactctgtttggatttggatcaagcaagtgtcttgctgtctttatttaggggttttgcgcgcgcggtaggcccgggaccagcggtctcggtcgttgagggtcctgtgtattttttccaggacgtggtaaaggtgactctggatgttcagatacatgggcataagcccgtctctggggtggaggtagcaccactgcagagcttcatgctgcggggtggtgttgtagatgatccagtcgtagcaggagcgctgggcgtggtgcctaaaaatgtctttcagtagcaagctgattgccaggggcaggcccttggtgtaagtgtttacaaagcggttaagctgggatgggtgcatacgtggggatatgagatgcatcttggactgtatttttaggttggctatgttcccagccatatccctccggggattcatgttgtgcagaaccaccagcacagtgtatccggtgcacttgggaaatttgtcatgtagcttagaaggaaatgcgtggaagaacttggagacgcccttgtgacctccaagattttccatgcattcgtccataatgatggcaatgggcccacgggcggcggcctgggcgaagatatttctgggatcactaacgtcatagttgtgttccaggatgagatcgtcataggccatttttacaaagcgcgggcggagggtgccagactgcggtataatggttccatccggcccaggggcgtagttaccctcacagatttgcatttcccacgctttgagttcagatggggggatcatgtctacctgcggggcgatgaagaaaacggtttccggggtaggggagatcagctgggaagaaagcaggttcctgagcagctgcgacttaccgcagccggtgggcccgtaaatcacacctattaccggctgcaactggtagttaagagagctgcagctgccgtcatccctgagcaggggggccacttcgttaagcatgtccctgactcgcatgttttccctgaccaaatccgccagaaggcgctcgccgcccagcgatagcagttcttgcaaggaagcaaagtttttcaacggtttgagaccgtccgccgtaggcatgcttttgagcgtttgaccaagcagttccaggcggtcccacagctcggtcacctgctctacggcatctcgatccagcatatctcctcgtttcgcgggttggggcggctttcgctgtacggcagtagtcggtgctcgtccagacgggccagggtcatgtctttccacgggcgcagggtcctcgtcagcgtagtctgggtcacggtgaaggggtgcgctccgggctgcgcgctggccagggtgcgcttgaggctggtcctgctggtgctgaagcgctgccggtcttcgccctgcgcgtcggccaggtagcatttgaccatggtgtcatagtccagcccctccgcggcgtggcccttggcgcgcagcttgcccttggaggaggcgccgcacgaggggcagtgcagacttttgagggcgtagagcttgggcgcgagaaataccgattccggggagtaggcatccgcgccgcaggccccgcagacggtctcgcattccacgagccaggtgagctctggccgttcggggtcaaaaaccaggtttcccccatgctttttgatgcgtttcttacctctggtttccatgagccggtgtccacgctcggtgacgaaaaggctgtccgtgtccccgtatacagacttgagaggcctgtcctcgagcggtgttccgcggtcctcctcgtatagaaactcggaccactctgagacaaaggctcgcgtccaggccagcacgaaggaggctaagtgggaggggtagcggtcgttgtccactagggggtccactcgctccagggtgtgaagacacatgtcgccctcttcggcatcaaggaaggtgattggtttgtaggtgtaggccacgtgaccgggtgttcctgaaggggggctataaaagggggtgggggcgcgttcgtcctcactctcttccgcatcgctgtctgcgagggccagctgttggggtgagtactccctctgaaaagcgggcatgacttctgcgctaagattgtcagtttccaaaaacgaggaggatttgatattcacctggcccgcggtgatgcctttgagggtggccgcatccatctggtcagaaaagacaatctttttgttgtcaagcttggtggcaaacgacccgtagagggcgttggacagcaacttggcgatggagcgcagggtttggtttttgtcgcgatcggcgcgctccttggccgcgatgtttagctgcacgtattcgcgcgcaacgcaccgccattcgggaaagacggtggtgcgctcgtcgggcaccaggtgcacgcgccaaccgcggttgtgcagggtgacaaggtcaacgctggtggctacctctccgcgtaggcgctcgttggtccagcagaggcggccgcccttgcgcgagcagaatggcggtagggggtctagctgcgtctcgtccggggggtctgcgtccacggtaaagaccccgggcagcaggcgcgcgtcgaagtagtctatcttgcatccttgcaagtctagcgcctgctgccatgcgcgggcggcaagcgcgcgctcgtatgggttgagtgggggaccccatggcatggggtgggtgagcgcggaggcgtacatgccgcaaatgtcgtaaacgtagaggggctctctgagtattccaagatatgtagggtagcatcttccaccgcggatgctggcgcgcacgtaatcgtatagttcgtgcgagggagcgaggaggtcgggaccgaggttgctacgggcgggctgctctgctcggaagactatctgcctgaagatggcatgtgagttggatgatatggttggacgctggaagacgttgaagctggcgtctgtgagacctaccgcgtcacgcacgaaggaggcgtaggagtcgcgcagcttgttgaccagctcggcggtgacctgcacgtctagggcgcagtagtccagggtttccttgatgatgtcatacttatcctgtcccttttttttccacagctcgcggttgaggacaaactcttcgcggtctttccagtactcttggatcggaaacccgtcggcctccgaacggtaagagcctagcatgtagaactggttgacggcctggtaggcgcagcatcccttttctacgggtagcgcgtatgcctgcgcggccttccggagcgaggtgtgggtgagcgcaaaggtgtccctgaccatgactttgaggtactggtatttgaagtcagtgtcgtcgcatccgccctgctcccagagcaaaaagtccgtgcgctttttggaacgcggatttggcagggcgaaggtgacatcgttgaagagtatctttcccgcgcgaggcataaagttgcgtgtgatgcggaagggtcccggcacctcggaacggttgttaattacctgggcggcgagcacgatctcgtcaaagccgttgatgttgtggcccacaatgtaaagttccaagaagcgcgggatgcccttgatggaaggcaattttttaagttcctcgtaggtgagctcttcaggggagctgagcccgtgctctgaaagggcccagtctgcaagatgagggttggaagcgacgaatgagctccacaggtcacgggccattagcatttgcaggtggtcgcgaaaggtcctaaactggcgacctatggccattttttctggggtgatgcagtagaaggtaagcgggtcttgttcccagcggtcccatccaaggttcgcggctaggtctcgcgcggcagtcactagaggctcatctccgccgaacttcatgaccagcatgaagggcacgagctgcttcccaaaggcccccatccaagtataggtctctacatcgtaggtgacaaagagacgctcggtgcgaggatgcgagccgatcgggaagaactggatctcccgccaccaattggaggagtggctattgatgtggtgaaagtagaagtccctgcgacgggccgaacactcgtgctggcttttgtaaaaacgtgcgcagtactggcagcggtgcacgggctgtacatcctgcacgaggttgacctgacgaccgcgcacaaggaagcagagtgggaatttgagcccctcgcctggcgggtttggctggtggtcttctacttcggctgcttgtccttgaccgtctggctgctcgaggggagttacggtggatcggaccaccacgccgcgcgagcccaaagtccagatgtccgcgcgcggcggtcggagcttgatgacaacatcgcgcagatgggagctgtccatggtctggagctcccgcggcgtcaggtcaggcgggagctcctgcaggtttacctcgcatagacgggtcagggcgcgggctagatccaggtgatacctaatttccaggggctggttggtggcggcgtcgatggcttgcaagaggccgcatccccgcggcgcgactacggtaccgcgcggcgggcggtgggccgcgggggtgtccttggatgatgcatctaaaagcggtgacgcgggcgagcccccggaggtagggggggctccggacccgccgggagagggggcaggggcacgtcggcgccgcgcgcgggcaggagctggtgctgcgcgcgtaggttgctggcgaacgcgacgacgcggcggttgatctcctgaatctggcgcctctgcgtgaagacgacgggcccggtgagcttgaacctgaaagagagttcgacagaatcaatttcggtgtcgttgacggcggcctggcgcaaaatctcctgcacgtctcctgagttgtcttgataggcgatctcggccatgaactgctcgatctcttcctcctggagatctccgcgtccggctcgctccacggtggcggcgaggtcgttggaaatgcgggccatgagctgcgagaaggcgttgaggcctccctcgttccagacgcggctgtagaccacgcccccttcggcatcgcgggcgcgcatgaccacctgcgcgagattgagctccacgtgccgggcgaagacggcgtagtttcgcaggcgctgaaagaggtagttgagggtggtggcggtgtgttctgccacgaagaagtacataacccagcgtcgcaacgtggattcgttgatatcccccaaggcctcaaggcgctccatggcctcgtagaagtccacggcgaagttgaaaaactgggagttgcgcgccgacacggttaactcctcctccagaagacggatgagctcggcgacagtgtcgcgcacctcgcgctcaaaggctacaggggcctcttcttcttcttcaatctcctcttccataagggcctccccttcttcttcttctggcggcggtgggggaggggggacacggcggcgacgacggcgcaccgggaggcggtcgacaaagcgctcgatcatctccccgcggcgacggcgcatggtctcggtgacggcgcggccgttctcgcgggggcgcagttggaagacgccgcccgtcatgtcccggttatgggttggcggggggctgccatgcggcagggatacggcgctaacgatgcatctcaacaattgttgtgtaggtactccgccgccgagggacctgagcgagtccgcatcgaccggatcggaaaacctctcgagaaaggcgtctaaccagtcacagtcgcaaggtaggctgagcaccgtggcgggcggcagcgggcggcggtcggggttgtttctggcggaggtgctgctgatgatgtaattaaagtaggcggtcttgagacggcggatggtcgacagaagcaccatgtccttgggtccggcctgctgaatgcgcaggcggtcggccatgccccaggcttcgttttgacatcggcgcaggtctttgtagtagtcttgcatgagcctttctaccggcacttcttcttctccttcctcttgtcctgcatctcttgcatctatcgctgcggcggcggcggagtttggccgtaggtggcgccctcttcctcccatgcgtgtgaccccgaagcccctcatcggctgaagcagggctaggtcggcgacaacgcgctcggctaatatggcctgctgcacctgcgtgagggtagactggaagtcatccatgtccacaaagcggtggtatgcgcccgtgttgatggtgtaagtgcagttggccataacggaccagttaacggtctggtgacccggctgcgagagctcggtgtacctgagacgcgagtaagccctcgagtcaaatacgtagtcgttgcaagtccgcaccaggtactggtatcccaccaaaaagtgcggcggcggctggcggtagaggggccagcgtagggtggccggggctccgggggcgagatcttccaacataaggcgatgatatccgtagatgtacctggacatccaggtgatgccggcggcggtggtggaggcgcgcggaaagtcgcggacgcggttccagatgttgcgcagcggcaaaaagtgctccatggtcgggacgctctggccggtcaggcgcgcgcaatcgttgacgctctagaccgtgcaaaaggagagcctgtaagcgggcactcttccgtggtctggtggataaattcgcaagggtatcatggcggacgaccggggttcgagccccgtatccggccgtccgccgtgatccatgcggttaccgcccgcgtgtcgaacccaggtgtgcgacgtcagacaacgggggagtgctccttttggcttccttccaggcgcggcggctgctgcgctagcttttttggccactggccgcgcgcagcgtaagcggttaggctggaaagcgaaagcattaagtggctcgctccctgtagccggagggttattttccaagggttgagtcgcgggacccccggttcgagtctcggaccggccggactgcggcgaacgggggtttgcctccccgtcatgcaagaccccgcttgcaaattcctccggaaacagggacgagccccttttttgcttttcccagatgcatccggtgctgcggcagatgcgcccccctcctcagcagcggcaagagcaagagcagcggcagacatgcagggcaccctcccctcctcctaccgcgtcaggaggggcgacatccgcggttgacgcggcagcagatggtgattacgaacccccgcggcgccgggcccggcactacctggacttggaggagggcgagggcctggcgcggctaggagcgccctctcctgagcggcacccaagggtgcagctgaagcgtgatacgcgtgaggcgtacgtgccgcggcagaacctgtttcgcgaccgcgagggagaggagcccgaggagatgcgggatcgaaagttccacgcagggcgcgagctgcggcatggcctgaatcgcgagcggttgctgcgcgaggaggactttgagcccgacgcgcgaaccgggattagtcccgcgcgcgcacacgtggcggccgccgacctggtaaccgcatacgagcagacggtgaaccaggagattaactttcaaaaaagctttaacaaccacgtgcgtacgcttgtggcgcgcgaggaggtggctataggactgatgcatctgtgggactttgtaagcgcgctggagcaaaacccaaatagcaagccgctcatggcgcagctgttccttatagtgcagcacagcagggacaacgaggcattcagggatgcgctgctaaacatagtagagcccgagggccgctggctgctcgatttgataaacatcctgcagagcatagtggtgcaggagcgcagcttgagcctggctgacaaggtggccgccatcaactattccatgcttagcctgggcaagttttacgcccgcaagatataccataccccttacgttcccatagacaaggaggtaaagatcgaggggttctacatgcgcatggcgctgaaggtgcttaccttgagcgacgacctgggcgtttatcgcaacgagcgcatccacaaggccgtgagcgtgagccggcggcgcgagctcagcgaccgcgagctgatgcacagcctgcaaagggccctggctggcacgggcagcggcgatagagaggccgagtcctactttgacgcgggcgctgacctgcgctgggccccaagccgacgcgccctggaggcagctggggccggacctgggctggcggtggcacccgcgcgcgctggcaacgtcggcggcgtggaggaatatgacgaggacgatgagtacgagccagaggacggcgagtactaagcggtgatgtttctgatcagatgatgcaagacgcaacggacccggcggtgcgggcggcgctgcagagccagccgtccggccttaactccacggacgactggcgccaggtcatggaccgcatcatgtcgctgactgcgcgcaatcctgacgcgttccggcagcagccgcaggccaaccggctctccgcaattctggaagcggtggtcccggcgcgcgcaaaccccacgcacgagaaggtgctggcgatcgtaaacgcgctggccgaaaacagggccatccggcccgacgaggccggcctggtctacgacgcgctgcttcagcgcgtggctcgttacaacagcggcaacgtgcagaccaacctggaccggctggtgggggatgtgcgcgaggccgtggcgcagcgtgagcgcgcgcagcagcagggcaacctgggctccatggttgcactaaacgccttcctgagtacacagcccgccaacgtgccgcggggacaggaggactacaccaactttgtgagcgcactgcggctaatggtgactgagacaccgcaaagtgaggtgtaccagtctgggccagactattttttccagaccagtagacaaggcctgcagaccgtaaacctgagccaggctttcaaaaacttgcaggggctgtggggggtgcgggctcccacaggcgaccgcgcgaccgtgtctagcttgctgacgcccaactcgcgcctgttgctgctgctaatagcgcccttcacggacagtggcagcgtgtcccgggacacatacctaggtcacttgctgacactgtaccgcgaggccataggtcaggcgcatgtggacgagcatactttccaggagattacaagtgtcagccgcgcgctggggcaggaggacacgggcagcctggaggcaaccctaaactacctgctgaccaaccggcggcagaagatcccctcgttgcacagtttaaacagcgaggaggagcgcattttgcgctacgtgcagcagagcgtgagccttaacctgatgcgcgacggggtaacgcccagcgtggcgctggacatgaccgcgcgcaacatggaaccgggcatgtatgcctcaaaccggccgtttatcaaccgcctaatggactacttgcatcgcgcggccgccgtgaaccccgagtatttcaccaatgccatcttgaacccgcactggctaccgccccctggtttctacaccgggggattcgaggtgcccgagggtaacgatggattcctctgggacgacatagacgacagcgtgttttccccgcaaccgcagaccctgctagagttgcaacagcgcgagcaggcagaggcggcgctgcgaaaggaaagcttccgcaggccaagcagcttgtccgatctaggcgctgcggccccgcggtcagatgctagtagcccatttccaagcttgatagggtctcttaccagcactcgcaccacccgcccgcgcctgctgggcgaggaggagtacctaaacaactcgctgctgcagccgcagcgcgaaaaaaacctgcctccggcatttcccaacaacgggatagagagcctagtggacaagatgagtagatggaagacgtacgcgcaggagcacagggacgtgccaggcccgcgcccgcccacccgtcgtcaaaggcacgaccgtcagcggggtctggtgtgggaggacgatgactcggcagacgacagcagcgtcctggatttgggagggagtggcaacccgtttgcgcaccttcgccccaggctggggagaatgttttaaaaaaaaaaaaagcatgatgcaaaataaaaaactcaccaaggccatggcaccgagcgttggttttcttgtattccccttagtatgcggcgcgcggcgatgtatgaggaaggtcctcctccctcctacgagagtgtggtgagcgcggcgccagtggcggcggcgctgggttctcccttcgatgctcccctggacccgccgtttgtgcctccgcggtacctgcggcctaccggggggagaaacagcatccgttactctgagttggcacccctattcgacaccacccgtgtgtacctggtggacaacaagtcaacggatgtggcatccctgaactaccagaacgaccacagcaactttctgaccacggtcattcaaaacaatgactacagcccgggggaggcaagcacacagaccatcaatcttgacgaccggtcgcactggggcggcgacctgaaaaccatcctgcataccaacatgccaaatgtgaacgagttcatgtttaccaataagtttaaggcgcgggtgatggtgtcgcgcttgcctactaaggacaatcaggtggagctgaaatacgagtgggtggagttcacgctgcccgagggcaactactccgagaccatgaccatagaccttatgaacaacgcgatcgtggagcactacttgaaagtgggcagacagaacggggttctggaaagcgacatcggggtaaagtttgacacccgcaacttcagactggggtttgaccccgtcactggtcttgtcatgcctggggtatatacaaacgaagccttccatccagacatcattttgctgccaggatgcggggtggacttcacccacagccgcctgagcaacttgttgggcatccgcaagcggcaacccttccaggagggctttaggatcacctacgatgatctggagggtggtaacattcccgcactgttggatgtggacgcctaccaggcgagcttgaaagatgacaccgaacagggcgggggtggcgcaggcggcagcaacagcagtggcagcggcgcggaagagaactccaacgcggcagccgcggcaatgcagccggtggaggacatgaacgatcatgccattcgcggcgacacctttgccacacgggctgaggagaagcgcgctgaggccgaagcagcggccgaagctgccgcccccgctgcgcaacccgaggtcgagaagcctcagaagaaaccggtgatcaaacccctgacagaggacagcaagaaacgcagttacaacctaataagcaatgacagcaccttcacccagtaccgcagctggtaccttgcatacaactacggcgaccctcagaccggaatccgctcatggaccctgctttgcactcctgacgtaacctgcggctcggagcaggtctactggtcgttgccagacatgatgcaagaccccgtgaccttccgctccacgcgccagatcagcaactttccggtggtgggcgccgagctgttgcccgtgcactccaagagcttctacaacgaccaggccgtctactcccaactcatccgccagtttacctctctgacccacgtgttcaatcgctttcccgagaaccagattttggcgcgcccgccagcccccaccatcaccaccgtcagtgaaaacgttcctgctctcacagatcacgggacgctaccgctgcgcaacagcatcggaggagtccagcgagtgaccattactgacgccagacgccgcacctgcccctacgtttacaaggccctgggcatagtctcgccgcgcgtcctatcgagccgcactttttgagcaagcatgtccatccttatatcgcccagcaataacacaggctggggcctgcgcttcccaagcaagatgtttggcggggccaagaagcgctccgaccaacacccagtgcgcgtgcgcgggcactaccgcgcgccctggggcgcgcacaaacgcggccgcactgggcgcaccaccgtcgatgacgccatcgacgcggtggtggaggaggcgcgcaactacacgcccacgccgccaccagtgtccacagtggacgcggccattcagaccgtggtgcgcggagcccggcgctatgctaaaatgaagagacggcggaggcgcgtagcacgtcgccaccgccgccgacccggcactgccgcccaacgcgcggcggcggccctgcttaaccgcgcacgtcgcaccggccgacgggcggccatgcgggccgctcgaaggctggccgcgggtattgtcactgtgccccccaggtccaggcgacgagcggccgccgcagcagccgcggccattagtgctatgactcagggtcgcaggggcaacgtgtattgggtgcgcgactcggttagcggcctgcgcgtgcccgtgcgcacccgccccccgcgcaactagattgcaagaaaaaactacttagactcgtactgttgtatgtatccagcggcggcggcgcgcaacgaagctatgtccaagcgcaaaatcaaagaagagatgctccaggtcatcgcgccggagatctatggccccccgaagaaggaagagcaggattacaagccccgaaagctaaagcgggtcaaaaagaaaaagaaagatgatgatgatgaacttgacgacgaggtggaactgctgcacgctaccgcgcccaggcgacgggtacagtggaaaggtcgacgcgtaaaacgtgttttgcgacccggcaccaccgtagtctttacgcccggtgagcgctccacccgcacctacaagcgcgtgtatgatgaggtgtacggcgacgaggacctgcttgagcaggccaacgagcgcctcggggagtttgcctacggaaagcggcataaggacatgctggcgttgccgctggacgagggcaacccaacacctagcctaaagcccgtaacactgcagcaggtgctgcccgcgcttgcaccgtccgaagaaaagcgcggcctaaagcgcgagtctggtgacttggcacccaccgtgcagctgatggtacccaagcgccagcgactggaagatgtcttggaaaaaatgaccgtggaacctgggctggagcccgaggtccgcgtgcggccaatcaagcaggtggcgccgggactgggcgtgcagaccgtggacgttcagatacccactaccagtagcaccagtattgccaccgccacagagggcatggagacacaaacgtccccggttgcctcagcggtggcggatgccgcggtgcaggcggtcgctgcggccgcgtccaagacctctacggaggtgcaaacggacccgtggatgtttcgcgtttcagccccccggcgcccgcgccgttcgaggaagtacggcgccgccagcgcgctactgcccgaatatgccctacatccttccattgcgcctacccccggctatcgtggctacacctaccgccccagaagacgagcaactacccgacgccgaaccaccactggaacccgccgccgccgtcgccgtcgccagcccgtgctggccccgatttccgtgcgcagggtggctcgcgaaggaggcaggaccctggtgctgccaacagcgcgctaccaccccagcatcgtttaaaagccggtctttgtggttcttgcagatatggccctcacctgccgcctccgtttcccggtgccgggattccgaggaagaatgcaccgtaggaggggcatggccggccacggcctgacgggcggcatgcgtcgtgcgcaccaccggcggcggcgcgcgtcgcaccgtcgcatgcgcggcggtatcctgcccctccttattccactgatcgccgcggcgattggcgccgtgcccggaattgcatccgtggccttgcaggcgcagagacactgattaaaaacaagttgcatgtggaaaaatcaaaataaaaagtctggactctcacgctcgcttggtcctgtaactattttgtagaatggaagacatcaactttgcgtctctggccccgcgacacggctcgcgcccgttcatgggaaactggcaagatatcggcaccagcaatatgagcggtggcgccttcagctggggctcgctgtggagcggcattaaaaatttcggttccaccgttaagaactatggcagcaaggcctggaacagcagcacaggccagatgctgagggataagttgaaagagcaaaatttccaacaaaaggtggtagatggcctggcctctggcattagcggggtggtggacctggccaaccaggcagtgcaaaataagattaacagtaagcttgatccccgccctcccgtagaggagcctccaccggccgtggagacagtgtctccagaggggcgtggcgaaaagcgtccgcgccccgacagggaagaaactctggtgacgcaaatagacgagcctccctcgtacgaggaggcactaaagcaaggcctgcccaccacccgtcccatcgcgcccatggctaccggagtgctgggccagcacacacccgtaacgctggacctgcctccccccgccgacacccagcagaaacctgtgctgccaggcccgaccgccgttgttgtaacccgtcctagccgcgcgtccctgcgccgcgccgccagcggtccgcgatcgttgcggcccgtagccagtggcaactggcaaagcacactgaacagcatcgtgggtctgggggtgcaatccctgaagcgccgacgatgcttctgatagctaacgtgtcgtatgtgtgtcatgtatgcgtccatgtcgccgccagaggagctgctgagccgccgcgcgcccgctttccaagatggctaccccttcgatgatgccgcagtggtcttacatgcacatctcgggccaggacgcctcggagtacctgagccccgggctggtgcagtttgcccgcgccaccgagacgtacttcagcctgaataacaagtttagaaaccccacggtggcgcctacgcacgacgtgaccacagaccggtcccagcgtttgacgctgcggttcatccctgtggaccgtgaggatactgcgtactcgtacaaggcgcggttcaccctagctgtgggtgataaccgtgtgctggacatggcttccacgtactttgacatccgcggcgtgctggacaggggccctacttttaagccctactctggcactgcctacaacgccctggctcccaagggtgccccaaatccttgcgaatgggatgaagctgctactgctcttgaaataaacctagaagaagaggacgatgacaacgaagacgaagtagacgagcaagctgagcagcaaaaaactcacgtatttgggcaggcgccttattctggtataaatattacaaaggagggtattcaaataggtgtcgaaggtcaaacacctaaatatgccgataaaacatttcaacctgaacctcaaataggagaatctcagtggtacgaaacagaaattaatcatgcagctgggagagtcctaaaaaagactaccccaatgaaaccatgttacggttcatatgcaaaacccacaaatgaaaatggagggcaaggcattcttgtaaagcaacaaaatggaaagctagaaagtcaagtggaaatgcaatttttctcaactactgaggcagccgcaggcaatggtgataacttgactcctaaagtggtattgtacagtgaagatgtagatatagaaaccccagacactcatatttcttacatgcccactattaaggaaggtaactcacgagaactaatgggccaacaatctatgcccaacaggcctaattacattgcttttagggacaattttattggtctaatgtattacaacagcacgggtaatatgggtgttctggcgggccaagcatcgcagttgaatgctgttgtagatttgcaagacagaaacacagagctttcataccagcttttgcttgattccattggtgatagaaccaggtacttttctatgtggaatcaggctgttgacagctatgatccagatgttagaattattgaaaatcatggaactgaagatgaacttccaaattactgctttccactgggaggtgtgattaatacagagactcttaccaaggtaaaacctaaaacaggtcaggaaaatggatgggaaaaagatgctacagaattttcagataaaaatgaaataagagttggaaataattttgccatggaaatcaatctaaatgccaacctgtggagaaatttcctgtactccaacatagcgctgtatttgcccgacaagctaaagtacagtccttccaacgtaaaaatttctgataacccaaacacctacgactacatgaacaagcgagtggtggctcccgggctagtggactgctacattaaccttggagcacgctggtcccttgactatatggacaacgtcaacccatttaaccaccaccgcaatgctggcctgcgctaccgctcaatgttgctgggcaatggtcgctatgtgcccttccacatccaggtgcctcagaagttctttgccattaaaaacctccttctcctgccgggctcatacacctacgagtggaacttcaggaaggatgttaacatggttctgcagagctccctaggaaatgacctaagggttgacggagccagcattaagtttgatagcatttgcctttacgccaccttcttccccatggcccacaacaccgcctccacgcttgaggccatgcttagaaacgacaccaacgaccagtcctttaacgactatctctccgccgccaacatgctctaccctatacccgccaacgctaccaacgtgcccatatccatcccctcccgcaactgggcggctttccgcggctgggccttcacgcgccttaagactaaggaaaccccatcactgggctcgggctacgacccttattacacctactctggctctataccctacctagatggaaccttttacctcaaccacacctttaagaaggtggccattacctttgactcttctgtcagctggcctggcaatgaccgcctgcttacccccaacgagtttgaaattaagcgctcagttgacggggagggttacaacgttgcccagtgtaacatgaccaaagactggttcctggtacaaatgctagctaactataacattggctaccagggcttctatatcccagagagctacaaggaccgcatgtactccttctttagaaacttccagcccatgagccgtcaggtggtggatgatactaaatacaaggactaccaacaggtgggcatcctacaccaacacaacaactctggatttgttggctaccttgcccccaccatgcgcgaaggacaggcctaccctgctaacttcccctatccgcttataggcaagaccgcagttgacagcattacccagaaaaagtttctttgcgatcgcaccctttggcgcatcccattctccagtaactttatgtccatgggcgcactcacagacctgggccaaaaccttctctacgccaactccgcccacgcgctagacatgacttttgaggtggatcccatggacgagcccacccttctttatgttttgtttgaagtctttgacgtggtccgtgtgcaccagccgcaccgcggcgtcatcgaaaccgtgtacctgcgcacgcccttctcggccggcaacgccacaacataaagaagcaagcaacatcaacaacagctgccgccatgggctccagtgagcaggaactgaaagccattgtcaaagatcttggttgtgggccatattttttgggcacctatgacaagcgctttccaggctttgtttctccacacaagctcgcctgcgccatagtcaatacggccggtcgcgagactgggggcgtacactggatggcctttgcctggaacccgcactcaaaaacatgctacctctttgagccctttggcttttctgaccagcgactcaagcaggtttaccagtttgagtacgagtcactcctgcgccgtagcgccattgcttcttcccccgaccgctgtataacgctggaaaagtccacccaaagcgtacaggggcccaactcggccgcctgtggactattctgctgcatgtttctccacgcctttgccaactggccccaaactcccatggatcacaaccccaccatgaaccttattaccggggtacccaactccatgctcaacagtccccaggtacagcccaccctgcgtcgcaaccaggaacagctctacagcttcctggagcgccactcgccctacttccgcagccacagtgcgcagattaggagcgccacttctttttgtcacttgaaaaacatgtaaaaataatgtactagagacactttcaataaaggcaaatgcttttatttgtacactctcgggtgattatttacccccacccttgccgtctgcgccgtttaaaaatcaaaggggttctgccgcgcatcgctatgcgccactggcagggacacgttgcgatactggtgtttagtgctccacttaaactcaggcacaaccatccgcggcagctcggtgaagttttcactccacaggctgcgcaccatcaccaacgcgtttagcaggtcgggcgccgatatcttgaagtcgcagttggggcctccgccctgcgcgcgcgagttgcgatacacagggttgcagcactggaacactatcagcgccgggtggtgcacgctggccagcacgctcttgtcggagatcagatccgcgtccaggtcctccgcgttgctcagggcgaacggagtcaactttggtagctgccttcccaaaaagggcgcgtgcccaggctttgagttgcactcgcaccgtagtggcatcaaaaggtgaccgtgcccggtctgggcgttaggatacagcgcctgcataaaagccttgatctgcttaaaagccacctgagcctttgcgccttcagagaagaacatgccgcaagacttgccggaaaactgattggccggacaggccgcgtcgtgcacgcagcaccttgcgtcggtgttggagatctgcaccacatttcggccccaccggttcttcacgatcttggccttgctagactgctccttcagcgcgcgctgcccgttttcgctcgtcacatccatttcaatcacgtgctccttatttatcataatgcttccgtgtagacacttaagctcgccttcgatctcagcgcagcggtgcagccacaacgcgcagcccgtgggctcgtgatgcttgtaggtcacctctgcaaacgactgcaggtacgcctgcaggaatcgccccatcatcgtcacaaaggtcttgttgctggtgaaggtcagctgcaacccgcggtgctcctcgttcagccaggtcttgcatacggccgccagagcttccacttggtcaggcagtagtttgaagttcgcctttagatcgttatccacgtggtacttgtccatcagcgcgcgcgcagcctccatgcccttctcccacgcagacacgatcggcacactcagcgggttcatcaccgtaatttcactttccgcttcgctgggctcttcctcttcctcttgcgtccgcataccacgcgccactgggtcgtcttcattcagccgccgcactgtgcgcttacctcctttgccatgcttgattagcaccggtgggttgctgaaacccaccatttgtagcgccacatcttctctttcttcctcgctgtccacgattacctctggtgatggcgggcgctcgggcttgggagaagggcgcttctttttcttcttgggcgcaatggccaaatccgccgccgaggtcgatggccgcgggctgggtgtgcgcggcaccagcgcgtcttgtgatgagtcttcctcgtcctcggactcgatacgccgcctcatccgcttttttgggggcgcccggggaggcggcggcgacggggacggggacgacacgtcctccatggttgggggacgtcgcgccgcaccgcgtccgcgctcgggggtggtttcgcgctgctcctcttcccgactggccatttccttctcctataggcagaaaaagatcatggagtcagtcgagaagaaggacagcctaaccgccccctctgagttcgccaccaccgcctccaccgatgccgccaacgcgcctaccaccttccccgtcgaggcacccccgcttgaggaggaggaagtgattatcgagcaggacccaggttttgtaagcgaagacgacgaggaccgctcagtaccaacagaggataaaaagcaagaccaggacaacgcagaggcaaacgaggaacaagtcgggcggggggacgaaaggcatggcgactacctagatgtgggagacgacgtgctgttgaagcatctgcagcgccagtgcgccattatctgcgacgcgttgcaagagcgcagcgatgtgcccctcgccatagcggatgtcagccttgcctacgaacgccacctattctcaccgcgcgtaccccccaaacgccaagaaaacggcacatgcgagcccaacccgcgcctcaacttctaccccgtatttgccgtgccagaggtgcttgccacctatcacatctttttccaaaactgcaagatacccctatcctgccgtgccaaccgcagccgagcggacaagcagctggccttgcggcagggcgctgtcatacctgatatcgcctcgctcaacgaagtgccaaaaatctttgagggtcttggacgcgacgagaagcgcgcggcaaacgctctgcaacaggaaaacagcgaaaatgaaagtcactctggagtgttggtggaactcgagggtgacaacgcgcgcctagccgtactaaaacgcagcatcgaggtcacccactttgcctacccggcacttaacctaccccccaaggtcatgagcacagtcatgagtgagctgatcgtgcgccgtgcgcagcccctggagagggatgcaaatttgcaagaacaaacagaggagggcctacccgcagttggcgacgagcagctagcgcgctggcttcaaacgcgcgagcctgccgacttggaggagcgacgcaaactaatgatggccgcagtgctcgttaccgtggagcttgagtgcatgcagcggttctttgctgacccggagatgcagcgcaagctagaggaaacattgcactacacctttcgacagggctacgtacgccaggcctgcaagatctccaacgtggagctctgcaacctggtctcctaccttggaattttgcacgaaaaccgccttgggcaaaacgtgcttcattccacgctcaagggcgaggcgcgccgcgactacgtccgcgactgcgtttacttatttctatgctacacctggcagacggccatgggcgtttggcagcagtgcttggaggagtgcaacctcaaggagctgcagaaactgctaaagcaaaacttgaaggacctatggacggccttcaacgagcgctccgtggccgcgcacctggcggacatcattttccccgaacgcctgcttaaaaccctgcaacagggtctgccagacttcaccagtcaaagcatgttgcagaactttaggaactttatcctagagcgctcaggaatcttgcccgccacctgctgtgcacttcctagcgactttgtgcccattaagtaccgcgaatgccctccgccgctttggggccactgctaccttctgcagctagccaactaccttgcctaccactctgacataatggaagacgtgagcggtgacggtctactggagtgtcactgtcgctgcaacctatgcaccccgcaccgctccctggtttgcaattcgcagctgcttaacgaaagtcaaattatcggtacctttgagctgcagggtccctcgcctgacgaaaagtccgcggctccggggttgaaactcactccggggctgtggacgtcggcttaccttcgcaaatttgtacctgaggactaccacgcccacgagattaggttctacgaagaccaatcccgcccgcctaatgcggagcttaccgcctgcgtcattacccagggccacattcttggccaattgcaagccatcaacaaagcccgccaagagtttctgctacgaaagggacggggggtttacttggacccccagtccggcgaggagctcaacccaatccccccgccgccgcagccctatcagcagcagccgcgggcccttgcttcccaggatggcacccaaaaagaagctgcagctgccgccgccacccacggacgaggaggaatactgggacagtcaggcagaggaggttttggacgaggaggaggaggacatgatggaagactgggagagcctagacgaggaagcttccgaggtcgaagaggtgtcagacgaaacaccgtcaccctcggtcgcattcccctcgccggcgccccagaaatcggcaaccggttccagcatggctacaacctccgctcctcaggcgccgccggcactgcccgttcgccgacccaaccgtagatgggacaccactggaaccagggccggtaagtccaagcagccgccgccgttagcccaagagcaacaacagcgccaaggctaccgctcatggcgcgggcacaagaacgccatagttgcttgcttgcaagactgtgggggcaacatctccttcgcccgccgctttcttctctaccatcacggcgtggccttcccccgtaacatcctgcattactaccgtcatctctacagcccatactgcaccggcggcagcggcagcaacagcagcggccacacagaagcaaaggcgaccggatagcaagactctgacaaagcccaagaaatccacagcggcggcagcagcaggaggaggagcgctgcgtctggcgcccaacgaacccgtatcgacccgcgagcttagaaacaggatttttcccactctgtatgctatatttcaacagagcaggggccaagaacaagagctgaaaataaaaaacaggtctctgcgatccctcacccgcagctgcctgtatcacaaaagcgaagatcagcttcggcgcacgctggaagacgcggaggctctcttcagtaaatactgcgcgctgactcttaaggactagtttcgcgccctttctcaaatttaagcgcgaaaactacgtcatctccagcggccacacccggcgccagcacctgttgtcagcgccattatgagcaaggaaattcccacgccctacatgtggagttaccagccacaaatgggacttgcggctggagctgcccaagactactcaacccgaataaactacatgagcgcgggaccccacatgatatcccgggtcaacggaatacgcgcccaccgaaaccgaattctcctggaacaggcggctattaccaccacacctcgtaataaccttaatccccgtagttggcccgctgccctggtgtaccaggaaagtcccgctcccaccactgtggtacttcccagagacgcccaggccgaagttcagatgactaactcaggggcgcagcttgcgggcggctttcgtcacagggtgcggtcgcccgggcagggtataactcacctgacaatcagagggcgaggtattcagctcaacgacgagtcggtgagctcctcgcttggtctccgtccggacgggacatttcagatcggcggcgccggccgctcttcattcacgcctcgtcaggcaatcctaactctgcagacctcgtcctctgagccgcgctctggaggcattggaactctgcaatttattgaggagtttgtgccatcggtctactttaaccccttctcgggacctcccggccactatccggatcaatttattcctaactttgacgcggtaaaggactcggcggacggctacgactgaatgttaagtggagaggcagagcaactgcgcctgaaacacctggtccactgtcgccgccacaagtgctttgcccgcgactccggtgagttttgctactttgaattgcccgaggatcatatcgagggcccggcgcacggcgtccggcttaccgcccagggagagcttgcccgtagcctgattcgggagtttacccagcgccccctgctagttgagcgggacaggggaccctgtgttctcactgtgatttgcaactgtcctaaccttggattacatcaagatctttgttgccatctctgtgctgagtataataaatacagaaattaaaatatactggggctcctatcgccatcctgtaaacgccaccgtcttcacccgcccaagcaaaccaaggcgaaccttacctggtacttttaacatctctccctctgtgatttacaacagtttcaacccagacggagtgagtctacgagagaacctctccgagctcagctactccatcagaaaaaacaccaccctccttacctgccgggaacgtacgagtgcgtcaccggccgctgcaccacacctaccgcctgaccgtaaaccagactttttccggacagacctcaataactctgtttaccagaacaggaggtgagcttagaaaacccttagggtattaggccaaaggcgcagctactgtggggtttatgaacaattcaagcaactctacgggctattctaattcaggtttctctagaatcggggttggggttattctctgtcttgtgattctctttattcttatactaacgcttctctgcctaaggctcgccgcctgctgtgtgcacatttgcatttattgtcagctttttaaacgctggggtcgccacccaagatgattaggtacataatcctaggtttactcacccttgcgtcagcccacggtaccacccaaaaggtggattttaaggagccagcctgtaatgttacattcgcagctgaagctaatgagtgcaccactcttataaaatgcaccacagaacatgaaaagctgcttattcgccacaaaaacaaaattggcaagtatgctgtttatgctatttggcagccaggtgacactacagagtataatgttacagttttccagggtaaaagtcataaaacttttatgtatacttttccattttatgaaatgtgcgacattaccatgtacatgagcaaacagtataagttgtggcccccacaaaattgtgtggaaaacactggcactttctgctgcactgctatgctaattacagtgctcgctttggtctgtaccctactctatattaaatacaaaagcagacgcagctttattgaggaaaagaaaatgccttaatttactaagttacaaagctaatgtcaccactaactgctttactcgctgcttgcaaaacaaattcaaaaagttagcattataattagaataggatttaaaccccccggtcatttcctgctcaataccattcccctgaacaattgactctatgtgggatatgctccagcgctacaaccttgaagtcaggcttcctggatgtcagcatctgactttggccagcacctgtcccgcggatttgttccagtccaactacagcgacccaccctaacagagatgaccaacacaaccaacgcggccgccgctaccggacttacatctaccacaaatacaccccaagtttctgcctttgtcaataactgggataacttgggcatgtggtggttctccatagcgcttatgtttgtatgccttattattatgtggctcatctgctgcctaaagcgcaaacgcgcccgaccacccatctatagtcccatcattgtgctacacccaaacaatgatggaatccatagattggacggactgaaacacatgttcttttctcttacagtatgattaaatgagacatgattcctcgagtttttatattactgacccttgttgcgcttttttgtgcgtgctccacattggctgcggtttctcacatcgaagtagactgcattccagccttcacagtctatttgctttacggatttgtcaccctcacgctcatctgcagcctcatcactgtggtcatcgcctttatccagtgcattgactgggtctgtgtgcgctttgcatatctcagacaccatccccagtacagggacaggactatagctgagcttcttagaattctttaattatgaaatttactgtgacttttctgctgattatttgcaccctatctgcgttttgttccccgacctccaagcctcaaagacatatatcatgcagattcactcgtatatggaatattccaagttgctacaatgaaaaaagcgatctttccgaagcctggttatatgcaatcatctctgttatggtgttctgcagtaccatcttagccctagctatatatccctaccttgacattggctggaaacgaatagatgccatgaaccacccaactttccccgcgcccgctatgcttccactgcaacaagttgttgccggcggctttgtcccagccaatcagcctcgccccacttctcccacccccactgaaatcagctactttaatctaacaggaggagatgactgacaccctagatctagaaatggacggaattattacagagcagcgcctgctagaaagacgcagggcagcggccgagcaacagcgcatgaatcaagagctccaagacatggttaacttgcaccagtgcaaaaggggtatcttttgtctggtaaagcaggccaaagtcacctacgacagtaataccaccggacaccgccttagctacaagttgccaaccaagcgtcagaaattggtggtcatggtgggagaaaagcccattaccataactcagcactcggtagaaaccgaaggctgcattcactcaccttgtcaaggacctgaggatctctgcacccttattaagaccctgtgcggtctcaaagatcttattccctttaactaataaaaaaaaataataaagcatcacttacttaaaatcagttagcaaatttctgtccagtttattcagcagcacctccttgccctcctcccagctctggtattgcagcttcctcctggctgcaaactttctccacaatctaaatggaatgtcagtttcctcctgttcctgtccatccgcacccactatcttcatgttgttgcagatgaagcgcgcaagaccgtctgaagataccttcaaccccgtgtatccatatgacacggaaaccggtcctccaactgtgccttttcttactcctccctttgtatcccccaatgggtttcaagagagtccccctggggtactctctttgcgcctatccgaacctctagttacctccaatggcatgcttgcgctcaaaatgggcaacggcctctctctggacgaggccggcaaccttacctcccaaaatgtaaccactgtgagcccacctctccgaggagacaagtcaaacataaacctggaaatatctgcacccctcacagttacctcagaagccctaactgtggctgccgccgcacctctaatggtcgcgggcaacacactcaccatgcaatcacaggccccgctaaccgtgcacgactccaaacttagcattgccacccaaggacccctcacagtgtcagaaggaaagctagccctgcaaacatcaggccccctcaccaccaccgatagcagtacccttactatcactgcctcaccccctctaactactgccactggtagcttgggcattgacttgaaagagcccatttatacacaaaatggaaaactaggactaaagtacggggctcctttgcatgtaacagacgacctaaacactttgaccgtagcaactggtccaggtgtgactattaataatacttccttgcaaactaaagttactggagccttgggttttgattcacaaggcaatatgcaacttaatgtagcaggaggactaaggattgattctcaaaacagacgccttatacttgatgttagttatccgtttgatgctcaaaaccaactaaatctaagactaggacagggccctctttttataaactcagcccacaacttggatattaactacaacaaaggcctttacttgtttacagcttcaaacaattccaaaaagcttgaggttaacctaagcactgccaaggggttgatgtttgacgctacagccatagccattaatgcaggagatgggcttgaatttggttcacctaatgcaccaaacacaaatcccctcaaaacaaaaattggccatggcctagaatttgattcaaacaaggctatggttcctaaactaggaactggccttagttttgacagcacaggtgccattacagtaggaaacaaaaataatgataagctaactttgtggaccacaccagctccatctcctaactgtagactaaatgcagagaaagatgctaaactcactttggtcttaacaaaatgtggcagtcaaatacttgctacagtttcagttttggctgttaaaggcagtttggctccaatatctggaacagttcaaagtgctcatcttattataagatttgacgaaaatggagtgctactaaacaattccttcctggacccagaatattggaactttagaaatggagatcttactgaaggcacagcctatacaaacgctgttggatttatgcctaacctatcagcttatccaaaatctcacggtaaaactgccaaaagtaacattgtcagtcaagtttacttaaacggagacaaaactaaacctgtaacactaaccattacactaaacggtacacaggaaacaggagacacaactccatctgcatactctatgtcattttcatgggactggtctggccacaactacattaatgaaatatttgccacatcctcttacactttttcatacattgcccaagaataaagaatcgtttgtgttatgtttcaacgtgtttatttttcaattgcagaaaatttcaagtcatttttcattcagtagtatagccccaccaccacatagcttatacagatcaccgtaccttaatcaaactcacagaaccctagtattcaacctgccacctccctcccaacacacagagtacacagtcctttctccccggctggccttaaaaagcatcatatcatgggtaacagacatattcttaggtgttatattccacacggtttcctgtcgagccaaacgctcatcagtgatattaataaactccccgggcagctcacttaagttcatgtcgctgtccagctgctgagccacaggctgctgtccaacttgcggttgcttaacgggcggcgaaggagaagtccacgcctacatgggggtagagtcataatcgtgcatcaggatagggcggtggtgctgcagcagcgcgcgaataaactgctgccgccgccgctccgtcctgcaggaatacaacatggcagtggtctcctcagcgatgattcgcaccgcccgcagcataaggcgccttgtcctccgggcacagcagcgcaccctgatctcacttaaatcagcacagtaactgcagcacagcaccacaatattgttcaaaatcccacagtgcaaggcgctgtatccaaagctcatggcggggaccacagaacccacgtggccatcataccacaagcgcaggtagattaagtggcgacccctcataaacacgctggacataaacattacctcttttggcatgttgtaattcaccacctcccggtaccatataaacctctgattaaacatggcgccatccaccaccatcctaaaccagctggccaaaacctgcccgccggctatacactgcagggaaccgggactggaacaatgacagtggagagcccaggactcgtaaccatggatcatcatgctcgtcatgatatcaatgttggcacaacacaggcacacgtgcatacacttcctcaggattacaagctcctcccgcgttagaaccatatcccagggaacaacccattcctgaatcagcgtaaatcccacactgcagggaagacctcgcacgtaactcacgttgtgcattgtcaaagtgttacattcgggcagcagcggatgatcctccagtatggtagcgcgggtttctgtctcaaaaggaggtagacgatccctactgtacggagtgcgccgagacaaccgagatcgtgttggtcgtagtgtcatgccaaatggaacgccggacgtagtcatatttcctgaagcaaaaccaggtgcgggcgtgacaaacagatctgcgtctccggtctcgccgcttagatcgctctgtgtagtagttgtagtatatccactctctcaaagcatccaggcgccccctggcttcgggttctatgtaaactccttcatgcgccgctgccctgataacatccaccaccgcagaataagccacacccagccaacctacacattcgttctgcgagtcacacacgggaggagcgggaagagctggaagaaccatgtttttttttttattccaaaagattatccaaaacctcaaaatgaagatctattaagtgaacgcgctcccctccggtggcgtggtcaaactctacagccaaagaacagataatggcatttgtaagatgttgcacaatggcttccaaaaggcaaacggccctcacgtccaagtggacgtaaaggctaaacccttcagggtgaatctcctctataaacattccagcaccttcaaccatgcccaaataattctcatctcgccaccttctcaatatatctctaagcaaatcccgaatattaagtccggccattgtaaaaatctgctccagagcgccctccaccttcagcctcaagcagcgaatcatgattgcaaaaattcaggttcctcacagacctgtataagattcaaaagcggaacattaacaaaaataccgcgatcccgtaggtcccttcgcagggccagctgaacataatcgtgcaggtctgcacggaccagcgcggccacttccccgccaggaaccatgacaaaagaacccacactgattatgacacgcatactcggagctatgctaaccagcgtagccccgatgtaagcttgttgcatgggcggcgatataaaatgcaaggtgctgctcaaaaaatcaggcaaagcctcgcgcaaaaaagaaagcacatcgtagtcatgctcatgcagataaaggcaggtaagctccggaaccaccacagaaaaagacaccatttttctctcaaacatgtctgcgggtttctgcataaacacaaaataaaataacaaaaaaacatttaaacattagaagcctgtcttacaacaggaaaaacaacccttataagcataagacggactacggccatgccggcgtgaccgtaaaaaaactggtcaccgtgattaaaaagcaccaccgacagctcctcggtcatgtccggagtcataatgtaagactcggtaaacacatcaggttgattcacatcggtcagtgctaaaaagcgaccgaaatagcccgggggaatacatacccgcaggcgtagagacaacattacagcccccataggaggtataacaaaattaataggagagaaaaacacataaacacctgaaaaaccctcctgcctaggcaaaatagcaccctcccgctccagaacaacatacagcgcttccacagcggcagccataacagtcagccttaccagtaaaaaagaaaacctattaaaaaaacaccactcgacacggcaccagctcaatcagtcacagtgtaaaaaagggccaagtgcagagcgagtatatataggactaaaaaatgacgtaacggttaaagtccacaaaaaacacccagaaaaccgcacgcgaacctacgcccagaaacgaaagccaaaaaacccacaacttcctcaaatcgtcacttccgttttcccacgttacgtcacttcccattttaagaaaactacaattcccaacacatacaagttactccgccctaaaacctacgtcacccgccccgttcccacgccccgcgccacgtcacaaactccaccccctcattatcatattggcttcaatccaaaataaggtatattattgatgatgtagggataacagggtaattaat

SEQ ID NO: 2 - DNA, 36156 bp, Artificial Sequence
  ICOVIR15K-gp100-tyr
catcatcaataatataccttattttggattgaagccaatatgataatgagggggtggagtttgtgacgtggcgcggggcgtgggaacggggcgggtgacgtagtagtgtggcggaagtgtgatgttgcaagtgtggcggaacacatgtaagcgacggatgtggcaaaagtgacgtttttggtgtgcgccggtgtacacaggaagtgacaattttcgcgcggttttaggcggatgttgtagtaaatttgggcgtaaccgagtaagatttggccattttcgcgggaaaactgaataagaggaagtgaaatctgaataattttgtgttactcatagcgcgtaatatttgtctagggccgcggggactttgaccgtttacgtggagactcgcccaggtgtttttctcaggtgttttccgcgtacgtcggcggctcgtggctctttcgcggcaaaaaggatttggcgcgtaaaagtggttcgagtacgtcggcggctcgtggctctttcgcggcaaaaaggatttggcgcgtaaaagtggttcgaagtacgtcgaccacaaaccccgcccagcgtcttgtcattggcgtcgacgctgtacggggtcaaagttggcgttttattattatagtcagctgacgtgtagtgtatttatacccggtgagttcctcaagaggccactcttgagtgccagcgagtagagttttctcctccgagccgctccgacaccgggactgaaaatgagacatattatctgccacggaggtgttattaccgaagaaatggccgccagtcttttggaccagctgatcgaagaggtactggctgataatcttccacctcctagccattttgaaccacctacccttcacgaactgtatgatttagacgtgacggcccccgaagatcccaacgaggaggcggtttcgcagatttttcccgactctgtaatgttggcggtgcaggaagggattgacttactcacttttccgccggcgcccggttctccggagccgcctcacctttcccggcagcccgagcagccggagcagagagccttgggtccggtttctatgccaaaccttgtaccggaggtgatcgatccacccagtgacgacgaggatgaagagggtgaggagtttgtgttagattatgtggagcaccccgggcacggttgcaggtcttgtcattatcaccggaggaatacgggggacccagatattatgtgttcgctttgctatatgaggacctgtggcatgtttgtctacagtaagtgaaaattatgggcagtgggtgatagagtggtgggtttggtgtggtaattttttttttaatttttacagttttgtggtttaaagaattttgtattgtgatttttttaaaaggtcctgtgtctgaacctgagcctgagcccgagccagaaccggagcctgcaagacctacccgccgtcctaaaatggcgcctgctatcctgagacgcccgacatcacctgtgtccagagaatgcaatagtagtacggatagctgtgactccggtccttctaacacacctcctgagatacacccggtggtcccgctgtgccccattaaaccagttgccgtgagagttggtgggcgtcgccaggctgtggaatgtatcgaggacttgcttaacgagcctgggcaacctttggacttgagctgtaaacgccccaggccataaggtgtaaacctgtgattgcgtgtgtggttaacgcctttgtttgctgaatgagttgatgtaagtttaataaagggtgagataatgtttaacttgcatggcgtgttaaatggggcggggcttaaagggtatataatgcgccgtgggctaatcttggttacatctgacctcatggaggcttgggagtgtttggaagatttttctgctgtgcgtaacttgctggaacagagctctaacagtacctcttggttttggaggtttctgtggggctcatcccaggcaaagttagtctgcagaattaaggaggattacaagtgggaatttgaagagcttttgaaatcctgtggtgagctgtttgattctttgaatctgggtcaccaggcgcttttccaagagaaggtcatcaagactttggatttttccacaccggggcgcgctgcggctgctgttgcttttttgagttttataaaggataaatggagcgaagaaacccatctgagcggggggtacctgctggattttctggccatgcatctgtggagagcggttgtgagacacaagaatcgcctgctactgttgtcttccgtccgcccggcgataataccgacggaggagcagcagcagcagcaggaggaagccaggcggcggcggcaggagcagagcccatggaacccgagagccggcctggaccctcgggaatgaatgttgtacaggtggctgaactgtatccagaactgagacgcattttgacaattacagaggatgggcaggggctaaagggggtaaagagggagcggggggcttgtgaggctacagaggaggctaggaatctagcttttagcttaatgaccagacaccgtcctgagtgtattacttttcaacagatcaaggataattgcgctaatgagcttgatctgctggcgcagaagtattccatagagcagctgaccacttactggctgcagccaggggatgattttgaggaggctattagggtatatgcaaaggtggcacttaggccagattgcaagtacaagatcagcaaacttgtaaatatcaggaattgttgctacatttctgggaacggggccgaggtggagatagatacggaggatagggtggcctttagatgtagcatgataaatatgtggccgggggtgcttggcatggacggggtggttattatgaatgtaaggtttactggccccaattttagcggtacggttttcctggccaataccaaccttatcctacacggtgtaagcttctatgggtttaacaatacctgtgtggaagcctggaccgatgtaagggttcggggctgtgccttttactgctgctggaagggggtggtgtgtcgccccaaaagcagggcttcaattaagaaatgcctctttgaaaggtgtaccttgggtatcctgtctgagggtaactccagggtgcgccacaatgtggcctccgactgtggttgcttcatgctagtgaaaagcgtggctgtgattaagcataacatggtatgtggcaactgcgaggacagggcctctcagatgctgacctgctcggacggcaactgtcacctgctgaagaccattcacgtagccagccactctcgcaaggcctggccagtgtttgagcataacatactgacccgctgttccttgcatttgggtaacaggaggggggtgttcctaccttaccaatgcaatttgagtcacactaagatattgcttgagcccgagagcatgtccaaggtgaacctgaacggggtgtttgacatgaccatgaagatctggaaggtgctgaggtacgatgagacccgcaccaggtgcagaccctgcgagtgtggcggtaaacatattaggaaccagcctgtgatgctggatgtgaccgaggagctgaggcccgatcacttggtgctggcctgcacccgcgctgagtttggctctagcgatgaagatacagattgaggtactgaaatgtgtgggcgtggcttaagggtgggaaagaatatataaggtgggggtcttatgtagttttgtatctgttttgcagcagccgccgccgccatgagcaccaactcgtttgatggaagcattgtgagctcatatttgacaacgcgcatgcccccatgggccggggtgcgtcagaatgtgatgggctccagcattgatggtcgccccgtcctgcccgcaaactctactaccttgacctacgagaccgtgtctggaacgccgttggagactgcagcctccgccgccgcttcagccgctgcagccaccgcccgcgggattgtgactgactttgctttcctgagcccgcttgcaagcagtgcagcttcccgttcatccgcccgcgatgacaagttgacggctcttttggcacaattggattctttgacccgggaacttaatgtcgtttctcagcagctgttggatctgcgccagcaggtttctgccctgaaggcttcctcccctcccaatgcggtttaaaacataaataaaaaaccagactctgtttggatttggatcaagcaagtgtcttgctgtctttatttaggggttttgcgcgcgcggtaggcccgggaccagcggtctcggtcgttgagggtcctgtgtattttttccaggacgtggtaaaggtgactctggatgttcagatacatgggcataagcccgtctctggggtggaggtagcaccactgcagagcttcatgctgcggggtggtgttgtagatgatccagtcgtagcaggagcgctgggcgtggtgcctaaaaatgtctttcagtagcaagctgattgccaggggcaggcccttggtgtaagtgtttacaaagcggttaagctgggatgggtgcatacgtggggatatgagatgcatcttggactgtatttttaggttggctatgttcccagccatatccctccggggattcatgttgtgcagaaccaccagcacagtgtatccggtgcacttgggaaatttgtcatgtagcttagaaggaaatgcgtggaagaacttggagacgcccttgtgacctccaagattttccatgcattcgtccataatgatggcaatgggcccacgggcggcggcctgggcgaagatatttctgggatcactaacgtcatagttgtgttccaggatgagatcgtcataggccatttttacaaagcgcgggcggagggtgccagactgcggtataatggttccatccggcccaggggcgtagttaccctcacagatttgcatttcccacgctttgagttcagatggggggatcatgtctacctgcggggcgatgaagaaaacggtttccggggtaggggagatcagctgggaagaaagcaggttcctgagcagctgcgacttaccgcagccggtgggcccgtaaatcacacctattaccgggtgcaactggtagttaagagagctgcagctgccgtcatccctgagcaggggggccacttcgttaagcatgtccctgactcgcatgttttccctgaccaaatccgccagaaggcgctcgccgcccagcgatagcagttcttgcaaggaagcaaagtttttcaacggtttgagaccgtccgccgtaggcatgcttttgagcgtttgaccaagcagttccaggcggtcccacagctcggtcacctgctctacggcatctcgatccagcatatctcctcgtttcgcgggttggggcggctttcgctgtacggcagtagtcggtgctcgtccagacgggccagggtcatgtctttccacgggcgcagggtcctcgtcagcgtagtctgggtcacggtgaaggggtgcgctccgggctgcgcgctggccagggtgcgcttgaggctggtcctgctggtgctgaagcgctgccggtcttcgccctgcgcgtcggccaggtagcatttgaccatggtgtcatagtccagcccctccgcggcgtggcccttggcgcgcagcttgcccttggaggaggcgccgcacgaggggcagtgcagacttttgagggcgtagagcttgggcgcgagaaataccgattccggggagtaggcatccgcgccgcaggccccgcagacggtctcgcattccacgagccaggtgagctctggccgttcggggtcaaaaaccaggtttcccccatgctttttgatgcgtttcttacctctggtttccatgagccggtgtccacgctcggtgacgaaaaggctgtccgtgtccccgtatacagacttgagaggcctgtcctcgagcggtgttccgcggtcctcctcgtatagaaactcggaccactctgagacaaaggctcgcgtccaggccagcacgaaggaggctaagtgggaggggtagcggtcgttgtccactagggggtccactcgctccagggtgtgaagacacatgtcgccctcttcggcatcaaggaaggtgattggtttgtaggtgtaggccacgtgaccgggtgttcctgaaggggggctataaaagggggtgggggcgcgttcgtcctcactctcttccgcatcgctgtctgcgagggccagctgttggggtgagtactccctctgaaaagcgggcatgacttctgcgctaagattgtcagtttccaaaaacgaggaggatttgatattcacctggcccgcggtgatgcctttgagggtggccgcatccatctggtcagaaaagacaatctttttgttgtcaagcttggtggcaaacgacccgtagagggcgttggacagcaacttggcgatggagcgcagggtttggtttttgtcgcgatcggcgcgctccttggccgcgatgtttagctgcacgtattcgcgcgcaacgcaccgccattcgggaaagacggtggtgcgctcgtcgggcaccaggtgcacgcgccaaccgcggttgtgcagggtgacaaggtcaacgctggtggctacctctccgcgtaggcgctcgttggtccagcagaggcggccgcccttgcgcgagcagaatggcggtagggggtctagctgcgtctcgtccggggggtctgcgtccacggtaaagaccccgggcagcaggcgcgcgtcgaagtagtctatcttgcatccttgcaagtctagcgcctgctgccatgcgcgggcggcaagcgcgcgctcgtatgggttgagtgggggaccccatggcatggggtgggtgagcgcggaggcgtacatgccgcaaatgtcgtaaacgtagaggggctctctgagtattccaagatatgtagggtagcatcttccaccgcggatgctggcgcgcacgtaatcgtatagttcgtgcgagggagcgaggaggtcgggaccgaggttgctacgggcgggctgctctgctcggaagactatctgcctgaagatggcatgtgagttggatgatatggttggacgctggaagacgttgaagctggcgtctgtgagacctaccgcgtcacgcacgaaggaggcgtaggagtcgcgcagcttgttgaccagctcggcggtgacctgcacgtctagggcgcagtagtccagggtttccttgatgatgtcatacttatcctgtcccttttttttccacagctcgcggttgaggacaaactcttcgcggtctttccagtactcttggatcggaaacccgtcggcctccgaacggtaagagcctagcatgtagaactggttgacggcctggtaggcgcagcatcccttttctacgggtagcgcgtatgcctgcgcggccttccggagcgaggtgtgggtgagcgcaaaggtgtccctgaccatgactttgaggtactggtatttgaagtcagtgtcgtcgcatccgccctgctcccagagcaaaaagtccgtgcgctttttggaacgcggatttggcagggcgaaggtgacatcgttgaagagtatctttcccgcgcgaggcataaagttgcgtgtgatgcggaagggtcccggcacctcggaacggttgttaattacctgggcggcgagcacgatctcgtcaaagccgttgatgttgtggcccacaatgtaaagttccaagaagcgcgggatgcccttgatggaaggcaattttttaagttcctcgtaggtgagctcttcaggggagctgagcccgtgctctgaaagggcccagtctgcaagatgagggttggaagcgacgaatgagctccacaggtcacgggccattagcatttgcaggtggtcgcgaaaggtcctaaactggcgacctatggccattttttctggggtgatgcagtagaaggtaagcgggtcttgttcccagcggtcccatccaaggttcgcggctaggtctcgcgcggcagtcactagaggctcatctccgccgaacttcatgaccagcatgaagggcacgagctgcttcccaaaggcccccatccaagtataggtctctacatcgtaggtgacaaagagacgctcggtgcgaggatgcgagccgatcgggaagaactggatctcccgccaccaattggaggagtggctattgatgtggtgaaagtagaagtccctgcgacgggccgaacactcgtgctggcttttgtaaaaacgtgcgcagtactggcagcggtgcacgggctgtacatcctgcacgaggttgacctgacgaccgcgcacaaggaagcagagtgggaatttgagcccctcgcctggcgggtttggctggtggtcttctacttcggctgcttgtccttgaccgtctggctgctcgaggggagttacggtggatcggaccaccacgccgcgcgagcccaaagtccagatgtccgcgcgcggcggtcggagcttgatgacaacatcgcgcagatgggagctgtccatggtctggagctcccgcggcgtcaggtcaggcgggagctcctgcaggtttacctcgcatagacgggtcagggcgcgggctagatccaggtgatacctaatttccaggggctggttggtggcggcgtcgatggcttgcaagaggccgcatccccgcggcgcgactacggtaccgcgcggcgggcggtgggccgcgggggtgtccttggatgatgcatctaaaagcggtgacgcgggcgagcccccggaggtagggggggctccggacccgccgggagagggggcaggggcacgtcggcgccgcgcgcgggcaggagctggtgctgcgcgcgtaggttgctggcgaacgcgacgacgcggcggttgatctcctgaatctggcgcctctgcgtgaagacgacgggcccggtgagcttgagcctgaaagagagttcgacagaatcaatttcggtgtcgttgacggcggcctggcgcaaaatctcctgcacgtctcctgagttgtcttgataggcgatctcggccatgaactgctcgatctcttcctcctggagatctccgcgtccggctcgctccacggtggcggcgaggtcgttggaaatgcgggccatgagctgcgagaaggcgttgaggcctccctcgttccagacgcggctgtagaccacgcccccttcggcatcgcgggcgcgcatgaccacctgcgcgagattgagctccacgtgccgggcgaagacggcgtagtttcgcaggcgctgaaagaggtagttgagggtggtggcggtgtgttctgccacgaagaagtacataacccagcgtcgcaacgtggattcgttgatatcccccaaggcctcaaggcgctccatggcctcgtagaagtccacggcgaagttgaaaaactgggagttgcgcgccgacacggttaactcctcctccagaagacggatgagctcggcgacagtgtcgcgcacctcgcgctcaaaggctacaggggcctcttcttcttcttcaatctcctcttccataagggcctccccttcttcttcttctggcggcggtgggggaggggggacacggcggcgacgacggcgcaccgggaggcggtcgacaaagcgctcgatcatctccccgcggcgacggcgcatggtctcggtgacggcgcggccgttctcgcgggggcgcagttggaagacgccgcccgtcatgtcccggttatgggttggcggggggctgccatgcggcagggatacggcgctaacgatgcatctcaacaattgttgtgtaggtactccgccgccgagggacctgagcgagtccgcatcgaccggatcggaaaacctctcgagaaaggcgtctaaccagtcacagtcgcaaggtaggctgagcaccgtggcgggcggcagcgggcggcggtcggggttgtttctggcggaggtgctgctgatgatgtaattaaagtaggcggtcttgagacggcggatggtcgacagaagcaccatgtccttgggtccggcctgctgaatgcgcaggcggtcggccatgccccaggcttcgttttgacatcggcgcaggtctttgtagtagtcttgcatgagcctttctaccggcacttcttcttctccttcctcttgtcctgcatctcttgcatctatcgctgcggcggcggcggagtttggccgtaggtggcgccctcttcctcccatgcgtgtgaccccgaagcccctcatcggctgaagcagggctaggtcggcgacaacgcgctcggctaatatggcctgctgcacctgcgtgagggtagactggaagtcatccatgtccacaaagcggtggtatgcgcccgtgttgatggtgtaagtgcagttggccataacggaccagttaacggtctggtgacccggctgcgagagctcggtgtacctgagacgcgagtaagccctcgagtcaaatacgtagtcgttgcaagtccgcaccaggtactggtatcccaccaaaaagtgcggcggcggctggcggtagaggggccagcgtagggtggccggggctccgggggcgagatcttccaacataaggcgatgatatccgtagatgtacctggacatccaggtgatgccggcggcggtggtggaggcgcgcggaaagtcgcggacgcggttccagatgttgcgcagcggcaaaaagtgctccatggtcgggacgctctggccggtcaggcgcgcgcaatcgttgacgctctagaccgtgcaaaaggagagcctgtaagcgggcactcttccgtggtctggtggataaattcgcaagggtatcatggcggacgaccggggttcgagccccgtatccggccgtccgccgtgatccatgcggttaccgcccgcgtgtcgaacccaggtgtgcgacgtcagacaacgggggagtgctccttttggcttccttccaggcgcggcggctgctgcgctagcttttttggccactggccgcgcgcagcgtaagcggttaggctggaaagcgaaagcattaagtggctcgctccctgtagccggagggttattttccaagggttgagtcgcgggacccccggttcgagtctcggaccggccggactgcggcgaacgggggtttgcctccccgtcatgcaagaccccgcttgcaaattcctccggaaacagggacgagccccttttttgcttttcccagatgcatccggtgctgcggcagatgcgcccccctcctcagcagcggcaagagcaagagcagcggcagacatgcagggcaccctcccctcctcctaccgcgtcaggaggggcgacatccgcggttgacgcggcagcagatggtgattacgaacccccgcggcgccgggcccggcactacctggacttggaggagggcgagggcctggcgcggctaggagcgccctctcctgagcggtacccaagggtgcagctgaagcgtgatacgcgtgaggcgtacgtgccgcggcagaacctgtttcgcgaccgcgagggagaggagcccgaggagatgcgggatcgaaagttccacgcagggcgcgagctgcggcatggcctgaatcgcgagcggttgctgcgcgaggaggactttgagcccgacgcgcgaaccgggattagtcccgcgcgcgcacacgtggcggccgccgacctggtaaccgcatacgagcagacggtgaaccaggagattaactttcaaaaaagctttaacaaccacgtgcgtacgcttgtggcgcgcgaggaggtggctataggactgatgcatctgtgggactttgtaagcgcgctggagcaaaacccaaatagcaagccgctcatggcgcagctgttccttatagtgcagcacagcagggacaacgaggcattcagggatgcgctgctaaacatagtagagcccgagggccgctggctgctcgatttgataaacatcctgcagagcatagtggtgcaggagcgcagcttgagcctggctgacaaggtggccgccatcaactattccatgcttagcctgggcaagttttacgcccgcaagatataccataccccttacgttcccatagacaaggaggtaaagatcgaggggttctacatgcgcatggcgctgaaggtgcttaccttgagcgacgacctgggcgtttatcgcaacgagcgcatccacaaggccgtgagcgtgagccggcggcgcgagctcagcgaccgcgagctgatgcacagcctgcaaagggccctggctggcacgggcagcggcgatagagaggccgagtcctactttgacgcgggcgctgacctgcgctgggccccaagccgacgcgccctggaggcagctggggccggacctgggctggcggtggcacccgcgcgcgctggcaacgtcggcggcgtggaggaatatgacgaggacgatgagtacgagccagaggacggcgagtactaagcggtgatgtttctgatcagatgatgcaagacgcaacggacccggcggtgcgggcggcgctgcagagccagccgtccggccttaactccacggacgactggcgccaggtcatggaccgcatcatgtcgctgactgcgcgcaatcctgacgcgttccggcagcagccgcaggccaaccggctctccgcaattctggaagcggtggtcccggcgcgcgcaaaccccacgcacgagaaggtgctggcgatcgtaaacgcgctggccgaaaacagggccatccggcccgacgaggccggcctggtctacgacgcgctgcttcagcgcgtggctcgttacaacagcggcaacgtgcagaccaacctggaccggctggtgggggatgtgcgcgaggccgtggcgcagcgtgagcgcgcgcagcagcagggcaacctgggctccatggttgcactaaacgccttcctgagtacacagcccgccaacgtgccgcggggacaggaggactacaccaactttgtgagcgcactgcggctaatggtgactgagacaccgcaaagtgaggtgtaccagtctgggccagactattttttccagaccagtagacaaggcctgcagaccgtaaacctgagccaggctttcaaaaacttgcaggggctgtggggggtgcgggctcccacaggcgaccgcgcgaccgtgtctagcttgctgacgcccaactcgcgcctgttgctgctgctaatagcgcccttcacggacagtggcagcgtgtcccgggacacatacctaggtcacttgctgacactgtaccgcgaggccataggtcaggcgcatgtggacgagcatactttccaggagattacaagtgtcagccgcgcgctggggcaggaggacacgggcagcctggaggcaaccctaaactacctgctgaccaaccggcggcagaagatcccctcgttgcacagtttaaacagcgaggaggagcgcattttgcgctacgtgcagcagagcgtgagccttaacctgatgcgcgacggggtaacgcccagcgtggcgctggacatgaccgcgcgcaacatggaaccgggcatgtatgcctcaaaccggccgtttatcaaccgcctaatggactacttgcatcgcgcggccgccgtgaaccccgagtatttcaccaatgccatcttgaacccgcactggctaccgccccctggtttctacaccgggggattcgaggtgcccgagggtaacgatggattcctctgggacgacatagacgacagcgtgttttccccgcaaccgcagaccctgctagagttgcaacagcgcgagcaggcagaggcggcgctgcgaaaggaaagcttccgcaggccaagcagcttgtccgatctaggcgctgcggccccgcggtcagatgctagtagcccatttccaagcttgatagggtctcttaccagcactcgcaccacccgcccgcgcctgctgggcgaggaggagtacctaaacaactcgctgctgcagccgcagcgcgaaaaaaacctgcctccggcatttcccaacaacgggatagagagcctagtggacaagatgagtagatggaagacgtacgcgcaggagcacagggacgtgccaggcccgcgcccgcccacccgtcgtcaaaggcacgaccgtcagcggggtctggtgtgggaggacgatgactcggcagacgacagcagcgtcctggatttgggagggagtggcaacccgtttgcgcaccttcgccccaggctggggagaatgttttaaaaaaaaaaaagcatgatgcaaaataaaaaactcaccaaggccatggcaccgagcgttggttttcttgtattccccttagtatgcggcgcgcggcgatgtatgaggaaggtcctcctccctcctacgagagtgtggtgagcgcggcgccagtggcggcggcgctgggttctcccttcgatgctcccctggacccgccgtttgtgcctccgcggtacctgcggcctaccggggggagaaacagcatccgttactctgagttggcacccctattcgacaccacccgtgtgtacctggtggacaacaagtcaacggatgtggcatccctgaactaccagaacgaccacagcaactttctgaccacggtcattcaaaacaatgactacagcccgggggaggcaagcacacagaccatcaatcttgacgaccggtcgcactggggcggcgacctgaaaaccatcctgcataccaacatgccaaatgtgaacgagttcatgtttaccaataagtttaaggcgcgggtgatggtgtcgcgcttgcctactaaggacaatcaggtggagctgaaatacgagtgggtggagttcacgctgcccgagggcaactactccgagaccatgaccatagaccttatgaacaacgcgatcgtggagcactacttgaaagtgggcagacagaacggggttctggaaagcgacatcggggtaaagtttgacacccgcaacttcagactggggtttgaccccgtcactggtcttgtcatgcctggggtatatacaaacgaagccttccatccagacatcattttgctgccaggatgcggggtggacttcacccacagccgcctgagcaacttgttgggcatccgcaagcggcaacccttccaggagggctttaggatcacctacgatgatctggagggtggtaacattcccgcactgttggatgtggacgcctaccaggcgagcttgaaagatgacaccgaacagggcgggggtggcgcaggcggcagcaacagcagtggcagcggcgcggaagagaactccaacgcggcagccgcggcaatgcagccggtggaggacatgaacgatcatgccattcgcggcgacacctttgccacacgggctgaggagaagcgcgctgaggccgaagcagcggccgaagctgccgcccccgctgcgcaacccgaggtcgagaagcctcagaagaaaccggtgatcaaacccctgacagaggacagcaagaaacgcagttacaacctaataagcaatgacagcaccttcacccagtaccgcagctggtaccttgcatacaactacggcgaccctcagaccggaatccgctcatggaccctgctttgcactcctgacgtaacctgcggctcggagcaggtctactggtcgttgccagacatgatgcaagaccccgtgaccttccgctccacgcgccagatcagcaactttccggtggtgggcgccgagctgttgcccgtgcactccaagagcttctacaacgaccaggccgtctactcccaactcatccgccagtttacctctctgacccacgtgttcaatcgctttcccgagaaccagattttggcgcgcccgccagcccccaccatcaccaccgtcagtgaaaacgttcctgctctcacagatcacgggacgctaccgctgcgcaacagcatcggaggagtccagcgagtgaccattactgacgccagacgccgcacctgcccctacgtttacaaggccctgggcatagtctcgccgcgcgtcctatcgagccgcactttttgagcaagcatgtccatccttatatcgcccagcaataacacaggctggggcctgcgcttcccaagcaagatgtttggcggggccaagaagcgctccgaccaacacccagtgcgcgtgcgcgggcactaccgcgcgccctggggcgcgcacaaacgcggccgcactgggcgcaccaccgtcgatgacgccatcgacgcggtggtggaggaggcgcgcaactacacgcccacgccgccaccagtgtccacagtggacgcggccattcagaccgtggtgcgcggagcccggcgctatgctaaaatgaagagacggcggaggcgcgtagcacgtcgccaccgccgccgacccggcactgccgcccaacgcgcggcggcggccctgcttaaccgcgcacgtcgcaccggccgacgggcggccatgcgggccgctcgaaggctggccgcgggtattgtcactgtgccccccaggtccaggcgacgagcggccgccgcagcagccgcggccattagtgctatgactcagggtcgcaggggcaacgtgtattgggtgcgcgactcggttagcggcctgcgcgtgcccgtgcgcacccgccccccgcgcaactagattgcaagaaaaaactacttagactcgtactgttgtatgtatccagcggcggcggcgcgcaacgaagctatgtccaagcgcaaaatcaaagaagagatgctccaggtcatcgcgccggagatctatggccccccgaagaaggaagagcaggattacaagccccgaaagctaaagcgggtcaaaaagaaaaagaaagatgatgatgatgaacttgacgacgaggtggaactgctgcacgctaccgcgcccaggcgacgggtacagtggaaaggtcgacgcgtaaaacgtgttttgcgacccggcaccaccgtagtctttacgcccggtgagcgctccacccgcacctacaagcgcgtgtatgatgaggtgtacggcgacgaggacctgcttgagcaggccaacgagcgcctcggggagtttgcctacggaaagcggcataaggacatgctggcgttgccgctggacgagggcaacccaacacctagcctaaagcccgtaacactgcagcaggtgctgcccgcgcttgcaccgtccgaagaaaagcgcggcctaaagcgcgagtctggtgacttggcacccaccgtgcagctgatggtacccaagcgccagcgactggaagatgtcttggaaaaaatgaccgtggaacctgggctggagcccgaggtccgcgtgcggccaatcaagcaggtggcgccgggactgggcgtgcagaccgtggacgttcagatacccactaccagtagcaccagtattgccaccgccacagagggcatggagacacaaacgtccccggttgcctcagcggtggcggatgccgcggtgcaggcggtcgctgcggccgcgtccaagacctctacggaggtgcaaacggacccgtggatgtttcgcgtttcagccccccggcgcccgcgcggttcgaggaagtacggcgccgccagcgcgctactgcccgaatatgccctacatccttccattgcgcctacccccggctatcgtggctacacctaccgccccagaagacgagcaactacccgacgccgaaccaccactggaacccgccgccgccgtcgccgtcgccagcccgtgctggccccgatttccgtgcgcagggtggctcgcgaaggaggcaggaccctggtgctgccaacagcgcgctaccaccccagcatcgtttaaaagccggtctttgtggttcttgcagatatggccctcacctgccgcctccgtttcccggtgccgggattccgaggaagaatgcaccgtaggaggggcatggccggccacggcctgacgggcggcatgcgtcgtgcgcaccaccggcggcggcgcgcgtcgcaccgtcgcatgcgcggcggtatcctgcccctccttattccactgatcgccgcggcgattggcgccgtgcccggaattgcatccgtggccttgcaggcgcagagacactgattaaaaacaagttgcatgtggaaaaatcaaaataaaaagtctggactctcacgctcgcttggtcctgtaactattttgtagaatggaagacatcaactttgcgtctctggccccgcgacacggctcgcgcccgttcatgggaaactggcaagatatcggcaccagcaatatgagcggtggcgccttcagctggggctcgctgtggagcggcattaaaaatttcggttccaccgttaagaactatggcagcaaggcctggaacagcagcacaggccagatgctgagggataagttgaaagagcaaaatttccaacaaaaggtggtagatggcctggcctctggcattagcggggtggtggacctggccaaccaggcagtgcaaaataagattaacagtaagcttgatccccgccctcccgtagaggagcctccaccggccgtggagacagtgtctccagaggggcgtggcgaaaagcgtccgcgccccgacagggaagaaactctggtgacgcaaatagacgagcctccctcgtacgaggaggcactaaagcaaggcctgcccaccacccgtcccatcgcgcccatggctaccggagtgctgggccagcacacacccgtaacgctggacctgcctccccccgccgacacccagcagaaacctgtgctgccaggcccgaccgccgttgttgtaacccgtcctagccgcgcgtccctgcgccgcgccgccagcggtccgcgatcgttgcggcccgtagccagtggcaactggcaaagcacactgaacagcatcgtgggtctgggggtgcaatccctgaagcgccgacgatgcttctgaatagctaacgtgtcgtatgtgtgtcatgtatgcgtccatgtcgccgccagaggagctgctgagccgccgcgcgcccgctttccaagatggctaccccttcgatgatgccgcagtggtcttacatgcacatctcgggccaggacgcctcggagtacctgagccccgggctggtgcagtttgcccgcgccaccgagacgtacttcagcctgaataacaagtttagaaaccccacggtggcgcctacgcacgacgtgaccacagaccggtcccagcgtttgacgctgcggttcatccctgtggaccgtgaggatactgcgtactcgtacaaggcgcggttcaccctagctgtgggtgataaccgtgtgctggacatggcttccacgtactttgacatccgcggcgtgctggacaggggccctacttttaagccctactctggcactgcctacaacgccctggctcccaagggtgccccaaatccttgcgaatgggatgaagctgctactgctcttgaaataaacctagaagaagaggacgatgacaacgaagacgaagtagacgagcaagctgagcagcaaaaaactcacgtatttgggcaggcgccttattctggtataaatattacaaaggagggtattcaaataggtgtcgaaggtcaaacacctaaatatgccgataaaacatttcaacctgaacctcaaataggagaatctcagtggtacgaaactgaaattaatcatgcagctgggagagtccttaaaaagactaccccaatgaaaccatgttacggttcatatgcaaaacccacaaatgaaaatggagggcaaggcattcttgtaaagcaacaaaatggaaagctagaaagtcaagtggaaatgcaatttttctcaactggaagcggttctcgctacctggagcctggcccagtgactgccgctggttccggaagcagatacatggacggaacaatgtcccaggttgccggttctggctcccctaaagtggtattgtacagtgaagatgtagatatagaaaccccagacactcatatttcttacatgcccactattaaggaaggtaactcacgagaactaatgggccaacaatctatgcccaacaggcctaattacattgcttttagggacaattttattggtctaatgtattacaacagcacgggtaatatgggtgttctggcgggccaagcatcgcagttgaatgctgttgtagatttgcaagacagaaacacagagctttcataccagcttttgcttgattccattggtgatagaaccaggtacttttctatgtggaatcaggctgttgacagctatgatccagatgttagaattattgaaaatcatggaactgaagatgaacttccaaattactgctttccactgggaggtgtgattaatacagagactcttaccaaggtaaaacctaaaacaggtcaggaaaatggatgggaaaaagatgctacagaattttcagataaaaatgaaataagagttggaaataattttgccatggaaatcaatctaaatgccaacctgtggagaaatttcctgtactccaacatagcgctgtatttgcccgacaagctaaagtacagtccttccaacgtaaaaatttctgataacccaaacacctacgactacatgaacaagcgagtggtggctcccgggttagtggactgctacattaaccttggagcacgctggtcccttgactatatggacaacgtcaacccatttaaccaccaccgcaatgctggcctgcgctaccgctcaatgttgctgggcaatggtcgctatgtgcccttccacatccaggtgcctcagaagttctttgccattaaaaacctccttctcctgccgggctcatacacctacgagtggaacttcaggaaggatgttaacatggttctgcagagctccctaggaaatgacctaagggttgacggagccagcattaagtttgatagcatttgcctttacgccaccttcttccccatggcccacaacaccgcctccacgcttgaggccatgcttagaaacgacaccaacgaccagtcctttaacgactatctctccgccgccaacatgctctaccctatacccgccaacgctaccaacgtgcccatatccatcccctcccgcaactgggcggctttccgcggctgggccttcacgcgccttaagactaaggaaaccccatcactgggctcgggctacgacccttattacacctactctggctctataccctacctagatggaaccttttacctcaaccacacctttaagaaggtggccattacctttgactcttctgtcagctggcctggcaatgaccgcctgcttacccccaacgagtttgaaattaagcgctcagttgacggggagggttacaacgttgcccagtgtaacatgaccaaagactggttcctggtacaaatgctagctaactacaacattggctaccagggcttctatatcccagagagctacaaggaccgcatgtactccttctttagaaacttccagcccatgagccgtcaggtggtggatgatactaaatacaaggactaccaacaggtgggcatcctacaccaacacaacaactctggatttgttggctaccttgcccccaccatgcgcgaaggacaggcctaccctgctaacttcccctatccgcttataggcaagaccgcagttgacagcattacccagaaaaagtttctttgcgatcgcaccctttggcgcatcccattctccagtaactttatgtccatgggcgcactcacagacctgggccaaaaccttctctacgccaactccgcccacgcgctagacatgacttttgaggtggatcccatggacgagcccacccttctttatgttttgtttgaagtctttgacgtggtccgtgtgcaccagccgcaccgcggcgtcatcgaaaccgtgtacctgcgcacgcccttctcggccggcaacgccacaacataaagaagcaagcaacatcaacaacagctgccgccatgggctccagtgagcaggaactgaaagccattgtcaaagatcttggttgtgggccatattttttgggcacctatgacaagcgctttccaggctttgtttctccacacaagctcgcctgcgccatagtcaatacggccggtcgcgagactgggggcgtacactggatggcctttgcctggaacccgcactcaaaaacatgctacctctttgagccctttggcttttctgaccagcgactcaagcaggtttaccagtttgagtacgagtcactcctgcgccgtagcgccattgcttcttcccccgaccgctgtataacgctggaaaagtccacccaaagcgtacaggggcccaactcggccgcctgtggactattctgctgcatgtttctccacgcctttgccaactggccccaaactcccatggatcacaaccccaccatgaaccttattaccggggtacccaactccatgctcaacagtccccaggtacagcccaccctgcgtcgcaaccaggaacagctctacagcttcctggagcgccactcgccctacttccgcagccacagtgcgcagattaggagcgccacttctttttgtcacttgaaaaacatgtaaaaataatgtactagagacactttcaataaaggcaaatgcttttatttgtacactctcgggtgattatttacccccacccttgccgtctgcgccgtttaaaaatcaaaggggttctgccgcgcatcgctatgcgccactggcagggacacgttgcgatactggtgtttagtgctccacttaaactcaggcacaaccatccgcggcagctcggtgaagttttcactccacaggctgcgcaccatcaccaacgcgtttagcaggtcgggcgccgatatcttgaagtcgcagttggggcctccgccctgcgcgcgcgagttgcgatacacagggttgcagcactggaacactatcagcgccgggtggtgcacgctggccagcacgctcttgtcggagatcagatccgcgtccaggtcctccgcgttgctcagggcgaacggagtcaactttggtagctgccttcccaaaaagggcgcgtgcccaggctttgagttgcactcgcaccgtagtggcatcaaaaggtgaccgtgcccggtctgggcgttaggatacagcgcctgcataaaagccttgatctgcttaaaagccacctgagcctttgcgccttcagagaagaacatgccgcaagacttgccggaaaactgattggccggacaggccgcgtcgtgcacgcagcaccttgcgtcggtgttggagatctgcaccacatttcggccccaccggttcttcacgatcttggccttgctagactgctccttcagcgcgcgctgcccgttttcgctcgtcacatccatttcaatcacgtgctccttatttatcataatgcttccgtgtagacacttaagctcgccttcgatctcagcgcagcggtgcagccacaacgcgcagcccgtgggctcgtgatgcttgtaggtcacctctgcaaacgactgcaggtacgcctgcaggaatcgccccatcatcgtcacaaaggtcttgttgctggtgaaggtcagctgcaacccgcggtgctcctcgttcagccaggtcttgcatacggccgccagagcttccacttggtcaggcagtagtttgaagttcgcctttagatcgttatccacgtggtacttgtccatcagcgcgcgcgcagcctccatgcccttctcccacgcagacacgatcggcacactcagcgggttcatcaccgtaatttcactttccgcttcgctgggctcttcctcttcctcttgcgtccgcataccacgcgccactgggtcgtcttcattcagccgccgcactgtgcgcttacctcctttgccatgcttgattagcaccggtgggttgctgaaacccaccatttgtagcgccacatcttctctttcttcctcgctgtccacgattacctctggtgatggcgggcgctcgggcttgggagaagggcgcttctttttcttcttgggcgcaatggccaaatccgccgccgaggtcgatggccgcgggctgggtgtgcgcggcaccagcgcgtcttgtgatgagtcttcctcgtcctcggactcgatacgccgcctcatccgcttttttgggggcgcccggggaggcggcggcgacggggacggggacgacacgtcctccatggttgggggacgtcgcgccgcaccgcgtccgcgctcgggggtggtttcgcgctgctcctcttcccgactggccatttccttctcctataggcagaaaaagatcatggagtcagtcgagaagaaggacagcctaaccgccccctctgagttcgccaccaccgcctccaccgatgccgccaacgcgcctaccaccttccccgtcgaggcacccccgcttgaggaggaggaagtgattatcgagcaggacccaggttttgtaagcgaagacgacgaggaccgctcagtaccaacagaggataaaaagcaagaccaggacaacgcagaggcaaacgaggaacaagtcgggcggggggacgaaaggcatggcgactacctagatgtgggagacgacgtgctgttgaagcatctgcagcgccagtgcgccattatctgcgacgcgttgcaagagcgcagcgatgtgcccctcgccatagcggatgtcagccttgcctacgaacgccacctattctcaccgcgcgtaccccccaaacgccaagaaaacggcacatgcgagcccaacccgcgcctcaacttctaccccgtatttgccgtgccagaggtgcttgccacctatcacatctttttccaaaactgcaagatacccctatcctgccgtgccaaccgcagccgagcggacaagcagctggccttgcggcagggcgctgtcatacctgatatcgcctcgctcaacgaagtgccaaaaatctttgagggtcttggacgcgacgagaagcgcgcggcaaacgctctgcaacaggaaaacagcgaaaatgaaagtcactctggagtgttggtggaactcgagggtgacaacgcgcgcctagccgtactaaaacgcagcatcgaggtcacccactttgcctacccggcacttaacctaccccccaaggtcatgagcacagtcatgagtgagctgatcgtgcgccgtgcgcagcccctggagagggatgcaaatttgcaagaacaaacagaggagggcctacccgcagttggcgacgagcagctagcgcgctggcttcaaacgcgcgagcctgccgacttggaggagcgacgcaaactaatgatggccgcagtgctcgttaccgtggagcttgagtgcatgcagcggttctttgctgacccggagatgcagcgcaagctagaggaaacattgcactacacctttcgacagggctacgtacgccaggcctgcaagatctccaacgtggagctctgcaacctggtctcctaccttggaattttgcacgaaaaccgccttgggcaaaacgtgcttcattccacgctcaagggcgaggcgcgccgcgactacgtccgcgactgcgtttacttatttctatgctacacctggcagacggccatgggcgtttggcagcagtgcttggaggagtgcaacctcaaggagctgcagaaactgctaaagcaaaacttgaaggacctatggacggccttcaacgagcgctccgtggccgcgcacctggcggacatcattttccccgaacgcctgcttaaaaccctgcaacagggtctgccagacttcaccagtcaaagcatgttgcagaactttaggaactttatcctagagcgctcaggaatcttgcccgccacctgctgtgcacttcctagcgactttgtgcccattaagtaccgcgaatgccctccgccgctttggggccactgctaccttctgcagctagccaactaccttgcctaccactctgacataatggaagacgtgagcggtgacggtctactggagtgtcactgtcgctgcaacctatgcaccccgcaccgctccctggtttgcaattcgcagctgcttaacgaaagtcaaattatcggtacctttgagctgcagggtccctcgcctgacgaaaagtccgcggctccggggttgaaactcactccggggctgtggacgtcggcttaccttcgcaaatttgtacctgaggactaccacgcccacgagattaggttctacgaagaccaatcccgcccgccaaatgcggagcttaccgcctgcgtcattacccagggccacattcttggccaattgcaagccatcaacaaagcccgccaagagtttctgctacgaaagggacggggggtttacttggacccccagtccggcgaggagctcaacccaatccccccgccgccgcagccctatcagcagcagccgcgggcccttgcttcccaggatggcacccaaaaagaagctgcagctgccgccgccacccacggacgaggaggaatactgggacagtcaggcagaggaggttttggacgaggaggaggaggacatgatggaagactgggagagcctagacgaggaagcttccgaggtcgaagaggtgtcagacgaaacaccgtcaccctcggtcgcattcccctcgccggcgccccagaaatcggcaaccggttccagcatggctacaacctccgctcctcaggcgccgccggcactgcccgttcgccgacccaaccgtagatgggacaccactggaaccagggccggtaagtccaagcagccgccgccgttagcccaagagcaacaacagcgccaaggctaccgctcatggcgcgggcacaagaacgccatagttgcttgcttgcaagactgtgggggcaacatctccttcgcccgccgctttcttctctaccatcacggcgtggccttcccccgtaacatcctgcattactaccgtcatctctacagcccatactgcaccggcggcagcggcagcggcagcaacagcagcggccacacagaagcaaaggcgaccggatagcaagactctgacaaagcccaagaaatccacagcggcggcagcagcaggaggaggagcgctgcgtctggcgcccaacgaacccgtatcgacccgcgagcttagaaacaggatttttcccactctgtatgctatatttcaacagagcaggggccaagaacaagagctgaaaataaaaaacaggtctctgcgatccctcacccgcagctgcctgtatcacaaaagcgaagatcagcttcggcgcacgctggaagacgcggaggctctcttcagtaaatactgcgcgctgactcttaaggactagtttcgcgccctttctcaaatttaagcgcgaaaactacgtcatctccagcggccacacccggcgccagcacctgtcgtcagcgccattatgagcaaggaaattcccacgccctacatgtggagttaccagccacaaatgggacttgcggctggagctgcccaagactactcaacccgaataaactacatgagcgcgggaccccacatgatatcccgggtcaacggaatccgcgcccaccgaaaccgaattctcttggaacaggcggctattaccaccacacctcgtaataaccttaatccccgtagttggcccgctgccctggtgtaccaggaaagtcccgctcccaccactgtggtacttcccagagacgcccaggccgaagttcagatgactaactcaggggcgcagcttgcgggcggctttcgtcacagggtgcggtcgcccgggcagggtataactcacctgacaatcagagggcgaggtattcagctcaacgacgagtcggtgagctcctcgcttggtctccgtccggacgggacatttcagatcggcggcgccggccgtccttcattcacgcctcgtcaggcaatcctaactctgcagacctcgtcctctgagccgcgctctggaggcattggaactctgcaatttattgaggagtttgtgccatcggtctactttaaccccttctcgggacctcccggccactatccggatcaatttattcctaactttgacgcggtaaaggactcggcggacggctacgactgaatgttaagtggagaggcagagcaactgcgcctgaaacacctggtccactgtcgccgccacaagtgctttgcccgcgactccggtgagttttgctactttgaattgcccgaggatcatatcgagggcccggcgcacggcgtccggcttaccgcccagggagagcttgcccgtagcctgattcgggagtttacccagcgccccctgctagttgagcgggacaggggaccctgtgttctcactgtgatttgcaactgtcctaaccttggattacatcaagatctttgttgccatctctgtgctgagtataataaatacagaaattaaaatatactggggctcctatcgccatcctgtaaacgccaccgtcttcacccgcccaagcaaaccaaggcgaaccttacctggtacttttaacatctctccctctgtgatttacaacagtttcaacccagacggagtgagtctacgagagaacctctccgagctcagctactccatcagaaaaaacaccaccctccttacctgccgggaacgtacgagtgcgtcaccggccgctgcaccacacctaccgcctgaccgtaaaccagactttttccggacagacctcaataactctgtttaccagaacaggaggtgagcttagaaaacccttagggtattaggccaaaggcgcagctactgtggggtttatgaacaattcaagcaactctacgggctattctaattcaggtttctctagaatcggggttggggttattctctgtcttgtgattctctttattcttatactaacgcttctctgcctaaggctcgccgcctgctgtgtgcacatttgcatttattgtcagctttttaaacgctggggtcgccacccaagatgattaggtacataatcctaggtttactcacccttgcgtcagcccacggtaccacccaaaaggtggattttaaggagccagcctgtaatgttacattcgcagctgaagctaatgagtgcaccactcttataaaatgcaccacagaacatgaaaagctgcttattcgccacaaaaacaaaattggcaagtatgctgtttatgctatttggcagccaggtgacactacagagtataatgttacagttttccagggtaaaagtcataaaacttttatgtatacttttccattttatgaaatgtgcgacattaccatgtacatgagcaaacagtataagttgtggcccccacaaaattgtgtggaaaacactggcactttctgctgcactgctatgctaattacagtgctcgctttggtctgtaccctactctatattaaatacaaaagcagacgcagctttattgaggaaaagaaaatgccttaatttactaagttacaaagctaatgtcaccactaactgctttactcgctgcttgcaaaacaaattcaaaaagttagcattataattagaataggatttaaaccccccggtcatttcctgctcaataccattcccctgaacaattgactctatgtgggatatgctccagcgctacaaccttgaagtcaggcttcctggatgtcagcatctgactttggccagcacctgtcccgcggatttgttccagtccaactacagcgacccaccctaacagagatgaccaacacaaccaacgcggccgccgctaccggacttacatctaccacaaatacaccccaagtttctgcctttgtcaataactgggataacttgggcatgtggtggttctccatagcgcttatgtttgtatgccttattattatgtggctcatctgctgcctaaagcgcaaacgcgcccgaccacccatctatagtcccatcattgtgctacacccaaacaatgatggaatccatagattggacggactgaaacacatgttcttttctcttacagtatgattaaatgagacatgattcctcgagtttttatattactgacccttgttgcgcttttttgtgcgtgctccacattggctgcggtttctcacatcgaagtagactgcattccagccttcacagtctatttgctttacggatttgtcaccctcacgctcatctgcagcctcatcactgtggtcatcgcctttatccagtgcattgactgggtctgtgtgcgctttgcatatctcagacaccatccccagtacagggacaggactatagctgagcttcttagaattctttaattatgaaatttactgtgacttttctgctgattatttgcaccctatctgcgttttgttccccgacctccaagcctcaaagacatatatcatgcagattcactcgtatatggaatattccaagttgctacaatgaaaaaagcgatctttccgaagcctggttatatgcaatcatctctgttatggtgttctgcagtaccatcttagccctagctatatatccctaccttgacattggctggaaacgaatagatgccatgaaccacccaactttccccgcgcccgctatgcttccactgcaacaagttgttgccggcggctttgtcccagccaatcagcctcgccccacttctcccacccccactgaaatcagctactttaatctaacaggaggagatgactgacaccctagatctagaaatggacggaattattacagagcagcgcctgctagaaagacgcagggcagcggccgagcaacagcgcatgaatcaagagctccaagacatggttaacttgcaccagtgcaaaaggggtatcttttgtctggtaaagcaggccaaagtcacctacgacagtaataccaccggacaccgccttagctacaagttgccaaccaagcgtcagaaattggtggtcatggtgggagaaaagcccattaccataactcagcactcggtagaaaccgaaggctgcattcactcaccttgtcaaggacctgaggatctctgcacccttattaagaccctgtgcggtctcaaagatcttattccctttaactaataaaaaaaaataataaagcatcacttacttaaaatcagttagcaaatttctgtccagtttattcagcagcacctccttgccctcctcccagctctggtattgcagcttcctcctggctgcaaactttctccacaatctaaatggaatgtcagtttcctcctgttcctgtccatccgcacccactatcttcatgttgttgcagatgaagcgcgcaagaccgtctgaagataccttcaaccccgtgtatccatatgacacggaaaccggtcctccaactgtgccttttcttactcctccctttgtatcccccaatgggtttcaagagagtccccctggggtactctctttgcgcctatccgaacctctagttacctccaatggcatgcttgcgctcaaaatgggcaacggcctctctctggacgaggccggcaaccttacctcccaaaatgtaaccactgtgagcccacctctccgaggagacaagtcaaacataaacctggaaatatctgcacccctcacagttacctcagaagccctaactgtggctgccgccgcacctctaatggtcgcgggcaacacactcaccatgcaatcacaggccccgctaaccgtgcacgactccaaacttagcattgccacccaaggacccctcacagtgtcagaaggaaagctagccctgcaaacatcaggccccctcaccaccaccgatagcagtacccttactatcactgcctcaccccctctaactactgccactggtagcttgggcattgacttgaaagagcccatttatacacaaaatggaaaactaggactaaagtacggggctcctttgcatgtaacagacgacctaaacactttgaccgtagcaactggtccaggtgtgactattaataatacttccttgcaaactaaagttactggagccttgggttttgattcacaaggcaatatgcaacttaatgtagcaggaggactaaggattgattctcaaaacagacgccttatacttgatgttagttatccgtttgatgctcaaaaccaactaaatctaagactaggacagggccctctttttataaactcagcccacaacttggatattaactacaacaaaggcctttacttgtttacagcttcaaacaattccaaaaagcttgaggttaacctaagcactgccaaggggttgatgtttgacgctacagccatagccattaatgcaggagatgggcttgaatttggttcacctaatgcaccaaacacaaatcccctcaaaacaaaaattggccatggcctagaatttgattcaaacaaggctatggttcctaaactaggaactggccttagttttgacagcacaggtgccattacagtaggaaacaaaaataatgataagctaactttgtggaccacaccagctccatctcctaactgtagactaaatgcagagaaagatgctaaactcactttggtcttaacaaaatgtggcagtcaaatacttgctacagtttcagttttggctgttaaaggcagtttggctccaatatctggaacagttcaaagtgctcatcttattataagatttgacgaaaatggagtgctactaaacaattccttcctggacccagaatattggaactttagaaatggagatcttactgaaggcacagcctatacaaacgctgttggatttatgcctaacctatcagcttatccaaaatctcacggtaaaactgccaaaagtaacattgtcagtcaagtttacttaaacggagacaaaactaaacctgtaacactaaccattacactaaacggtacacaggaaacaggagacacaactccaagtgcatactctatgtcattttcatgggactggtctggccacaactacattaatgaaatatttgccacatcctcttacactttttcatacattgcccaagaataaagaatcgtttgtgttatgtttcaacgtgtttatttttcaattgcagaaaatttcaagtcatttttcattcagtagtatagccccaccaccacatagcttatacagatcaccgtaccttaatcaaactcacagaaccctagtattcaacctgccacctccctcccaacacacagagtacacagtcctttctccccggctggccttaaaaagcatcatatcatgggtaacagacatattcttaggtgttatattccacacggtttcctgtcgagccaaacgctcatcagtgatattaataaactccccgggcagctcacttaagttcatgtcgctgtccagctgctgagccacaggctgctgtccaacttgcggttgcttaacgggcggcgaaggagaagtccacgcctacatgggggtagagtcataatcgtgcatcaggatagggcggtggtgctgcagcagcgcgcgaataaactgctgccgccgccgctccgtcctgcaggaatacaacatggcagtggtctcctcagcgatgattcgcaccgcccgcagcataaggcgccttgtcctccgggcacagcagcgcaccctgatctcacttaaatcagcacagtaactgcagcacagcaccacaatattgttcaaaatcccacagtgcaaggcgctgtatccaaagctcatggcggggaccacagaacccacgtggccatcataccacaagcgcaggtagattaagtggcgacccctcataaacacgctggacataaacattacctcttttggcatgttgtaattcaccacctcccggtaccatataaacctctgattaaacatggcgccatccaccaccatcctaaaccagctggccaaaacctgcccgccggctatacactgcagggaaccgggactggaacaatgacagtggagagcccaggactcgtaaccatggatcatcatgctcgtcatgatatcaatgttggcacaacacaggcacacgtgcatacacttcctcaggattacaagctcctcccgcgttagaaccatatcccagggaacaacccattcctgaatcagcgtaaatcccacactgcagggaagacctcgcacgtaactcacgttgtgcattgtcaaagtgttacattcgggcagcagcggatgatcctccagtatggtagcgcgggtttctgtctcaaaaggaggtagacgatccctactgtacggagtgcgccgagacaaccgagatcgtgttggtcgtagtgtcatgccaaatggaacgccggacgtagtcatatttcctgaagcaaaaccaggtgcgggcgtgacaaacagatctgcgtctccggtctcgccgcttagatcgctctgtgtagtagttgtagtatatccactctctcaaagcatccaggcgccccctggcttcgggttctatgtaaactccttcatgcgccgctgccctgataacatccaccaccgcagaataagccacacccagccaacctacacattcgttctgcgagtcacacacgggaggagcgggaagagctggaagaaccatgtttttttttttattccaaaagattatccaaaacctcaaaatgaagatctattaagtgaacgcgctcccctccggtggcgtggtcaaactctacagccaaagaacagataatggcatttgtaagatgttgcacaatggcttccaaaaggcaaacggccctcacgtccaagtggacgtaaaggctaaacccttcagggtgaatctcctctataaacattccagcaccttcaaccatgcccaaataattctcatctcgccaccttctcaatatatctctaagcaaatcccgaatattaagtccggccattgtaaaaatctgctccagagcgccctccaccttcagcctcaagcagcgaatcatgattgcaaaaattcaggttcctcacagacctgtataagattcaaaagcggaacattaacaaaaataccgcgatcccgtaggtcccttcgcagggccagctgaacataatcgtgcaggtctgcacggaccagcgcggccacttccccgccaggaaccatgacaaaagaacccacactgattatgacacgcatactcggagctatgctaaccagcgtagccccgatgtaagcttgttgcatgggcggcgatataaaatgcaaggtgctgctcaaaaaatcaggcaaagcctcgcgcaaaaaagaaagcacatcgtagtcatgctcatgcagataaaggcaggtaagctccggaaccaccacagaaaaagacaccatttttctctcaaacatgtctgcgggtttctgcataaacacaaaataaaataacaaaaaaacatttaaacattagaagcctgtcttacaacaggaaaaacaacccttataagcataagacggactacggccatgccggcgtgaccgtaaaaaaactggtcaccgtgattaaaaagcaccaccgacagctcctcggtcatgtccggagtcataatgtaagactcggtaaacacatcaggttgattcacatcggtcagtgctaaaaagcgaccgaaatagcccgggggaatacatacccgcaggcgtagagacaacattacagcccccataggaggtataacaaaattaataggagagaaaaacacataaacacctgaaaaaccctcctgcctaggcaaaatagcaccctcccgctccagaacaacatacagcgcttccacagcggcagccataacagtcagccttaccagtaaaaaagaaaacctattaaaaaaacaccactcgacacggcaccagctcaatcagtcacagtgtaaaaaagggccaagtgcagagcgagtatatataggactaaaaaatgacgtaacggttaaagtccacaaaaaacacccagaaaaccgcacgcgaacctacgcccagaaacgaaagccaaaaaacccacaacttcctcaaatcgtcacttccgttttcccacgttacgtcacttcccattttaagaaaactacaattcccaacacatactagttactccgccctaaaacctacgtcacccgccccgttcccacgccccgcgccacgtcacaaactccaccccctcattatcatattggcttcaatccaaaataaggtatattattgatgatgt

SEQ ID NO: 3 - DNA, 36090 bp, Artificial Sequence
  ICOVIR15K-TD
catcatcaataatataccttattttggattgaagccaatatgataatgagggggtggagtttgtgacgtggcgcggggcgtgggaacggggcgggtgacgtagtagtgtggcggaagtgtgatgttgcaagtgtggcggaacacatgtaagcgacggatgtggcaaaagtgacgtttttggtgtgcgccggtgtacacaggaagtgacaattttcgcgcggttttaggcggatgttgtagtaaatttgggcgtaaccgagtaagatttggccattttcgcgggaaaactgaataagaggaagtgaaatctgaataattttgtgttactcatagcgcgtaatatttgtctagggccgcggggactttgaccgtttacgtggagactcgcccaggtgtttttctcaggtgttttccgcgtacgtcggcggctcgtggctctttcgcggcaaaaaggatttggcgcgtaaaagtggttcgagtacgtcggcggctcgtggctctttcgcggcaaaaaggatttggcgcgtaaaagtggttcgaagtacgtcgaccacaaaccccgcccagcgtcttgtcattggcgtcgacgctgtacggggtcaaagttggcgttttattattatagtcagctgacgtgtagtgtatttatacccggtgagttcctcaagaggccactcttgagtgccagcgagtagagttttctcctccgagccgctccgacaccgggactgaaaatgagacatattatctgccacggaggtgttattaccgaagaaatggccgccagtcttttggaccagctgatcgaagaggtactggctgataatcttccacctcctagccattttgaaccacctacccttcacgaactgtatgatttagacgtgacggcccccgaagatcccaacgaggaggcggtttcgcagatttttcccgactctgtaatgttggcggtgcaggaagggattgacttactcacttttccgccggcgcccggttctccggagccgcctcacctttcccggcagcccgagcagccggagcagagagccttgggtccggtttctatgccaaaccttgtaccggaggtgatcgatccacccagtgacgacgaggatgaagagggtgaggagtttgtgttagattatgtggagcaccccgggcacggttgcaggtcttgtcattatcaccggaggaatacgggggacccagatattatgtgttcgctttgctatatgaggacctgtggcatgtttgtctacagtaagtgaaaattatgggcagtgggtgatagagtggtgggtttggtgtggtaattttttttttaatttttacagttttgtggtttaaagaattttgtattgtgatttttttaaaaggtcctgtgtctgaacctgagcctgagcccgagccagaaccggagcctgcaagacctacccgccgtcctaaaatggcgcctgctatcctgagacgcccgacatcacctgtgtccagagaatgcaatagtagtacggatagctgtgactccggtccttctaacacacctcctgagatacacccggtggtcccgctgtgccccattaaaccagttgccgtgagagttggtgggcgtcgccaggctgtggaatgtatcgaggacttgcttaacgagcctgggcaacctttggacttgagctgtaaacgccccaggccataaggtgtaaacctgtgattgcgtgtgtggttaacgcctttgtttgctgaatgagttgatgtaagtttaataaagggtgagataatgtttaacttgcatggcgtgttaaatggggcggggcttaaagggtatataatgcgccgtgggctaatcttggttacatctgacctcatggaggcttgggagtgtttggaagatttttctgctgtgcgtaacttgctggaacagagctctaacagtacctcttggttttggaggtttctgtggggctcatcccaggcaaagttagtctgcagaattaaggaggattacaagtgggaatttgaagagcttttgaaatcctgtggtgagctgtttgattctttgaatctgggtcaccaggcgcttttccaagagaaggtcatcaagactttggatttttccacaccggggcgcgctgcggctgctgttgcttttttgagttttataaaggataaatggagcgaagaaacccatctgagcggggggtacctgctggattttctggccatgcatctgtggagagcggttgtgagacacaagaatcgcctgctactgttgtcttccgtccgcccggcgataataccgacggaggagcagcagcagcagcaggaggaagccaggcggcggcggcaggagcagagcccatggaacccgagagccggcctggaccctcgggaatgaatgttgtacaggtggctgaactgtatccagaactgagacgcattttgacaattacagaggatgggcaggggctaaagggggtaaagagggagcggggggcttgtgaggctacagaggaggctaggaatctagcttttagcttaatgaccagacaccgtcctgagtgtattacttttcaacagatcaaggataattgcgctaatgagcttgatctgctggcgcagaagtattccatagagcagctgaccacttactggctgcagccaggggatgattttgaggaggctattagggtatatgcaaaggtggcacttaggccagattgcaagtacaagatcagcaaacttgtaaatatcaggaattgttgctacatttctgggaacggggccgaggtggagatagatacggaggatagggtggcctttagatgtagcatgataaatatgtggccgggggtgcttggcatggacggggtggttattatgaatgtaaggtttactggccccaattttagcggtacggttttcctggccaataccaaccttatcctacacggtgtaagcttctatgggtttaacaatacctgtgtggaagcctggaccgatgtaagggttcggggctgtgccttttactgctgctggaagggggtggtgtgtcgccccaaaagcagggcttcaattaagaaatgcctctttgaaaggtgtaccttgggtatcctgtctgagggtaactccagggtgcgccacaatgtggcctccgactgtggttgcttcatgctagtgaaaagcgtggctgtgattaagcataacatggtatgtggcaactgcgaggacagggcctctcagatgctgacctgctcggacggcaactgtcacctgctgaagaccattcacgtagccagccactctcgcaaggcctggccagtgtttgagcataacatactgacccgctgttccttgcatttgggtaacaggaggggggtgttcctaccttaccaatgcaatttgagtcacactaagatattgcttgagcccgagagcatgtccaaggtgaacctgaacggggtgtttgacatgaccatgaagatctggaaggtgctgaggtacgatgagacccgcaccaggtgcagaccctgcgagtgtggcggtaaacatattaggaaccagcctgtgatgctggatgtgaccgaggagctgaggcccgatcacttggtgctggcctgcacccgcgctgagtttggctctagcgatgaagatacagattgaggtactgaaatgtgtgggcgtggcttaagggtgggaaagaatatataaggtgggggtcttatgtagttttgtatctgttttgcagcagccgccgccgccatgagcaccaactcgtttgatggaagcattgtgagctcatatttgacaacgcgcatgcccccatgggccggggtgcgtcagaatgtgatgggctccagcattgatggtcgccccgtcctgcccgcaaactctactaccttgacctacgagaccgtgtctggaacgccgttggagactgcagcctccgccgccgcttcagccgctgcagccaccgcccgcgggattgtgactgactttgctttcctgagcccgcttgcaagcagtgcagcttcccgttcatccgcccgcgatgacaagttgacggctcttttggcacaattggattctttgacccgggaacttaatgtcgtttctcagcagctgttggatctgcgccagcaggtttctgccctgaaggcttcctcccctcccaatgcggtttaaaacataaataaaaaaccagactctgtttggatttggatcaagcaagtgtcttgctgtctttatttaggggttttgcgcgcgcggtaggcccgggaccagcggtctcggtcgttgagggtcctgtgtattttttccaggacgtggtaaaggtgactctggatgttcagatacatgggcataagcccgtctctggggtggaggtagcaccactgcagagcttcatgctgcggggtggtgttgtagatgatccagtcgtagcaggagcgctgggcgtggtgcctaaaaatgtctttcagtagcaagctgattgccaggggcaggcccttggtgtaagtgtttacaaagcggttaagctgggatgggtgcatacgtggggatatgagatgcatcttggactgtatttttaggttggctatgttcccagccatatccctccggggattcatgttgtgcagaaccaccagcacagtgtatccggtgcacttgggaaatttgtcatgtagcttagaaggaaatgcgtggaagaacttggagacgcccttgtgacctccaagattttccatgcattcgtccataatgatggcaatgggcccacgggcggcggcctgggcgaagatatttctgggatcactaacgtcatagttgtgttccaggatgagatcgtcataggccatttttacaaagcgcgggcggagggtgccagactgcggtataatggttccatccggcccaggggcgtagttaccctcacagatttgcatttcccacgctttgagttcagatggggggatcatgtctacctgcggggcgatgaagaaaacggtttccggggtaggggagatcagctgggaagaaagcaggttcctgagcagctgcgacttaccgcagccggtgggcccgtaaatcacacctattaccgggtgcaactggtagttaagagagctgcagctgccgtcatccctgagcaggggggccacttcgttaagcatgtccctgactcgcatgttttccctgaccaaatccgccagaaggcgctcgccgcccagcgatagcagttcttgcaaggaagcaaagtttttcaacggtttgagaccgtccgccgtaggcatgcttttgagcgtttgaccaagcagttccaggcggtcccacagctcggtcacctgctctacggcatctcgatccagcatatctcctcgtttcgcgggttggggcggctttcgctgtacggcagtagtcggtgctcgtccagacgggccagggtcatgtctttccacgggcgcagggtcctcgtcagcgtagtctgggtcacggtgaaggggtgcgctccgggctgcgcgctggccagggtgcgcttgaggctggtcctgctggtgctgaagcgctgccggtcttcgccctgcgcgtcggccaggtagcatttgaccatggtgtcatagtccagcccctccgcggcgtggcccttggcgcgcagcttgcccttggaggaggcgccgcacgaggggcagtgcagacttttgagggcgtagagcttgggcgcgagaaataccgattccggggagtaggcatccgcgccgcaggccccgcagacggtctcgcattccacgagccaggtgagctctggccgttcggggtcaaaaaccaggtttcccccatgctttttgatgcgtttcttacctctggtttccatgagccggtgtccacgctcggtgacgaaaaggctgtccgtgtccccgtatacagacttgagaggcctgtcctcgagcggtgttccgcggtcctcctcgtatagaaactcggaccactctgagacaaaggctcgcgtccaggccagcacgaaggaggctaagtgggaggggtagcggtcgttgtccactagggggtccactcgctccagggtgtgaagacacatgtcgccctcttcggcatcaaggaaggtgattggtttgtaggtgtaggccacgtgaccgggtgttcctgaaggggggctataaaagggggtgggggcgcgttcgtcctcactctcttccgcatcgctgtctgcgagggccagctgttggggtgagtactccctctgaaaagcgggcatgacttctgcgctaagattgtcagtttccaaaaacgaggaggatttgatattcacctggcccgcggtgatgcctttgagggtggccgcatccatctggtcagaaaagacaatctttttgttgtcaagcttggtggcaaacgacccgtagagggcgttggacagcaacttggcgatggagcgcagggtttggtttttgtcgcgatcggcgcgctccttggccgcgatgtttagctgcacgtattcgcgcgcaacgcaccgccattcgggaaagacggtggtgcgctcgtcgggcaccaggtgcacgcgccaaccgcggttgtgcagggtgacaaggtcaacgctggtggctacctctccgcgtaggcgctcgttggtccagcagaggcggccgcccttgcgcgagcagaatggcggtagggggtctagctgcgtctcgtccggggggtctgcgtccacggtaaagaccccgggcagcaggcgcgcgtcgaagtagtctatcttgcatccttgcaagtctagcgcctgctgccatgcgcgggcggcaagcgcgcgctcgtatgggttgagtgggggaccccatggcatggggtgggtgagcgcggaggcgtacatgccgcaaatgtcgtaaacgtagaggggctctctgagtattccaagatatgtagggtagcatcttccaccgcggatgctggcgcgcacgtaatcgtatagttcgtgcgagggagcgaggaggtcgggaccgaggttgctacgggcgggctgctctgctcggaagactatctgcctgaagatggcatgtgagttggatgatatggttggacgctggaagacgttgaagctggcgtctgtgagacctaccgcgtcacgcacgaaggaggcgtaggagtcgcgcagcttgttgaccagctcggcggtgacctgcacgtctagggcgcagtagtccagggtttccttgatgatgtcatacttatcctgtcccttttttttccacagctcgcggttgaggacaaactcttcgcggtctttccagtactcttggatcggaaacccgtcggcctccgaacggtaagagcctagcatgtagaactggttgacggcctggtaggcgcagcatcccttttctacgggtagcgcgtatgcctgcgcggccttccggagcgaggtgtgggtgagcgcaaaggtgtccctgaccatgactttgaggtactggtatttgaagtcagtgtcgtcgcatccgccctgctcccagagcaaaaagtccgtgcgctttttggaacgcggatttggcagggcgaaggtgacatcgttgaagagtatctttcccgcgcgaggcataaagttgcgtgtgatgcggaagggtcccggcacctcggaacggttgttaattacctgggcggcgagcacgatctcgtcaaagccgttgatgttgtggcccacaatgtaaagttccaagaagcgcgggatgcccttgatggaaggcaattttttaagttcctcgtaggtgagctcttcaggggagctgagcccgtgctctgaaagggcccagtctgcaagatgagggttggaagcgacgaatgagctccacaggtcacgggccattagcatttgcaggtggtcgcgaaaggtcctaaactggcgacctatggccattttttctggggtgatgcagtagaaggtaagcgggtcttgttcccagcggtcccatccaaggttcgcggctaggtctcgcgcggcagtcactagaggctcatctccgccgaacttcatgaccagcatgaagggcacgagctgcttcccaaaggcccccatccaagtataggtctctacatcgtaggtgacaaagagacgctcggtgcgaggatgcgagccgatcgggaagaactggatctcccgccaccaattggaggagtggctattgatgtggtgaaagtagaagtccctgcgacgggccgaacactcgtgctggcttttgtaaaaacgtgcgcagtactggcagcggtgcacgggctgtacatcctgcacgaggttgacctgacgaccgcgcacaaggaagcagagtgggaatttgagcccctcgcctggcgggtttggctggtggtcttctacttcggctgcttgtccttgaccgtctggctgctcgaggggagttacggtggatcggaccaccacgccgcgcgagcccaaagtccagatgtccgcgcgcggcggtcggagcttgatgacaacatcgcgcagatgggagctgtccatggtctggagctcccgcggcgtcaggtcaggcgggagctcctgcaggtttacctcgcatagacgggtcagggcgcgggctagatccaggtgatacctaatttccaggggctggttggtggcggcgtcgatggcttgcaagaggccgcatccccgcggcgcgactacggtaccgcgcggcgggcggtgggccgcgggggtgtccttggatgatgcatctaaaagcggtgacgcgggcgagcccccggaggtagggggggctccggacccgccgggagagggggcaggggcacgtcggcgccgcgcgcgggcaggagctggtgctgcgcgcgtaggttgctggcgaacgcgacgacgcggcggttgatctcctgaatctggcgcctctgcgtgaagacgacgggcccggtgagcttgagcctgaaagagagttcgacagaatcaatttcggtgtcgttgacggcggcctggcgcaaaatctcctgcacgtctcctgagttgtcttgataggcgatctcggccatgaactgctcgatctcttcctcctggagatctccgcgtccggctcgctccacggtggcggcgaggtcgttggaaatgcgggccatgagctgcgagaaggcgttgaggcctccctcgttccagacgcggctgtagaccacgcccccttcggcatcgcgggcgcgcatgaccacctgcgcgagattgagctccacgtgccgggcgaagacggcgtagtttcgcaggcgctgaaagaggtagttgagggtggtggcggtgtgttctgccacgaagaagtacataacccagcgtcgcaacgtggattcgttgatatcccccaaggcctcaaggcgctccatggcctcgtagaagtccacggcgaagttgaaaaactgggagttgcgcgccgacacggttaactcctcctccagaagacggatgagctcggcgacagtgtcgcgcacctcgcgctcaaaggctacaggggcctcttcttcttcttcaatctcctcttccataagggcctccccttcttcttcttctggcggcggtgggggaggggggacacggcggcgacgacggcgcaccgggaggcggtcgacaaagcgctcgatcatctccccgcggcgacggcgcatggtctcggtgacggcgcggccgttctcgcgggggcgcagttggaagacgccgcccgtcatgtcccggttatgggttggcggggggctgccatgcggcagggatacggcgctaacgatgcatctcaacaattgttgtgtaggtactccgccgccgagggacctgagcgagtccgcatcgaccggatcggaaaacctctcgagaaaggcgtctaaccagtcacagtcgcaaggtaggctgagcaccgtggcgggcggcagcgggcggcggtcggggttgtttctggcggaggtgctgctgatgatgtaattaaagtaggcggtcttgagacggcggatggtcgacagaagcaccatgtccttgggtccggcctgctgaatgcgcaggcggtcggccatgccccaggcttcgttttgacatcggcgcaggtctttgtagtagtcttgcatgagcctttctaccggcacttcttcttctccttcctcttgtcctgcatctcttgcatctatcgctgcggcggcggcggagtttggccgtaggtggcgccctcttcctcccatgcgtgtgaccccgaagcccctcatcggctgaagcagggctaggtcggcgacaacgcgctcggctaatatggcctgctgcacctgcgtgagggtagactggaagtcatccatgtccacaaagcggtggtatgcgcccgtgttgatggtgtaagtgcagttggccataacggaccagttaacggtctggtgacccggctgcgagagctcggtgtacctgagacgcgagtaagccctcgagtcaaatacgtagtcgttgcaagtccgcaccaggtactggtatcccaccaaaaagtgcggcggcggctggcggtagaggggccagcgtagggtggccggggctccgggggcgagatcttccaacataaggcgatgatatccgtagatgtacctggacatccaggtgatgccggcggcggtggtggaggcgcgcggaaagtcgcggacgcggttccagatgttgcgcagcggcaaaaagtgctccatggtcgggacgctctggccggtcaggcgcgcgcaatcgttgacgctctagaccgtgcaaaaggagagcctgtaagcgggcactcttccgtggtctggtggataaattcgcaagggtatcatggcggacgaccggggttcgagccccgtatccggccgtccgccgtgatccatgcggttaccgcccgcgtgtcgaacccaggtgtgcgacgtcagacaacgggggagtgctccttttggcttccttccaggcgcggcggctgctgcgctagcttttttggccactggccgcgcgcagcgtaagcggttaggctggaaagcgaaagcattaagtggctcgctccctgtagccggagggttattttccaagggttgagtcgcgggacccccggttcgagtctcggaccggccggactgcggcgaacgggggtttgcctccccgtcatgcaagaccccgcttgcaaattcctccggaaacagggacgagccccttttttgcttttcccagatgcatccggtgctgcggcagatgcgcccccctcctcagcagcggcaagagcaagagcagcggcagacatgcagggcaccctcccctcctcctaccgcgtcaggaggggcgacatccgcggttgacgcggcagcagatggtgattacgaacccccgcggcgccgggcccggcactacctggacttggaggagggcgagggcctggcgcggctaggagcgccctctcctgagcggtacccaagggtgcagctgaagcgtgatacgcgtgaggcgtacgtgccgcggcagaacctgtttcgcgaccgcgagggagaggagcccgaggagatgcgggatcgaaagttccacgcagggcgcgagctgcggcatggcctgaatcgcgagcggttgctgcgcgaggaggactttgagcccgacgcgcgaaccgggattagtcccgcgcgcgcacacgtggcggccgccgacctggtaaccgcatacgagcagacggtgaaccaggagattaactttcaaaaaagctttaacaaccacgtgcgtacgcttgtggcgcgcgaggaggtggctataggactgatgcatctgtgggactttgtaagcgcgctggagcaaaacccaaatagcaagccgctcatggcgcagctgttccttatagtgcagcacagcagggacaacgaggcattcagggatgcgctgctaaacatagtagagcccgagggccgctggctgctcgatttgataaacatcctgcagagcatagtggtgcaggagcgcagcttgagcctggctgacaaggtggccgccatcaactattccatgcttagcctgggcaagttttacgcccgcaagatataccataccccttacgttcccatagacaaggaggtaaagatcgaggggttctacatgcgcatggcgctgaaggtgcttaccttgagcgacgacctgggcgtttatcgcaacgagcgcatccacaaggccgtgagcgtgagccggcggcgcgagctcagcgaccgcgagctgatgcacagcctgcaaagggccctggctggcacgggcagcggcgatagagaggccgagtcctactttgacgcgggcgctgacctgcgctgggccccaagccgacgcgccctggaggcagctggggccggacctgggctggcggtggcacccgcgcgcgctggcaacgtcggcggcgtggaggaatatgacgaggacgatgagtacgagccagaggacggcgagtactaagcggtgatgtttctgatcagatgatgcaagacgcaacggacccggcggtgcgggcggcgctgcagagccagccgtccggccttaactccacggacgactggcgccaggtcatggaccgcatcatgtcgctgactgcgcgcaatcctgacgcgttccggcagcagccgcaggccaaccggctctccgcaattctggaagcggtggtcccggcgcgcgcaaaccccacgcacgagaaggtgctggcgatcgtaaacgcgctggccgaaaacagggccatccggcccgacgaggccggcctggtctacgacgcgctgcttcagcgcgtggctcgttacaacagcggcaacgtgcagaccaacctggaccggctggtgggggatgtgcgcgaggccgtggcgcagcgtgagcgcgcgcagcagcagggcaacctgggctccatggttgcactaaacgccttcctgagtacacagcccgccaacgtgccgcggggacaggaggactacaccaactttgtgagcgcactgcggctaatggtgactgagacaccgcaaagtgaggtgtaccagtctgggccagactattttttccagaccagtagacaaggcctgcagaccgtaaacctgagccaggctttcaaaaacttgcaggggctgtggggggtgcgggctcccacaggcgaccgcgcgaccgtgtctagcttgctgacgcccaactcgcgcctgttgctgctgctaatagcgcccttcacggacagtggcagcgtgtcccgggacacatacctaggtcacttgctgacactgtaccgcgaggccataggtcaggcgcatgtggacgagcatactttccaggagattacaagtgtcagccgcgcgctggggcaggaggacacgggcagcctggaggcaaccctaaactacctgctgaccaaccggcggcagaagatcccctcgttgcacagtttaaacagcgaggaggagcgcattttgcgctacgtgcagcagagcgtgagccttaacctgatgcgcgacggggtaacgcccagcgtggcgctggacatgaccgcgcgcaacatggaaccgggcatgtatgcctcaaaccggccgtttatcaaccgcctaatggactacttgcatcgcgcggccgccgtgaaccccgagtatttcaccaatgccatcttgaacccgcactggctaccgccccctggtttctacaccgggggattcgaggtgcccgagggtaacgatggattcctctgggacgacatagacgacagcgtgttttccccgcaaccgcagaccctgctagagttgcaacagcgcgagcaggcagaggcggcgctgcgaaaggaaagcttccgcaggccaagcagcttgtccgatctaggcgctgcggccccgcggtcagatgctagtagcccatttccaagcttgatagggtctcttaccagcactcgcaccacccgcccgcgcctgctgggcgaggaggagtacctaaacaactcgctgctgcagccgcagcgcgaaaaaaacctgcctccggcatttcccaacaacgggatagagagcctagtggacaagatgagtagatggaagacgtacgcgcaggagcacagggacgtgccaggcccgcgcccgcccacccgtcgtcaaaggcacgaccgtcagcggggtctggtgtgggaggacgatgactcggcagacgacagcagcgtcctggatttgggagggagtggcaacccgtttgcgcaccttcgccccaggctggggagaatgttttaaaaaaaaaaaagcatgatgcaaaataaaaaactcaccaaggccatggcaccgagcgttggttttcttgtattccccttagtatgcggcgcgcggcgatgtatgaggaaggtcctcctccctcctacgagagtgtggtgagcgcggcgccagtggcggcggcgctgggttctcccttcgatgctcccctggacccgccgtttgtgcctccgcggtacctgcggcctaccggggggagaaacagcatccgttactctgagttggcacccctattcgacaccacccgtgtgtacctggtggacaacaagtcaacggatgtggcatccctgaactaccagaacgaccacagcaactttctgaccacggtcattcaaaacaatgactacagcccgggggaggcaagcacacagaccatcaatcttgacgaccggtcgcactggggcggcgacctgaaaaccatcctgcataccaacatgccaaatgtgaacgagttcatgtttaccaataagtttaaggcgcgggtgatggtgtcgcgcttgcctactaaggacaatcaggtggagctgaaatacgagtgggtggagttcacgctgcccgagggcaactactccgagaccatgaccatagaccttatgaacaacgcgatcgtggagcactacttgaaagtgggcagacagaacggggttctggaaagcgacatcggggtaaagtttgacacccgcaacttcagactggggtttgaccccgtcactggtcttgtcatgcctggggtatatacaaacgaagccttccatccagacatcattttgctgccaggatgcggggtggacttcacccacagccgcctgagcaacttgttgggcatccgcaagcggcaacccttccaggagggctttaggatcacctacgatgatctggagggtggtaacattcccgcactgttggatgtggacgcctaccaggcgagcttgaaagatgacaccgaacagggcgggggtggcgcaggcggcagcaacagcagtggcagcggcgcggaagagaactccaacgcggcagccgcggcaatgcagccggtggaggacatgaacgatcatgccattcgcggcgacacctttgccacacgggctgaggagaagcgcgctgaggccgaagcagcggccgaagctgccgcccccgctgcgcaacccgaggtcgagaagcctcagaagaaaccggtgatcaaacccctgacagaggacagcaagaaacgcagttacaacctaataagcaatgacagcaccttcacccagtaccgcagctggtaccttgcatacaactacggcgaccctcagaccggaatccgctcatggaccctgctttgcactcctgacgtaacctgcggctcggagcaggtctactggtcgttgccagacatgatgcaagaccccgtgaccttccgctccacgcgccagatcagcaactttccggtggtgggcgccgagctgttgcccgtgcactccaagagcttctacaacgaccaggccgtctactcccaactcatccgccagtttacctctctgacccacgtgttcaatcgctttcccgagaaccagattttggcgcgcccgccagcccccaccatcaccaccgtcagtgaaaacgttcctgctctcacagatcacgggacgctaccgctgcgcaacagcatcggaggagtccagcgagtgaccattactgacgccagacgccgcacctgcccctacgtttacaaggccctgggcatagtctcgccgcgcgtcctatcgagccgcactttttgagcaagcatgtccatccttatatcgcccagcaataacacaggctggggcctgcgcttcccaagcaagatgtttggcggggccaagaagcgctccgaccaacacccagtgcgcgtgcgcgggcactaccgcgcgccctggggcgcgcacaaacgcggccgcactgggcgcaccaccgtcgatgacgccatcgacgcggtggtggaggaggcgcgcaactacacgcccacgccgccaccagtgtccacagtggacgcggccattcagaccgtggtgcgcggagcccggcgctatgctaaaatgaagagacggcggaggcgcgtagcacgtcgccaccgccgccgacccggcactgccgcccaacgcgcggcggcggccctgcttaaccgcgcacgtcgcaccggccgacgggcggccatgcgggccgctcgaaggctggccgcgggtattgtcactgtgccccccaggtccaggcgacgagcggccgccgcagcagccgcggccattagtgctatgactcagggtcgcaggggcaacgtgtattgggtgcgcgactcggttagcggcctgcgcgtgcccgtgcgcacccgccccccgcgcaactagattgcaagaaaaaactacttagactcgtactgttgtatgtatccagcggcggcggcgcgcaacgaagctatgtccaagcgcaaaatcaaagaagagatgctccaggtcatcgcgccggagatctatggccccccgaagaaggaagagcaggattacaagccccgaaagctaaagcgggtcaaaaagaaaaagaaagatgatgatgatgaacttgacgacgaggtggaactgctgcacgctaccgcgcccaggcgacgggtacagtggaaaggtcgacgcgtaaaacgtgttttgcgacccggcaccaccgtagtctttacgcccggtgagcgctccacccgcacctacaagcgcgtgtatgatgaggtgtacggcgacgaggacctgcttgagcaggccaacgagcgcctcggggagtttgcctacggaaagcggcataaggacatgctggcgttgccgctggacgagggcaacccaacacctagcctaaagcccgtaacactgcagcaggtgctgcccgcgcttgcaccgtccgaagaaaagcgcggcctaaagcgcgagtctggtgacttggcacccaccgtgcagctgatggtacccaagcgccagcgactggaagatgtcttggaaaaaatgaccgtggaacctgggctggagcccgaggtccgcgtgcggccaatcaagcaggtggcgccgggactgggcgtgcagaccgtggacgttcagatacccactaccagtagcaccagtattgccaccgccacagagggcatggagacacaaacgtccccggttgcctcagcggtggcggatgccgcggtgcaggcggtcgctgcggccgcgtccaagacctctacggaggtgcaaacggacccgtggatgtttcgcgtttcagccccccggcgcccgcgcggttcgaggaagtacggcgccgccagcgcgctactgcccgaatatgccctacatccttccattgcgcctacccccggctatcgtggctacacctaccgccccagaagacgagcaactacccgacgccgaaccaccactggaacccgccgccgccgtcgccgtcgccagcccgtgctggccccgatttccgtgcgcagggtggctcgcgaaggaggcaggaccctggtgctgccaacagcgcgctaccaccccagcatcgtttaaaagccggtctttgtggttcttgcagatatggccctcacctgccgcctccgtttcccggtgccgggattccgaggaagaatgcaccgtaggaggggcatggccggccacggcctgacgggcggcatgcgtcgtgcgcaccaccggcggcggcgcgcgtcgcaccgtcgcatgcgcggcggtatcctgcccctccttattccactgatcgccgcggcgattggcgccgtgcccggaattgcatccgtggccttgcaggcgcagagacactgattaaaaacaagttgcatgtggaaaaatcaaaataaaaagtctggactctcacgctcgcttggtcctgtaactattttgtagaatggaagacatcaactttgcgtctctggccccgcgacacggctcgcgcccgttcatgggaaactggcaagatatcggcaccagcaatatgagcggtggcgccttcagctggggctcgctgtggagcggcattaaaaatttcggttccaccgttaagaactatggcagcaaggcctggaacagcagcacaggccagatgctgagggataagttgaaagagcaaaatttccaacaaaaggtggtagatggcctggcctctggcattagcggggtggtggacctggccaaccaggcagtgcaaaataagattaacagtaagcttgatccccgccctcccgtagaggagcctccaccggccgtggagacagtgtctccagaggggcgtggcgaaaagcgtccgcgccccgacagggaagaaactctggtgacgcaaatagacgagcctccctcgtacgaggaggcactaaagcaaggcctgcccaccacccgtcccatcgcgcccatggctaccggagtgctgggccagcacacacccgtaacgctggacctgcctccccccgccgacacccagcagaaacctgtgctgccaggcccgaccgccgttgttgtaacccgtcctagccgcgcgtccctgcgccgcgccgccagcggtccgcgatcgttgcggcccgtagccagtggcaactggcaaagcacactgaacagcatcgtgggtctgggggtgcaatccctgaagcgccgacgatgcttctgaatagctaacgtgtcgtatgtgtgtcatgtatgcgtccatgtcgccgccagaggagctgctgagccgccgcgcgcccgctttccaagatggctaccccttcgatgatgccgcagtggtcttacatgcacatctcgggccaggacgcctcggagtacctgagccccgggctggtgcagtttgcccgcgccaccgagacgtacttcagcctgaataacaagtttagaaaccccacggtggcgcctacgcacgacgtgaccacagaccggtcccagcgtttgacgctgcggttcatccctgtggaccgtgaggatactgcgtactcgtacaaggcgcggttcaccctagctgtgggtgataaccgtgtgctggacatggcttccacgtactttgacatccgcggcgtgctggacaggggccctacttttaagccctactctggcactgcctacaacgccctggctcccaagggtgccccaaatccttgcgaatgggatgaagctgctactgctcttgaaataaacctagaagaagaggacgatgacaacgaagacgaagtagacgagcaagctgagcagcaaaaaactcacgtatttgggcaggcgccttattctggtataaatattacaaaggagggtattcaaataggtgtcgaaggtcaaacacctaaatatgccgataaaacatttcaacctgaacctcaaataggagaatctcagtggtacgaaactgaaattaatcatgcagctgggagagtccttaaaaagactaccccaatgaaaccatgttacggttcatatgcaaaacccacaaatgaaaatggagggcaaggcattcttgtaaagcaacaaaatggaaagctagaaagtcaagtggaaatgcaatttttctcaactactgaggcgaccgcaggcaatggtgataacttgactcctaaagtggtattgtacagtgaagatgtagatatagaaaccccagacactcatatttcttacatgcccactattaaggaaggtaactcacgagaactaatgggccaacaatctatgcccaacaggcctaattacattgcttttagggacaattttattggtctaatgtattacaacagcacgggtaatatgggtgttctggcgggccaagcatcgcagttgaatgctgttgtagatttgcaagacagaaacacagagctttcataccagcttttgcttgattccattggtgatagaaccaggtacttttctatgtggaatcaggctgttgacagctatgatccagatgttagaattattgaaaatcatggaactgaagatgaacttccaaattactgctttccactgggaggtgtgattaatacagagactcttaccaaggtaaaacctaaaacaggtcaggaaaatggatgggaaaaagatgctacagaattttcagataaaaatgaaataagagttggaaataattttgccatggaaatcaatctaaatgccaacctgtggagaaatttcctgtactccaacatagcgctgtatttgcccgacaagctaaagtacagtccttccaacgtaaaaatttctgataacccaaacacctacgactacatgaacaagcgagtggtggctcccgggttagtggactgctacattaaccttggagcacgctggtcccttgactatatggacaacgtcaacccatttaaccaccaccgcaatgctggcctgcgctaccgctcaatgttgctgggcaatggtcgctatgtgcccttccacatccaggtgcctcagaagttctttgccattaaaaacctccttctcctgccgggctcatacacctacgagtggaacttcaggaaggatgttaacatggttctgcagagctccctaggaaatgacctaagggttgacggagccagcattaagtttgatagcatttgcctttacgccaccttcttccccatggcccacaacaccgcctccacgcttgaggccatgcttagaaacgacaccaacgaccagtcctttaacgactatctctccgccgccaacatgctctaccctatacccgccaacgctaccaacgtgcccatatccatcccctcccgcaactgggcggctttccgcggctgggccttcacgcgccttaagactaaggaaaccccatcactgggctcgggctacgacccttattacacctactctggctctataccctacctagatggaaccttttacctcaaccacacctttaagaaggctgccattacctttgactcttctgtcagctggcctggcaatgaccgcctgcttacccccaacgagtttgaaattaagcgctcagttgacggggagggttacaacgttgcccagtgtaacatgaccaaagactggttcctggtacaaatgctagctaactataacattggctaccagggcttctatatcccagagagctacaaggaccgcatgtactccttctttagaaacttccagcccatgagccgtcaggtggtggatgatactaaatacaaggactaccaacaggtgggcatcctacaccaacacaacaactctggatttgttggctaccttgcccccaccatgcgcgaaggacaggcctaccctgctaacttcccctatccgcttataggcaagaccgcagttgacagcattacccagaaaaagtttctttgcgatcgcaccctttggcgcatcccattctccagtaactttatgtccatgggcgcactcacagacctgggccaaaaccttctctacgccaactccgcccactccctagacatgacttttgaggtggatcccatggacgagcccacccttctttatgttttgtttgaagtctttgacaaggtccgtgtgcaccagccgcaccgcggcgtcatcgaaaccgtgtacctgcgcacgcccttctcggccggcaacgccacaacataaagaagcaagcaacatcaacaacagctgccgccatgggctccagtgagcaggaactgaaagccattgtcaaagatcttggttgtgggccatattttttgggcacctatgacaagcgctttccaggctttgtttctccacacaagctcgcctgcgccatagtcaatacggccggtcgcgagactgggggcgtacactggatggcctttgcctggaacccgcactcaaaaacatgctacctctttgagccctttggcttttctgaccagcgactcaagcaggtttaccagtttgagtacgagtcactcctgcgccgtagcgccattgcttcttcccccgaccgctgtataacgctggaaaagtccacccaaagcgtacaggggcccaactcggccgcctgtggactattctgctgcatgtttctccacgcctttgccaactggccccaaactcccatggatcacaaccccaccatgaaccttattaccggggtacccaactccatgctcaacagtccccaggtacagcccaccctgcgtcgcaaccaggaacagctctacagcttcctggagcgccactcgccctacttccgcagccacagtgcgcagattaggagcgccacttctttttgtcacttgaaaaacatgtaaaaataatgtactagagacactttcaataaaggcaaatgcttttatttgtacactctcgggtgattatttacccccacccttgccgtctgcgccgtttaaaaatcaaaggggttctgccgcgcatcgctatgcgccactggcagggacacgttgcgatactggtgtttagtgctccacttaaactcaggcacaaccatccgcggcagctcggtgaagttttcactccacaggctgcgcaccatcaccaacgcgtttagcaggtcgggcgccgatatcttgaagtcgcagttggggcctccgccctgcgcgcgcgagttgcgatacacagggttgcagcactggaacactatcagcgccgggtggtgcacgctggccagcacgctcttgtcggagatcagatccgcgtccaggtcctccgcgttgctcagggcgaacggagtcaactttggtagctgccttcccaaaaagggcgcgtgcccaggctttgagttgcactcgcaccgtagtggcatcaaaaggtgaccgtgcccggtctgggcgttaggatacagcgcctgcataaaagccttgatctgcttaaaagccacctgagcctttgcgccttcagagaagaacatgccgcaagacttgccggaaaactgattggccggacaggccgcgtcgtgcacgcagcaccttgcgtcggtgttggagatctgcaccacatttcggccccaccggttcttcacgatcttggccttgctagactgctccttcagcgcgcgctgcccgttttcgctcgtcacatccatttcaatcacgtgctccttatttatcataatgcttccgtgtagacacttaagctcgccttcgatctcagcgcagcggtgcagccacaacgcgcagcccgtgggctcgtgatgcttgtaggtcacctctgcaaacgactgcaggtacgcctgcaggaatcgccccatcatcgtcacaaaggtcttgttgctggtgaaggtcagctgcaacccgcggtgctcctcgttcagccaggtcttgcatacggccgccagagcttccacttggtcaggcagtagtttgaagttcgcctttagatcgttatccacgtggtacttgtccatcagcgcgcgcgcagcctccatgcccttctcccacgcagacacgatcggcacactcagcgggttcatcaccgtaatttcactttccgcttcgctgggctcttcctcttcctcttgcgtccgcataccacgcgccactgggtcgtcttcattcagccgccgcactgtgcgcttacctcctttgccatgcttgattagcaccggtgggttgctgaaacccaccatttgtagcgccacatcttctctttcttcctcgctgtccacgattacctctggtgatggcgggcgctcgggcttgggagaagggcgcttctttttcttcttgggcgcaatggccaaatccgccgccgaggtcgatggccgcgggctgggtgtgcgcggcaccagcgcgtcttgtgatgagtcttcctcgtcctcggactcgatacgccgcctcatccgcttttttgggggcgcccggggaggcggcggcgacggggacggggacgacacgtcctccatggttgggggacgtcgcgccgcaccgcgtccgcgctcgggggtggtttcgcgctgctcctcttcccgactggccatttccttctcctataggcagaaaaagatcatggagtcagtcgagaagaaggacagcctaaccgccccctctgagttcgccaccaccgcctccaccgatgccgccaacgcgcctaccaccttccccgtcgaggcacccccgcttgaggaggaggaagtgattatcgagcaggacccaggttttgtaagcgaagacgacgaggaccgctcagtaccaacagaggataaaaagcaagaccaggacaacgcagaggcaaacgaggaacaagtcgggcggggggacgaaaggcatggcgactacctagatgtgggagacgacgtgctgttgaagcatctgcagcgccagtgcgccattatctgcgacgcgttgcaagagcgcagcgatgtgcccctcgccatagcggatgtcagccttgcctacgaacgccacctattctcaccgcgcgtaccccccaaacgccaagaaaacggcacatgcgagcccaacccgcgcctcaacttctaccccgtatttgccgtgccagaggtgcttgccacctatcacatctttttccaaaactgcaagatacccctatcctgccgtgccaaccgcagccgagcggacaagcagctggccttgcggcagggcgctgtcatacctgatatcgcctcgctcaacgaagtgccaaaaatctttgagggtcttggacgcgacgagaagcgcgcggcaaacgctctgcaacaggaaaacagcgaaaatgaaagtcactctggagtgttggtggaactcgagggtgacaacgcgcgcctagccgtactaaaacgcagcatcgaggtcacccactttgcctacccggcacttaacctaccccccaaggtcatgagcacagtcatgagtgagctgatcgtgcgccgtgcgcagcccctggagagggatgcaaatttgcaagaacaaacagaggagggcctacccgcagttggcgacgagcagctagcgcgctggcttcaaacgcgcgagcctgccgacttggaggagcgacgcaaactaatgatggccgcagtgctcgttaccgtggagcttgagtgcatgcagcggttctttgctgacccggagatgcagcgcaagctagaggaaacattgcactacacctttcgacagggctacgtacgccaggcctgcaagatctccaacgtggagctctgcaacctggtctcctaccttggaattttgcacgaaaaccgccttgggcaaaacgtgcttcattccacgctcaagggcgaggcgcgccgcgactacgtccgcgactgcgtttacttatttctatgctacacctggcagacggccatgggcgtttggcagcagtgcttggaggagtgcaacctcaaggagctgcagaaactgctaaagcaaaacttgaaggacctatggacggccttcaacgagcgctccgtggccgcgcacctggcggacatcattttccccgaacgcctgcttaaaaccctgcaacagggtctgccagacttcaccagtcaaagcatgttgcagaactttaggaactttatcctagagcgctcaggaatcttgcccgccacctgctgtgcacttcctagcgactttgtgcccattaagtaccgcgaatgccctccgccgctttggggccactgctaccttctgcagctagccaactaccttgcctaccactctgacataatggaagacgtgagcggtgacggtctactggagtgtcactgtcgctgcaacctatgcaccccgcaccgctccctggtttgcaattcgcagctgcttaacgaaagtcaaattatcggtacctttgagctgcagggtccctcgcctgacgaaaagtccgcggctccggggttgaaactcactccggggctgtggacgtcggcttaccttcgcaaatttgtacctgaggactaccacgcccacgagattaggttctacgaagaccaatcccgcccgccaaatgcggagcttaccgcctgcgtcattacccagggccacattcttggccaattgcaagccatcaacaaagcccgccaagagtttctgctacgaaagggacggggggtttacttggacccccagtccggcgaggagctcaacccaatccccccgccgccgcagccctatcagcagcagccgcgggcccttgcttcccaggatggcacccaaaaagaagctgcagctgccgccgccacccacggacgaggaggaatactgggacagtcaggcagaggaggttttggacgaggaggaggaggacatgatggaagactgggagagcctagacgaggaagcttccgaggtcgaagaggtgtcagacgaaacaccgtcaccctcggtcgcattcccctcgccggcgccccagaaatcggcaaccggttccagcatggctacaacctccgctcctcaggcgccgccggcactgcccgttcgccgacccaaccgtagatgggacaccactggaaccagggccggtaagtccaagcagccgccgccgttagcccaagagcaacaacagcgccaaggctaccgctcatggcgcgggcacaagaacgccatagttgcttgcttgcaagactgtgggggcaacatctccttcgcccgccgctttcttctctaccatcacggcgtggccttcccccgtaacatcctgcattactaccgtcatctctacagcccatactgcaccggcggcagcggcagcggcagcaacagcagcggccacacagaagcaaaggcgaccggatagcaagactctgacaaagcccaagaaatccacagcggcggcagcagcaggaggaggagcgctgcgtctggcgcccaacgaacccgtatcgacccgcgagcttagaaacaggatttttcccactctgtatgctatatttcaacagagcaggggccaagaacaagagctgaaaataaaaaacaggtctctgcgatccctcacccgcagctgcctgtatcacaaaagcgaagatcagcttcggcgcacgctggaagacgcggaggctctcttcagtaaatactgcgcgctgactcttaaggactagtttcgcgccctttctcaaatttaagcgcgaaaactacgtcatctccagcggccacacccggcgccagcacctgtcgtcagcgccattatgagcaaggaaattcccacgccctacatgtggagttaccagccacaaatgggacttgcggctggagctgcccaagactactcaacccgaataaactacatgagcgcgggaccccacatgatatcccgggtcaacggaatccgcgcccaccgaaaccgaattctcttggaacaggcggctattaccaccacacctcgtaataaccttaatccccgtagttggcccgctgccctggtgtaccaggaaagtcccgctcccaccactgtggtacttcccagagacgcccaggccgaagttcagatgactaactcaggggcgcagcttgcgggcggctttcgtcacagggtgcggtcgcccgggcagggtataactcacctgacaatcagagggcgaggtattcagctcaacgacgagtcggtgagctcctcgcttggtctccgtccggacgggacatttcagatcggcggcgccggccgtccttcattcacgcctcgtcaggcaatcctaactctgcagacctcgtcctctgagccgcgctctggaggcattggaactctgcaatttattgaggagtttgtgccatcggtctactttaaccccttctcgggacctcccggccactatccggatcaatttattcctaactttgacgcggtaaaggactcggcggacggctacgactgaatgttaagtggagaggcagagcaactgcgcctgaaacacctggtccactgtcgccgccacaagtgctttgcccgcgactccggtgagttttgctactttgaattgcccgaggatcatatcgagggcccggcgcacggcgtccggcttaccgcccagggagagcttgcccgtagcctgattcgggagtttacccagcgccccctgctagttgagcgggacaggggaccctgtgttctcactgtgatttgcaactgtcctaaccttggattacatcaagatctttgttgccatctctgtgctgagtataataaatacagaaattaaaatatactggggctcctatcgccatcctgtaaacgccaccgtcttcacccgcccaagcaaaccaaggcgaaccttacctggtacttttaacatctctccctctgtgatttacaacagtttcaacccagacggagtgagtctacgagagaacctctccgagctcagctactccatcagaaaaaacaccaccctccttacctgccgggaacgtacgagtgcgtcaccggccgctgcaccacacctaccgcctgaccgtaaaccagactttttccggacagacctcaataactctgtttaccagaacaggaggtgagcttagaaaacccttagggtattaggccaaaggcgcagctactgtggggtttatgaacaattcaagcaactctacgggctattctaattcaggtttctctagaatcggggttggggttattctctgtcttgtgattctctttattcttatactaacgcttctctgcctaaggctcgccgcctgctgtgtgcacatttgcatttattgtcagctttttaaacgctggggtcgccacccaagatgattaggtacataatcctaggtttactcacccttgcgtcagcccacggtaccacccaaaaggtggattttaaggagccagcctgtaatgttacattcgcagctgaagctaatgagtgcaccactcttataaaatgcaccacagaacatgaaaagctgcttattcgccacaaaaacaaaattggcaagtatgctgtttatgctatttggcagccaggtgacactacagagtataatgttacagttttccagggtaaaagtcataaaacttttatgtatacttttccattttatgaaatgtgcgacattaccatgtacatgagcaaacagtataagttgtggcccccacaaaattgtgtggaaaacactggcactttctgctgcactgctatgctaattacagtgctcgctttggtctgtaccctactctatattaaatacaaaagcagacgcagctttattgaggaaaagaaaatgccttaatttactaagttacaaagctaatgtcaccactaactgctttactcgctgcttgcaaaacaaattcaaaaagttagcattataattagaataggatttaaaccccccggtcatttcctgctcaataccattcccctgaacaattgactctatgtgggatatgctccagcgctacaaccttgaagtcaggcttcctggatgtcagcatctgactttggccagcacctgtcccgcggatttgttccagtccaactacagcgacccaccctaacagagatgaccaacacaaccaacgcggccgccgctaccggacttacatctaccacaaatacaccccaagtttctgcctttgtcaataactgggataacttgggcatgtggtggttctccatagcgcttatgtttgtatgccttattattatgtggctcatctgctgcctaaagcgcaaacgcgcccgaccacccatctatagtcccatcattgtgctacacccaaacaatgatggaatccatagattggacggactgaaacacatgttcttttctcttacagtatgattaaatgagacatgattcctcgagtttttatattactgacccttgttgcgcttttttgtgcgtgctccacattggctgcggtttctcacatcgaagtagactgcattccagccttcacagtctatttgctttacggatttgtcaccctcacgctcatctgcagcctcatcactgtggtcatcgcctttatccagtgcattgactgggtctgtgtgcgctttgcatatctcagacaccatccccagtacagggacaggactatagctgagcttcttagaattctttaattatgaaatttactgtgacttttctgctgattatttgcaccctatctgcgttttgttccccgacctccaagcctcaaagacatatatcatgcagattcactcgtatatggaatattccaagttgctacaatgaaaaaagcgatctttccgaagcctggttatatgcaatcatctctgttatggtgttctgcagtaccatcttagccctagctatatatccctaccttgacattggctggaaacgaatagatgccatgaaccacccaactttccccgcgcccgctatgcttccactgcaacaagttgttgccggcggctttgtcccagccaatcagcctcgccccacttctcccacccccactgaaatcagctactttaatctaacaggaggagatgactgacaccctagatctagaaatggacggaattattacagagcagcgcctgctagaaagacgcagggcagcggccgagcaacagcgcatgaatcaagagctccaagacatggttaacttgcaccagtgcaaaaggggtatcttttgtctggtaaagcaggccaaagtcacctacgacagtaataccaccggacaccgccttagctacaagttgccaaccaagcgtcagaaattggtggtcatggtgggagaaaagcccattaccataactcagcactcggtagaaaccgaaggctgcattcactcaccttgtcaaggacctgaggatctctgcacccttattaagaccctgtgcggtctcaaagatcttattccctttaactaataaaaaaaaataataaagcatcacttacttaaaatcagttagcaaatttctgtccagtttattcagcagcacctccttgccctcctcccagctctggtattgcagcttcctcctggctgcaaactttctccacaatctaaatggaatgtcagtttcctcctgttcctgtccatccgcacccactatcttcatgttgttgcagatgaagcgcgcaagaccgtctgaagataccttcaaccccgtgtatccatatgacacggaaaccggtcctccaactgtgccttttcttactcctccctttgtatcccccaatgggtttcaagagagtccccctggggtactctctttgcgcctatccgaacctctagttacctccaatggcatgcttgcgctcaaaatgggcaacggcctctctctggacgaggccggcaaccttacctcccaaaatgtaaccactgtgagcccacctctccgaggagacaagtcaaacataaacctggaaatatctgcacccctcacagttacctcagaagccctaactgtggctgccgccgcacctctaatggtcgcgggcaacacactcaccatgcaatcacaggccccgctaaccgtgcacgactccaaacttagcattgccacccaaggacccctcacagtgtcagaaggaaagctagccctgcaaacatcaggccccctcaccaccaccgatagcagtacccttactatcactgcctcaccccctctaactactgccactggtagcttgggcattgacttgaaagagcccatttatacacaaaatggaaaactaggactaaagtacggggctcctttgcatgtaacagacgacctaaacactttgaccgtagcaactggtccaggtgtgactattaataatacttccttgcaaactaaagttactggagccttgggttttgattcacaaggcaatatgcaacttaatgtagcaggaggactaaggattgattctcaaaacagacgccttatacttgatgttagttatccgtttgatgctcaaaaccaactaaatctaagactaggacagggccctctttttataaactcagcccacaacttggatattaactacaacaaaggcctttacttgtttacagcttcaaacaattccaaaaagcttgaggttaacctaagcactgccaaggggttgatgtttgacgctacagccatagccattaatgcaggagatgggcttgaatttggttcacctaatgcaccaaacacaaatcccctcaaaacaaaaattggccatggcctagaatttgattcaaacaaggctatggttcctaaactaggaactggccttagttttgacagcacaggtgccattacagtaggaaacaaaaataatgataagctaactttgtggaccacaccagctccatctcctaactgtagactaaatgcagagaaagatgctaaactcactttggtcttaacaaaatgtggcagtcaaatacttgctacagtttcagttttggctgttaaaggcagtttggctccaatatctggaacagttcaaagtgctcatcttattataagatttgacgaaaatggagtgctactaaacaattccttcctggacccagaatattggaactttagaaatggagatcttactgaaggcacagcctatacaaacgctgttggatttatgcctaacctatcagcttatccaaaatctcacggtaaaactgccaaaagtaacattgtcagtcaagtttacttaaacggagacaaaactaaacctgtaacactaaccattacactaaacggtacacaggaaacaggagacacaactccaagtgcatactctatgtcattttcatgggactggtctggccacaactacattaatgaaatatttgccacatcctcttacactttttcatacattgcccaagaataaagaatcgtttgtgttatgtttcaacgtgtttatttttcaattgcagaaaatttcaagtcatttttcattcagtagtatagccccaccaccacatagcttatacagatcaccgtaccttaatcaaactcacagaaccctagtattcaacctgccacctccctcccaacacacagagtacacagtcctttctccccggctggccttaaaaagcatcatatcatgggtaacagacatattcttaggtgttatattccacacggtttcctgtcgagccaaacgctcatcagtgatattaataaactccccgggcagctcacttaagttcatgtcgctgtccagctgctgagccacaggctgctgtccaacttgcggttgcttaacgggcggcgaaggagaagtccacgcctacatgggggtagagtcataatcgtgcatcaggatagggcggtggtgctgcagcagcgcgcgaataaactgctgccgccgccgctccgtcctgcaggaatacaacatggcagtggtctcctcagcgatgattcgcaccgcccgcagcataaggcgccttgtcctccgggcacagcagcgcaccctgatctcacttaaatcagcacagtaactgcagcacagcaccacaatattgttcaaaatcccacagtgcaaggcgctgtatccaaagctcatggcggggaccacagaacccacgtggccatcataccacaagcgcaggtagattaagtggcgacccctcataaacacgctggacataaacattacctcttttggcatgttgtaattcaccacctcccggtaccatataaacctctgattaaacatggcgccatccaccaccatcctaaaccagctggccaaaacctgcccgccggctatacactgcagggaaccgggactggaacaatgacagtggagagcccaggactcgtaaccatggatcatcatgctcgtcatgatatcaatgttggcacaacacaggcacacgtgcatacacttcctcaggattacaagctcctcccgcgttagaaccatatcccagggaacaacccattcctgaatcagcgtaaatcccacactgcagggaagacctcgcacgtaactcacgttgtgcattgtcaaagtgttacattcgggcagcagcggatgatcctccagtatggtagcgcgggtttctgtctcaaaaggaggtagacgatccctactgtacggagtgcgccgagacaaccgagatcgtgttggtcgtagtgtcatgccaaatggaacgccggacgtagtcatatttcctgaagcaaaaccaggtgcgggcgtgacaaacagatctgcgtctccggtctcgccgcttagatcgctctgtgtagtagttgtagtatatccactctctcaaagcatccaggcgccccctggcttcgggttctatgtaaactccttcatgcgccgctgccctgataacatccaccaccgcagaataagccacacccagccaacctacacattcgttctgcgagtcacacacgggaggagcgggaagagctggaagaaccatgtttttttttttattccaaaagattatccaaaacctcaaaatgaagatctattaagtgaacgcgctcccctccggtggcgtggtcaaactctacagccaaagaacagataatggcatttgtaagatgttgcacaatggcttccaaaaggcaaacggccctcacgtccaagtggacgtaaaggctaaacccttcagggtgaatctcctctataaacattccagcaccttcaaccatgcccaaataattctcatctcgccaccttctcaatatatctctaagcaaatcccgaatattaagtccggccattgtaaaaatctgctccagagcgccctccaccttcagcctcaagcagcgaatcatgattgcaaaaattcaggttcctcacagacctgtataagattcaaaagcggaacattaacaaaaataccgcgatcccgtaggtcccttcgcagggccagctgaacataatcgtgcaggtctgcacggaccagcgcggccacttccccgccaggaaccatgacaaaagaacccacactgattatgacacgcatactcggagctatgctaaccagcgtagccccgatgtaagcttgttgcatgggcggcgatataaaatgcaaggtgctgctcaaaaaatcaggcaaagcctcgcgcaaaaaagaaagcacatcgtagtcatgctcatgcagataaaggcaggtaagctccggaaccaccacagaaaaagacaccatttttctctcaaacatgtctgcgggtttctgcataaacacaaaataaaataacaaaaaaacatttaaacattagaagcctgtcttacaacaggaaaaacaacccttataagcataagacggactacggccatgccggcgtgaccgtaaaaaaactggtcaccgtgattaaaaagcaccaccgacagctcctcggtcatgtccggagtcataatgtaagactcggtaaacacatcaggttgattcacatcggtcagtgctaaaaagcgaccgaaatagcccgggggaatacatacccgcaggcgtagagacaacattacagcccccataggaggtataacaaaattaataggagagaaaaacacataaacacctgaaaaaccctcctgcctaggcaaaatagcaccctcccgctccagaacaacatacagcgcttccacagcggcagccataacagtcagccttaccagtaaaaaagaaaacctattaaaaaaacaccactcgacacggcaccagctcaatcagtcacagtgtaaaaaagggccaagtgcagagcgagtatatataggactaaaaaatgacgtaacggttaaagtccacaaaaaacacccagaaaaccgcacgcgaacctacgcccagaaacgaaagccaaaaaacccacaacttcctcaaatcgtcacttccgttttcccacgttacgtcacttcccattttaagaaaactacaattcccaacacatactagttactccgccctaaaacctacgtcacccgccccgttcccacgccccgcgccacgtcacaaactccaccccctcattatcatattggcttcaatccaaaataaggtatattattgatgatgt

SEQ ID NO: 4 - DNA, 36156 bp, Artificial Sequence
  ICOVIR15K-TD-gp100-tyr
catcatcaataatataccttattttggattgaagccaatatgataatgagggggtggagtttgtgacgtggcgcggggcgtgggaacggggcgggtgacgtagtagtgtggcggaagtgtgatgttgcaagtgtggcggaacacatgtaagcgacggatgtggcaaaagtgacgtttttggtgtgcgccggtgtacacaggaagtgacaattttcgcgcggttttaggcggatgttgtagtaaatttgggcgtaaccgagtaagatttggccattttcgcgggaaaactgaataagaggaagtgaaatctgaataattttgtgttactcatagcgcgtaatatttgtctagggccgcggggactttgaccgtttacgtggagactcgcccaggtgtttttctcaggtgttttccgcgtacgtcggcggctcgtggctctttcgcggcaaaaaggatttggcgcgtaaaagtggttcgagtacgtcggcggctcgtggctctttcgcggcaaaaaggatttggcgcgtaaaagtggttcgaagtacgtcgaccacaaaccccgcccagcgtcttgtcattggcgtcgacgctgtacggggtcaaagttggcgttttattattatagtcagctgacgtgtagtgtatttatacccggtgagttcctcaagaggccactcttgagtgccagcgagtagagttttctcctccgagccgctccgacaccgggactgaaaatgagacatattatctgccacggaggtgttattaccgaagaaatggccgccagtcttttggaccagctgatcgaagaggtactggctgataatcttccacctcctagccattttgaaccacctacccttcacgaactgtatgatttagacgtgacggcccccgaagatcccaacgaggaggcggtttcgcagatttttcccgactctgtaatgttggcggtgcaggaagggattgacttactcacttttccgccggcgcccggttctccggagccgcctcacctttcccggcagcccgagcagccggagcagagagccttgggtccggtttctatgccaaaccttgtaccggaggtgatcgatccacccagtgacgacgaggatgaagagggtgaggagtttgtgttagattatgtggagcaccccgggcacggttgcaggtcttgtcattatcaccggaggaatacgggggacccagatattatgtgttcgctttgctatatgaggacctgtggcatgtttgtctacagtaagtgaaaattatgggcagtgggtgatagagtggtgggtttggtgtggtaattttttttttaatttttacagttttgtggtttaaagaattttgtattgtgatttttttaaaaggtcctgtgtctgaacctgagcctgagcccgagccagaaccggagcctgcaagacctacccgccgtcctaaaatggcgcctgctatcctgagacgcccgacatcacctgtgtccagagaatgcaatagtagtacggatagctgtgactccggtccttctaacacacctcctgagatacacccggtggtcccgctgtgccccattaaaccagttgccgtgagagttggtgggcgtcgccaggctgtggaatgtatcgaggacttgcttaacgagcctgggcaacctttggacttgagctgtaaacgccccaggccataaggtgtaaacctgtgattgcgtgtgtggttaacgcctttgtttgctgaatgagttgatgtaagtttaataaagggtgagataatgtttaacttgcatggcgtgttaaatggggcggggcttaaagggtatataatgcgccgtgggctaatcttggttacatctgacctcatggaggcttgggagtgtttggaagatttttctgctgtgcgtaacttgctggaacagagctctaacagtacctcttggttttggaggtttctgtggggctcatcccaggcaaagttagtctgcagaattaaggaggattacaagtgggaatttgaagagcttttgaaatcctgtggtgagctgtttgattctttgaatctgggtcaccaggcgcttttccaagagaaggtcatcaagactttggatttttccacaccggggcgcgctgcggctgctgttgcttttttgagttttataaaggataaatggagcgaagaaacccatctgagcggggggtacctgctggattttctggccatgcatctgtggagagcggttgtgagacacaagaatcgcctgctactgttgtcttccgtccgcccggcgataataccgacggaggagcagcagcagcagcaggaggaagccaggcggcggcggcaggagcagagcccatggaacccgagagccggcctggaccctcgggaatgaatgttgtacaggtggctgaactgtatccagaactgagacgcattttgacaattacagaggatgggcaggggctaaagggggtaaagagggagcggggggcttgtgaggctacagaggaggctaggaatctagcttttagcttaatgaccagacaccgtcctgagtgtattacttttcaacagatcaaggataattgcgctaatgagcttgatctgctggcgcagaagtattccatagagcagctgaccacttactggctgcagccaggggatgattttgaggaggctattagggtatatgcaaaggtggcacttaggccagattgcaagtacaagatcagcaaacttgtaaatatcaggaattgttgctacatttctgggaacggggccgaggtggagatagatacggaggatagggtggcctttagatgtagcatgataaatatgtggccgggggtgcttggcatggacggggtggttattatgaatgtaaggtttactggccccaattttagcggtacggttttcctggccaataccaaccttatcctacacggtgtaagcttctatgggtttaacaatacctgtgtggaagcctggaccgatgtaagggttcggggctgtgccttttactgctgctggaagggggtggtgtgtcgccccaaaagcagggcttcaattaagaaatgcctctttgaaaggtgtaccttgggtatcctgtctgagggtaactccagggtgcgccacaatgtggcctccgactgtggttgcttcatgctagtgaaaagcgtggctgtgattaagcataacatggtatgtggcaactgcgaggacagggcctctcagatgctgacctgctcggacggcaactgtcacctgctgaagaccattcacgtagccagccactctcgcaaggcctggccagtgtttgagcataacatactgacccgctgttccttgcatttgggtaacaggaggggggtgttcctaccttaccaatgcaatttgagtcacactaagatattgcttgagcccgagagcatgtccaaggtgaacctgaacggggtgtttgacatgaccatgaagatctggaaggtgctgaggtacgatgagacccgcaccaggtgcagaccctgcgagtgtggcggtaaacatattaggaaccagcctgtgatgctggatgtgaccgaggagctgaggcccgatcacttggtgctggcctgcacccgcgctgagtttggctctagcgatgaagatacagattgaggtactgaaatgtgtgggcgtggcttaagggtgggaaagaatatataaggtgggggtcttatgtagttttgtatctgttttgcagcagccgccgccgccatgagcaccaactcgtttgatggaagcattgtgagctcatatttgacaacgcgcatgcccccatgggccggggtgcgtcagaatgtgatgggctccagcattgatggtcgccccgtcctgcccgcaaactctactaccttgacctacgagaccgtgtctggaacgccgttggagactgcagcctccgccgccgcttcagccgctgcagccaccgcccgcgggattgtgactgactttgctttcctgagcccgcttgcaagcagtgcagcttcccgttcatccgcccgcgatgacaagttgacggctcttttggcacaattggattctttgacccgggaacttaatgtcgtttctcagcagctgttggatctgcgccagcaggtttctgccctgaaggcttcctcccctcccaatgcggtttaaaacataaataaaaaaccagactctgtttggatttggatcaagcaagtgtcttgctgtctttatttaggggttttgcgcgcgcggtaggcccgggaccagcggtctcggtcgttgagggtcctgtgtattttttccaggacgtggtaaaggtgactctggatgttcagatacatgggcataagcccgtctctggggtggaggtagcaccactgcagagcttcatgctgcggggtggtgttgtagatgatccagtcgtagcaggagcgctgggcgtggtgcctaaaaatgtctttcagtagcaagctgattgccaggggcaggcccttggtgtaagtgtttacaaagcggttaagctgggatgggtgcatacgtggggatatgagatgcatcttggactgtatttttaggttggctatgttcccagccatatccctccggggattcatgttgtgcagaaccaccagcacagtgtatccggtgcacttgggaaatttgtcatgtagcttagaaggaaatgcgtggaagaacttggagacgcccttgtgacctccaagattttccatgcattcgtccataatgatggcaatgggcccacgggcggcggcctgggcgaagatatttctgggatcactaacgtcatagttgtgttccaggatgagatcgtcataggccatttttacaaagcgcgggcggagggtgccagactgcggtataatggttccatccggcccaggggcgtagttaccctcacagatttgcatttcccacgctttgagttcagatggggggatcatgtctacctgcggggcgatgaagaaaacggtttccggggtaggggagatcagctgggaagaaagcaggttcctgagcagctgcgacttaccgcagccggtgggcccgtaaatcacacctattaccgggtgcaactggtagttaagagagctgcagctgccgtcatccctgagcaggggggccacttcgttaagcatgtccctgactcgcatgttttccctgaccaaatccgccagaaggcgctcgccgcccagcgatagcagttcttgcaaggaagcaaagtttttcaacggtttgagaccgtccgccgtaggcatgcttttgagcgtttgaccaagcagttccaggcggtcccacagctcggtcacctgctctacggcatctcgatccagcatatctcctcgtttcgcgggttggggcggctttcgctgtacggcagtagtcggtgctcgtccagacgggccagggtcatgtctttccacgggcgcagggtcctcgtcagcgtagtctgggtcacggtgaaggggtgcgctccgggctgcgcgctggccagggtgcgcttgaggctggtcctgctggtgctgaagcgctgccggtcttcgccctgcgcgtcggccaggtagcatttgaccatggtgtcatagtccagcccctccgcggcgtggcccttggcgcgcagcttgcccttggaggaggcgccgcacgaggggcagtgcagacttttgagggcgtagagcttgggcgcgagaaataccgattccggggagtaggcatccgcgccgcaggccccgcagacggtctcgcattccacgagccaggtgagctctggccgttcggggtcaaaaaccaggtttcccccatgctttttgatgcgtttcttacctctggtttccatgagccggtgtccacgctcggtgacgaaaaggctgtccgtgtccccgtatacagacttgagaggcctgtcctcgagcggtgttccgcggtcctcctcgtatagaaactcggaccactctgagacaaaggctcgcgtccaggccagcacgaaggaggctaagtgggaggggtagcggtcgttgtccactagggggtccactcgctccagggtgtgaagacacatgtcgccctcttcggcatcaaggaaggtgattggtttgtaggtgtaggccacgtgaccgggtgttcctgaaggggggctataaaagggggtgggggcgcgttcgtcctcactctcttccgcatcgctgtctgcgagggccagctgttggggtgagtactccctctgaaaagcgggcatgacttctgcgctaagattgtcagtttccaaaaacgaggaggatttgatattcacctggcccgcggtgatgcctttgagggtggccgcatccatctggtcagaaaagacaatctttttgttgtcaagcttggtggcaaacgacccgtagagggcgttggacagcaacttggcgatggagcgcagggtttggtttttgtcgcgatcggcgcgctccttggccgcgatgtttagctgcacgtattcgcgcgcaacgcaccgccattcgggaaagacggtggtgcgctcgtcgggcaccaggtgcacgcgccaaccgcggttgtgcagggtgacaaggtcaacgctggtggctacctctccgcgtaggcgctcgttggtccagcagaggcggccgcccttgcgcgagcagaatggcggtagggggtctagctgcgtctcgtccggggggtctgcgtccacggtaaagaccccgggcagcaggcgcgcgtcgaagtagtctatcttgcatccttgcaagtctagcgcctgctgccatgcgcgggcggcaagcgcgcgctcgtatgggttgagtgggggaccccatggcatggggtgggtgagcgcggaggcgtacatgccgcaaatgtcgtaaacgtagaggggctctctgagtattccaagatatgtagggtagcatcttccaccgcggatgctggcgcgcacgtaatcgtatagttcgtgcgagggagcgaggaggtcgggaccgaggttgctacgggcgggctgctctgctcggaagactatctgcctgaagatggcatgtgagttggatgatatggttggacgctggaagacgttgaagctggcgtctgtgagacctaccgcgtcacgcacgaaggaggcgtaggagtcgcgcagcttgttgaccagctcggcggtgacctgcacgtctagggcgcagtagtccagggtttccttgatgatgtcatacttatcctgtcccttttttttccacagctcgcggttgaggacaaactcttcgcggtctttccagtactcttggatcggaaacccgtcggcctccgaacggtaagagcctagcatgtagaactggttgacggcctggtaggcgcagcatcccttttctacgggtagcgcgtatgcctgcgcggccttccggagcgaggtgtgggtgagcgcaaaggtgtccctgaccatgactttgaggtactggtatttgaagtcagtgtcgtcgcatccgccctgctcccagagcaaaaagtccgtgcgctttttggaacgcggatttggcagggcgaaggtgacatcgttgaagagtatctttcccgcgcgaggcataaagttgcgtgtgatgcggaagggtcccggcacctcggaacggttgttaattacctgggcggcgagcacgatctcgtcaaagccgttgatgttgtggcccacaatgtaaagttccaagaagcgcgggatgcccttgatggaaggcaattttttaagttcctcgtaggtgagctcttcaggggagctgagcccgtgctctgaaagggcccagtctgcaagatgagggttggaagcgacgaatgagctccacaggtcacgggccattagcatttgcaggtggtcgcgaaaggtcctaaactggcgacctatggccattttttctggggtgatgcagtagaaggtaagcgggtcttgttcccagcggtcccatccaaggttcgcggctaggtctcgcgcggcagtcactagaggctcatctccgccgaacttcatgaccagcatgaagggcacgagctgcttcccaaaggcccccatccaagtataggtctctacatcgtaggtgacaaagagacgctcggtgcgaggatgcgagccgatcgggaagaactggatctcccgccaccaattggaggagtggctattgatgtggtgaaagtagaagtccctgcgacgggccgaacactcgtgctggcttttgtaaaaacgtgcgcagtactggcagcggtgcacgggctgtacatcctgcacgaggttgacctgacgaccgcgcacaaggaagcagagtgggaatttgagcccctcgcctggcgggtttggctggtggtcttctacttcggctgcttgtccttgaccgtctggctgctcgaggggagttacggtggatcggaccaccacgccgcgcgagcccaaagtccagatgtccgcgcgcggcggtcggagcttgatgacaacatcgcgcagatgggagctgtccatggtctggagctcccgcggcgtcaggtcaggcgggagctcctgcaggtttacctcgcatagacgggtcagggcgcgggctagatccaggtgatacctaatttccaggggctggttggtggcggcgtcgatggcttgcaagaggccgcatccccgcggcgcgactacggtaccgcgcggcgggcggtgggccgcgggggtgtccttggatgatgcatctaaaagcggtgacgcgggcgagcccccggaggtagggggggctccggacccgccgggagagggggcaggggcacgtcggcgccgcgcgcgggcaggagctggtgctgcgcgcgtaggttgctggcgaacgcgacgacgcggcggttgatctcctgaatctggcgcctctgcgtgaagacgacgggcccggtgagcttgagcctgaaagagagttcgacagaatcaatttcggtgtcgttgacggcggcctggcgcaaaatctcctgcacgtctcctgagttgtcttgataggcgatctcggccatgaactgctcgatctcttcctcctggagatctccgcgtccggctcgctccacggtggcggcgaggtcgttggaaatgcgggccatgagctgcgagaaggcgttgaggcctccctcgttccagacgcggctgtagaccacgcccccttcggcatcgcgggcgcgcatgaccacctgcgcgagattgagctccacgtgccgggcgaagacggcgtagtttcgcaggcgctgaaagaggtagttgagggtggtggcggtgtgttctgccacgaagaagtacataacccagcgtcgcaacgtggattcgttgatatcccccaaggcctcaaggcgctccatggcctcgtagaagtccacggcgaagttgaaaaactgggagttgcgcgccgacacggttaactcctcctccagaagacggatgagctcggcgacagtgtcgcgcacctcgcgctcaaaggctacaggggcctcttcttcttcttcaatctcctcttccataagggcctccccttcttcttcttctggcggcggtgggggaggggggacacggcggcgacgacggcgcaccgggaggcggtcgacaaagcgctcgatcatctccccgcggcgacggcgcatggtctcggtgacggcgcggccgttctcgcgggggcgcagttggaagacgccgcccgtcatgtcccggttatgggttggcggggggctgccatgcggcagggatacggcgctaacgatgcatctcaacaattgttgtgtaggtactccgccgccgagggacctgagcgagtccgcatcgaccggatcggaaaacctctcgagaaaggcgtctaaccagtcacagtcgcaaggtaggctgagcaccgtggcgggcggcagcgggcggcggtcggggttgtttctggcggaggtgctgctgatgatgtaattaaagtaggcggtcttgagacggcggatggtcgacagaagcaccatgtccttgggtccggcctgctgaatgcgcaggcggtcggccatgccccaggcttcgttttgacatcggcgcaggtctttgtagtagtcttgcatgagcctttctaccggcacttcttcttctccttcctcttgtcctgcatctcttgcatctatcgctgcggcggcggcggagtttggccgtaggtggcgccctcttcctcccatgcgtgtgaccccgaagcccctcatcggctgaagcagggctaggtcggcgacaacgcgctcggctaatatggcctgctgcacctgcgtgagggtagactggaagtcatccatgtccacaaagcggtggtatgcgcccgtgttgatggtgtaagtgcagttggccataacggaccagttaacggtctggtgacccggctgcgagagctcggtgtacctgagacgcgagtaagccctcgagtcaaatacgtagtcgttgcaagtccgcaccaggtactggtatcccaccaaaaagtgcggcggcggctggcggtagaggggccagcgtagggtggccggggctccgggggcgagatcttccaacataaggcgatgatatccgtagatgtacctggacatccaggtgatgccggcggcggtggtggaggcgcgcggaaagtcgcggacgcggttccagatgttgcgcagcggcaaaaagtgctccatggtcgggacgctctggccggtcaggcgcgcgcaatcgttgacgctctagaccgtgcaaaaggagagcctgtaagcgggcactcttccgtggtctggtggataaattcgcaagggtatcatggcggacgaccggggttcgagccccgtatccggccgtccgccgtgatccatgcggttaccgcccgcgtgtcgaacccaggtgtgcgacgtcagacaacgggggagtgctccttttggcttccttccaggcgcggcggctgctgcgctagcttttttggccactggccgcgcgcagcgtaagcggttaggctggaaagcgaaagcattaagtggctcgctccctgtagccggagggttattttccaagggttgagtcgcgggacccccggttcgagtctcggaccggccggactgcggcgaacgggggtttgcctccccgtcatgcaagaccccgcttgcaaattcctccggaaacagggacgagccccttttttgcttttcccagatgcatccggtgctgcggcagatgcgcccccctcctcagcagcggcaagagcaagagcagcggcagacatgcagggcaccctcccctcctcctaccgcgtcaggaggggcgacatccgcggttgacgcggcagcagatggtgattacgaacccccgcggcgccgggcccggcactacctggacttggaggagggcgagggcctggcgcggctaggagcgccctctcctgagcggtacccaagggtgcagctgaagcgtgatacgcgtgaggcgtacgtgccgcggcagaacctgtttcgcgaccgcgagggagaggagcccgaggagatgcgggatcgaaagttccacgcagggcgcgagctgcggcatggcctgaatcgcgagcggttgctgcgcgaggaggactttgagcccgacgcgcgaaccgggattagtcccgcgcgcgcacacgtggcggccgccgacctggtaaccgcatacgagcagacggtgaaccaggagattaactttcaaaaaagctttaacaaccacgtgcgtacgcttgtggcgcgcgaggaggtggctataggactgatgcatctgtgggactttgtaagcgcgctggagcaaaacccaaatagcaagccgctcatggcgcagctgttccttatagtgcagcacagcagggacaacgaggcattcagggatgcgctgctaaacatagtagagcccgagggccgctggctgctcgatttgataaacatcctgcagagcatagtggtgcaggagcgcagcttgagcctggctgacaaggtggccgccatcaactattccatgcttagcctgggcaagttttacgcccgcaagatataccataccccttacgttcccatagacaaggaggtaaagatcgaggggttctacatgcgcatggcgctgaaggtgcttaccttgagcgacgacctgggcgtttatcgcaacgagcgcatccacaaggccgtgagcgtgagccggcggcgcgagctcagcgaccgcgagctgatgcacagcctgcaaagggccctggctggcacgggcagcggcgatagagaggccgagtcctactttgacgcgggcgctgacctgcgctgggccccaagccgacgcgccctggaggcagctggggccggacctgggctggcggtggcacccgcgcgcgctggcaacgtcggcggcgtggaggaatatgacgaggacgatgagtacgagccagaggacggcgagtactaagcggtgatgtttctgatcagatgatgcaagacgcaacggacccggcggtgcgggcggcgctgcagagccagccgtccggccttaactccacggacgactggcgccaggtcatggaccgcatcatgtcgctgactgcgcgcaatcctgacgcgttccggcagcagccgcaggccaaccggctctccgcaattctggaagcggtggtcccggcgcgcgcaaaccccacgcacgagaaggtgctggcgatcgtaaacgcgctggccgaaaacagggccatccggcccgacgaggccggcctggtctacgacgcgctgcttcagcgcgtggctcgttacaacagcggcaacgtgcagaccaacctggaccggctggtgggggatgtgcgcgaggccgtggcgcagcgtgagcgcgcgcagcagcagggcaacctgggctccatggttgcactaaacgccttcctgagtacacagcccgccaacgtgccgcggggacaggaggactacaccaactttgtgagcgcactgcggctaatggtgactgagacaccgcaaagtgaggtgtaccagtctgggccagactattttttccagaccagtagacaaggcctgcagaccgtaaacctgagccaggctttcaaaaacttgcaggggctgtggggggtgcgggctcccacaggcgaccgcgcgaccgtgtctagcttgctgacgcccaactcgcgcctgttgctgctgctaatagcgcccttcacggacagtggcagcgtgtcccgggacacatacctaggtcacttgctgacactgtaccgcgaggccataggtcaggcgcatgtggacgagcatactttccaggagattacaagtgtcagccgcgcgctggggcaggaggacacgggcagcctggaggcaaccctaaactacctgctgaccaaccggcggcagaagatcccctcgttgcacagtttaaacagcgaggaggagcgcattttgcgctacgtgcagcagagcgtgagccttaacctgatgcgcgacggggtaacgcccagcgtggcgctggacatgaccgcgcgcaacatggaaccgggcatgtatgcctcaaaccggccgtttatcaaccgcctaatggactacttgcatcgcgcggccgccgtgaaccccgagtatttcaccaatgccatcttgaacccgcactggctaccgccccctggtttctacaccgggggattcgaggtgcccgagggtaacgatggattcctctgggacgacatagacgacagcgtgttttccccgcaaccgcagaccctgctagagttgcaacagcgcgagcaggcagaggcggcgctgcgaaaggaaagcttccgcaggccaagcagcttgtccgatctaggcgctgcggccccgcggtcagatgctagtagcccatttccaagcttgatagggtctcttaccagcactcgcaccacccgcccgcgcctgctgggcgaggaggagtacctaaacaactcgctgctgcagccgcagcgcgaaaaaaacctgcctccggcatttcccaacaacgggatagagagcctagtggacaagatgagtagatggaagacgtacgcgcaggagcacagggacgtgccaggcccgcgcccgcccacccgtcgtcaaaggcacgaccgtcagcggggtctggtgtgggaggacgatgactcggcagacgacagcagcgtcctggatttgggagggagtggcaacccgtttgcgcaccttcgccccaggctggggagaatgttttaaaaaaaaaaaagcatgatgcaaaataaaaaactcaccaaggccatggcaccgagcgttggttttcttgtattccccttagtatgcggcgcgcggcgatgtatgaggaaggtcctcctccctcctacgagagtgtggtgagcgcggcgccagtggcggcggcgctgggttctcccttcgatgctcccctggacccgccgtttgtgcctccgcggtacctgcggcctaccggggggagaaacagcatccgttactctgagttggcacccctattcgacaccacccgtgtgtacctggtggacaacaagtcaacggatgtggcatccctgaactaccagaacgaccacagcaactttctgaccacggtcattcaaaacaatgactacagcccgggggaggcaagcacacagaccatcaatcttgacgaccggtcgcactggggcggcgacctgaaaaccatcctgcataccaacatgccaaatgtgaacgagttcatgtttaccaataagtttaaggcgcgggtgatggtgtcgcgcttgcctactaaggacaatcaggtggagctgaaatacgagtgggtggagttcacgctgcccgagggcaactactccgagaccatgaccatagaccttatgaacaacgcgatcgtggagcactacttgaaagtgggcagacagaacggggttctggaaagcgacatcggggtaaagtttgacacccgcaacttcagactggggtttgaccccgtcactggtcttgtcatgcctggggtatatacaaacgaagccttccatccagacatcattttgctgccaggatgcggggtggacttcacccacagccgcctgagcaacttgttgggcatccgcaagcggcaacccttccaggagggctttaggatcacctacgatgatctggagggtggtaacattcccgcactgttggatgtggacgcctaccaggcgagcttgaaagatgacaccgaacagggcgggggtggcgcaggcggcagcaacagcagtggcagcggcgcggaagagaactccaacgcggcagccgcggcaatgcagccggtggaggacatgaacgatcatgccattcgcggcgacacctttgccacacgggctgaggagaagcgcgctgaggccgaagcagcggccgaagctgccgcccccgctgcgcaacccgaggtcgagaagcctcagaagaaaccggtgatcaaacccctgacagaggacagcaagaaacgcagttacaacctaataagcaatgacagcaccttcacccagtaccgcagctggtaccttgcatacaactacggcgaccctcagaccggaatccgctcatggaccctgctttgcactcctgacgtaacctgcggctcggagcaggtctactggtcgttgccagacatgatgcaagaccccgtgaccttccgctccacgcgccagatcagcaactttccggtggtgggcgccgagctgttgcccgtgcactccaagagcttctacaacgaccaggccgtctactcccaactcatccgccagtttacctctctgacccacgtgttcaatcgctttcccgagaaccagattttggcgcgcccgccagcccccaccatcaccaccgtcagtgaaaacgttcctgctctcacagatcacgggacgctaccgctgcgcaacagcatcggaggagtccagcgagtgaccattactgacgccagacgccgcacctgcccctacgtttacaaggccctgggcatagtctcgccgcgcgtcctatcgagccgcactttttgagcaagcatgtccatccttatatcgcccagcaataacacaggctggggcctgcgcttcccaagcaagatgtttggcggggccaagaagcgctccgaccaacacccagtgcgcgtgcgcgggcactaccgcgcgccctggggcgcgcacaaacgcggccgcactgggcgcaccaccgtcgatgacgccatcgacgcggtggtggaggaggcgcgcaactacacgcccacgccgccaccagtgtccacagtggacgcggccattcagaccgtggtgcgcggagcccggcgctatgctaaaatgaagagacggcggaggcgcgtagcacgtcgccaccgccgccgacccggcactgccgcccaacgcgcggcggcggccctgcttaaccgcgcacgtcgcaccggccgacgggcggccatgcgggccgctcgaaggctggccgcgggtattgtcactgtgccccccaggtccaggcgacgagcggccgccgcagcagccgcggccattagtgctatgactcagggtcgcaggggcaacgtgtattgggtgcgcgactcggttagcggcctgcgcgtgcccgtgcgcacccgccccccgcgcaactagattgcaagaaaaaactacttagactcgtactgttgtatgtatccagcggcggcggcgcgcaacgaagctatgtccaagcgcaaaatcaaagaagagatgctccaggtcatcgcgccggagatctatggccccccgaagaaggaagagcaggattacaagccccgaaagctaaagcgggtcaaaaagaaaaagaaagatgatgatgatgaacttgacgacgaggtggaactgctgcacgctaccgcgcccaggcgacgggtacagtggaaaggtcgacgcgtaaaacgtgttttgcgacccggcaccaccgtagtctttacgcccggtgagcgctccacccgcacctacaagcgcgtgtatgatgaggtgtacggcgacgaggacctgcttgagcaggccaacgagcgcctcggggagtttgcctacggaaagcggcataaggacatgctggcgttgccgctggacgagggcaacccaacacctagcctaaagcccgtaacactgcagcaggtgctgcccgcgcttgcaccgtccgaagaaaagcgcggcctaaagcgcgagtctggtgacttggcacccaccgtgcagctgatggtacccaagcgccagcgactggaagatgtcttggaaaaaatgaccgtggaacctgggctggagcccgaggtccgcgtgcggccaatcaagcaggtggcgccgggactgggcgtgcagaccgtggacgttcagatacccactaccagtagcaccagtattgccaccgccacagagggcatggagacacaaacgtccccggttgcctcagcggtggcggatgccgcggtgcaggcggtcgctgcggccgcgtccaagacctctacggaggtgcaaacggacccgtggatgtttcgcgtttcagccccccggcgcccgcgcggttcgaggaagtacggcgccgccagcgcgctactgcccgaatatgccctacatccttccattgcgcctacccccggctatcgtggctacacctaccgccccagaagacgagcaactacccgacgccgaaccaccactggaacccgccgccgccgtcgccgtcgccagcccgtgctggccccgatttccgtgcgcagggtggctcgcgaaggaggcaggaccctggtgctgccaacagcgcgctaccaccccagcatcgtttaaaagccggtctttgtggttcttgcagatatggccctcacctgccgcctccgtttcccggtgccgggattccgaggaagaatgcaccgtaggaggggcatggccggccacggcctgacgggcggcatgcgtcgtgcgcaccaccggcggcggcgcgcgtcgcaccgtcgcatgcgcggcggtatcctgcccctccttattccactgatcgccgcggcgattggcgccgtgcccggaattgcatccgtggccttgcaggcgcagagacactgattaaaaacaagttgcatgtggaaaaatcaaaataaaaagtctggactctcacgctcgcttggtcctgtaactattttgtagaatggaagacatcaactttgcgtctctggccccgcgacacggctcgcgcccgttcatgggaaactggcaagatatcggcaccagcaatatgagcggtggcgccttcagctggggctcgctgtggagcggcattaaaaatttcggttccaccgttaagaactatggcagcaaggcctggaacagcagcacaggccagatgctgagggataagttgaaagagcaaaatttccaacaaaaggtggtagatggcctggcctctggcattagcggggtggtggacctggccaaccaggcagtgcaaaataagattaacagtaagcttgatccccgccctcccgtagaggagcctccaccggccgtggagacagtgtctccagaggggcgtggcgaaaagcgtccgcgccccgacagggaagaaactctggtgacgcaaatagacgagcctccctcgtacgaggaggcactaaagcaaggcctgcccaccacccgtcccatcgcgcccatggctaccggagtgctgggccagcacacacccgtaacgctggacctgcctccccccgccgacacccagcagaaacctgtgctgccaggcccgaccgccgttgttgtaacccgtcctagccgcgcgtccctgcgccgcgccgccagcggtccgcgatcgttgcggcccgtagccagtggcaactggcaaagcacactgaacagcatcgtgggtctgggggtgcaatccctgaagcgccgacgatgcttctgaatagctaacgtgtcgtatgtgtgtcatgtatgcgtccatgtcgccgccagaggagctgctgagccgccgcgcgcccgctttccaagatggctaccccttcgatgatgccgcagtggtcttacatgcacatctcgggccaggacgcctcggagtacctgagccccgggctggtgcagtttgcccgcgccaccgagacgtacttcagcctgaataacaagtttagaaaccccacggtggcgcctacgcacgacgtgaccacagaccggtcccagcgtttgacgctgcggttcatccctgtggaccgtgaggatactgcgtactcgtacaaggcgcggttcaccctagctgtgggtgataaccgtgtgctggacatggcttccacgtactttgacatccgcggcgtgctggacaggggccctacttttaagccctactctggcactgcctacaacgccctggctcccaagggtgccccaaatccttgcgaatgggatgaagctgctactgctcttgaaataaacctagaagaagaggacgatgacaacgaagacgaagtagacgagcaagctgagcagcaaaaaactcacgtatttgggcaggcgccttattctggtataaatattacaaaggagggtattcaaataggtgtcgaaggtcaaacacctaaatatgccgataaaacatttcaacctgaacctcaaataggagaatctcagtggtacgaaactgaaattaatcatgcagctgggagagtccttaaaaagactaccccaatgaaaccatgttacggttcatatgcaaaacccacaaatgaaaatggagggcaaggcattcttgtaaagcaacaaaatggaaagctagaaagtcaagtggaaatgcaatttttctcaactggaagcggttctcgctacctggagcctggcccagtgactgccgctggttccggaagcagatacatggacggaacaatgtcccaggttgccggttctggctcccctaaagtggtattgtacagtgaagatgtagatatagaaaccccagacactcatatttcttacatgcccactattaaggaaggtaactcacgagaactaatgggccaacaatctatgcccaacaggcctaattacattgcttttagggacaattttattggtctaatgtattacaacagcacgggtaatatgggtgttctggcgggccaagcatcgcagttgaatgctgttgtagatttgcaagacagaaacacagagctttcataccagcttttgcttgattccattggtgatagaaccaggtacttttctatgtggaatcaggctgttgacagctatgatccagatgttagaattattgaaaatcatggaactgaagatgaacttccaaattactgctttccactgggaggtgtgattaatacagagactcttaccaaggtaaaacctaaaacaggtcaggaaaatggatgggaaaaagatgctacagaattttcagataaaaatgaaataagagttggaaataattttgccatggaaatcaatctaaatgccaacctgtggagaaatttcctgtactccaacatagcgctgtatttgcccgacaagctaaagtacagtccttccaacgtaaaaatttctgataacccaaacacctacgactacatgaacaagcgagtggtggctcccgggttagtggactgctacattaaccttggagcacgctggtcccttgactatatggacaacgtcaacccatttaaccaccaccgcaatgctggcctgcgctaccgctcaatgttgctgggcaatggtcgctatgtgcccttccacatccaggtgcctcagaagttctttgccattaaaaacctccttctcctgccgggctcatacacctacgagtggaacttcaggaaggatgttaacatggttctgcagagctccctaggaaatgacctaagggttgacggagccagcattaagtttgatagcatttgcctttacgccaccttcttccccatggcccacaacaccgcctccacgcttgaggccatgcttagaaacgacaccaacgaccagtcctttaacgactatctctccgccgccaacatgctctaccctatacccgccaacgctaccaacgtgcccatatccatcccctcccgcaactgggcggctttccgcggctgggccttcacgcgccttaagactaaggaaaccccatcactgggctcgggctacgacccttattacacctactctggctctataccctacctagatggaaccttttacctcaaccacacctttaagaaggctgccattacctttgactcttctgtcagctggcctggcaatgaccgcctgcttacccccaacgagtttgaaattaagcgctcagttgacggggagggttacaacgttgcccagtgtaacatgaccaaagactggttcctggtacaaatgctagctaactataacattggctaccagggcttctatatcccagagagctacaaggaccgcatgtactccttctttagaaacttccagcccatgagccgtcaggtggtggatgatactaaatacaaggactaccaacaggtgggcatcctacaccaacacaacaactctggatttgttggctaccttgcccccaccatgcgcgaaggacaggcctaccctgctaacttcccctatccgcttataggcaagaccgcagttgacagcattacccagaaaaagtttctttgcgatcgcaccctttggcgcatcccattctccagtaactttatgtccatgggcgcactcacagacctgggccaaaaccttctctacgccaactccgcccactccctagacatgacttttgaggtggatcccatggacgagcccacccttctttatgttttgtttgaagtctttgacaaggtccgtgtgcaccagccgcaccgcggcgtcatcgaaaccgtgtacctgcgcacgcccttctcggccggcaacgccacaacataaagaagcaagcaacatcaacaacagctgccgccatgggctccagtgagcaggaactgaaagccattgtcaaagatcttggttgtgggccatattttttgggcacctatgacaagcgctttccaggctttgtttctccacacaagctcgcctgcgccatagtcaatacggccggtcgcgagactgggggcgtacactggatggcctttgcctggaacccgcactcaaaaacatgctacctctttgagccctttggcttttctgaccagcgactcaagcaggtttaccagtttgagtacgagtcactcctgcgccgtagcgccattgcttcttcccccgaccgctgtataacgctggaaaagtccacccaaagcgtacaggggcccaactcggccgcctgtggactattctgctgcatgtttctccacgcctttgccaactggccccaaactcccatggatcacaaccccaccatgaaccttattaccggggtacccaactccatgctcaacagtccccaggtacagcccaccctgcgtcgcaaccaggaacagctctacagcttcctggagcgccactcgccctacttccgcagccacagtgcgcagattaggagcgccacttctttttgtcacttgaaaaacatgtaaaaataatgtactagagacactttcaataaaggcaaatgcttttatttgtacactctcgggtgattatttacccccacccttgccgtctgcgccgtttaaaaatcaaaggggttctgccgcgcatcgctatgcgccactggcagggacacgttgcgatactggtgtttagtgctccacttaaactcaggcacaaccatccgcggcagctcggtgaagttttcactccacaggctgcgcaccatcaccaacgcgtttagcaggtcgggcgccgatatcttgaagtcgcagttggggcctccgccctgcgcgcgcgagttgcgatacacagggttgcagcactggaacactatcagcgccgggtggtgcacgctggccagcacgctcttgtcggagatcagatccgcgtccaggtcctccgcgttgctcagggcgaacggagtcaactttggtagctgccttcccaaaaagggcgcgtgcccaggctttgagttgcactcgcaccgtagtggcatcaaaaggtgaccgtgcccggtctgggcgttaggatacagcgcctgcataaaagccttgatctgcttaaaagccacctgagcctttgcgccttcagagaagaacatgccgcaagacttgccggaaaactgattggccggacaggccgcgtcgtgcacgcagcaccttgcgtcggtgttggagatctgcaccacatttcggccccaccggttcttcacgatcttggccttgctagactgctccttcagcgcgcgctgcccgttttcgctcgtcacatccatttcaatcacgtgctccttatttatcataatgcttccgtgtagacacttaagctcgccttcgatctcagcgcagcggtgcagccacaacgcgcagcccgtgggctcgtgatgcttgtaggtcacctctgcaaacgactgcaggtacgcctgcaggaatcgccccatcatcgtcacaaaggtcttgttgctggtgaaggtcagctgcaacccgcggtgctcctcgttcagccaggtcttgcatacggccgccagagcttccacttggtcaggcagtagtttgaagttcgcctttagatcgttatccacgtggtacttgtccatcagcgcgcgcgcagcctccatgcccttctcccacgcagacacgatcggcacactcagcgggttcatcaccgtaatttcactttccgcttcgctgggctcttcctcttcctcttgcgtccgcataccacgcgccactgggtcgtcttcattcagccgccgcactgtgcgcttacctcctttgccatgcttgattagcaccggtgggttgctgaaacccaccatttgtagcgccacatcttctctttcttcctcgctgtccacgattacctctggtgatggcgggcgctcgggcttgggagaagggcgcttctttttcttcttgggcgcaatggccaaatccgccgccgaggtcgatggccgcgggctgggtgtgcgcggcaccagcgcgtcttgtgatgagtcttcctcgtcctcggactcgatacgccgcctcatccgcttttttgggggcgcccggggaggcggcggcgacggggacggggacgacacgtcctccatggttgggggacgtcgcgccgcaccgcgtccgcgctcgggggtggtttcgcgctgctcctcttcccgactggccatttccttctcctataggcagaaaaagatcatggagtcagtcgagaagaaggacagcctaaccgccccctctgagttcgccaccaccgcctccaccgatgccgccaacgcgcctaccaccttccccgtcgaggcacccccgcttgaggaggaggaagtgattatcgagcaggacccaggttttgtaagcgaagacgacgaggaccgctcagtaccaacagaggataaaaagcaagaccaggacaacgcagaggcaaacgaggaacaagtcgggcggggggacgaaaggcatggcgactacctagatgtgggagacgacgtgctgttgaagcatctgcagcgccagtgcgccattatctgcgacgcgttgcaagagcgcagcgatgtgcccctcgccatagcggatgtcagccttgcctacgaacgccacctattctcaccgcgcgtaccccccaaacgccaagaaaacggcacatgcgagcccaacccgcgcctcaacttctaccccgtatttgccgtgccagaggtgcttgccacctatcacatctttttccaaaactgcaagatacccctatcctgccgtgccaaccgcagccgagcggacaagcagctggccttgcggcagggcgctgtcatacctgatatcgcctcgctcaacgaagtgccaaaaatctttgagggtcttggacgcgacgagaagcgcgcggcaaacgctctgcaacaggaaaacagcgaaaatgaaagtcactctggagtgttggtggaactcgagggtgacaacgcgcgcctagccgtactaaaacgcagcatcgaggtcacccactttgcctacccggcacttaacctaccccccaaggtcatgagcacagtcatgagtgagctgatcgtgcgccgtgcgcagcccctggagagggatgcaaatttgcaagaacaaacagaggagggcctacccgcagttggcgacgagcagctagcgcgctggcttcaaacgcgcgagcctgccgacttggaggagcgacgcaaactaatgatggccgcagtgctcgttaccgtggagcttgagtgcatgcagcggttctttgctgacccggagatgcagcgcaagctagaggaaacattgcactacacctttcgacagggctacgtacgccaggcctgcaagatctccaacgtggagctctgcaacctggtctcctaccttggaattttgcacgaaaaccgccttgggcaaaacgtgcttcattccacgctcaagggcgaggcgcgccgcgactacgtccgcgactgcgtttacttatttctatgctacacctggcagacggccatgggcgtttggcagcagtgcttggaggagtgcaacctcaaggagctgcagaaactgctaaagcaaaacttgaaggacctatggacggccttcaacgagcgctccgtggccgcgcacctggcggacatcattttccccgaacgcctgcttaaaaccctgcaacagggtctgccagacttcaccagtcaaagcatgttgcagaactttaggaactttatcctagagcgctcaggaatcttgcccgccacctgctgtgcacttcctagcgactttgtgcccattaagtaccgcgaatgccctccgccgctttggggccactgctaccttctgcagctagccaactaccttgcctaccactctgacataatggaagacgtgagcggtgacggtctactggagtgtcactgtcgctgcaacctatgcaccccgcaccgctccctggtttgcaattcgcagctgcttaacgaaagtcaaattatcggtacctttgagctgcagggtccctcgcctgacgaaaagtccgcggctccggggttgaaactcactccggggctgtggacgtcggcttaccttcgcaaatttgtacctgaggactaccacgcccacgagattaggttctacgaagaccaatcccgcccgccaaatgcggagcttaccgcctgcgtcattacccagggccacattcttggccaattgcaagccatcaacaaagcccgccaagagtttctgctacgaaagggacggggggtttacttggacccccagtccggcgaggagctcaacccaatccccccgccgccgcagccctatcagcagcagccgcgggcccttgcttcccaggatggcacccaaaaagaagctgcagctgccgccgccacccacggacgaggaggaatactgggacagtcaggcagaggaggttttggacgaggaggaggaggacatgatggaagactgggagagcctagacgaggaagcttccgaggtcgaagaggtgtcagacgaaacaccgtcaccctcggtcgcattcccctcgccggcgccccagaaatcggcaaccggttccagcatggctacaacctccgctcctcaggcgccgccggcactgcccgttcgccgacccaaccgtagatgggacaccactggaaccagggccggtaagtccaagcagccgccgccgttagcccaagagcaacaacagcgccaaggctaccgctcatggcgcgggcacaagaacgccatagttgcttgcttgcaagactgtgggggcaacatctccttcgcccgccgctttcttctctaccatcacggcgtggccttcccccgtaacatcctgcattactaccgtcatctctacagcccatactgcaccggcggcagcggcagcggcagcaacagcagcggccacacagaagcaaaggcgaccggatagcaagactctgacaaagcccaagaaatccacagcggcggcagcagcaggaggaggagcgctgcgtctggcgcccaacgaacccgtatcgacccgcgagcttagaaacaggatttttcccactctgtatgctatatttcaacagagcaggggccaagaacaagagctgaaaataaaaaacaggtctctgcgatccctcacccgcagctgcctgtatcacaaaagcgaagatcagcttcggcgcacgctggaagacgcggaggctctcttcagtaaatactgcgcgctgactcttaaggactagtttcgcgccctttctcaaatttaagcgcgaaaactacgtcatctccagcggccacacccggcgccagcacctgtcgtcagcgccattatgagcaaggaaattcccacgccctacatgtggagttaccagccacaaatgggacttgcggctggagctgcccaagactactcaacccgaataaactacatgagcgcgggaccccacatgatatcccgggtcaacggaatccgcgcccaccgaaaccgaattctcttggaacaggcggctattaccaccacacctcgtaataaccttaatccccgtagttggcccgctgccctggtgtaccaggaaagtcccgctcccaccactgtggtacttcccagagacgcccaggccgaagttcagatgactaactcaggggcgcagcttgcgggcggctttcgtcacagggtgcggtcgcccgggcagggtataactcacctgacaatcagagggcgaggtattcagctcaacgacgagtcggtgagctcctcgcttggtctccgtccggacgggacatttcagatcggcggcgccggccgtccttcattcacgcctcgtcaggcaatcctaactctgcagacctcgtcctctgagccgcgctctggaggcattggaactctgcaatttattgaggagtttgtgccatcggtctactttaaccccttctcgggacctcccggccactatccggatcaatttattcctaactttgacgcggtaaaggactcggcggacggctacgactgaatgttaagtggagaggcagagcaactgcgcctgaaacacctggtccactgtcgccgccacaagtgctttgcccgcgactccggtgagttttgctactttgaattgcccgaggatcatatcgagggcccggcgcacggcgtccggcttaccgcccagggagagcttgcccgtagcctgattcgggagtttacccagcgccccctgctagttgagcgggacaggggaccctgtgttctcactgtgatttgcaactgtcctaaccttggattacatcaagatctttgttgccatctctgtgctgagtataataaatacagaaattaaaatatactggggctcctatcgccatcctgtaaacgccaccgtcttcacccgcccaagcaaaccaaggcgaaccttacctggtacttttaacatctctccctctgtgatttacaacagtttcaacccagacggagtgagtctacgagagaacctctccgagctcagctactccatcagaaaaaacaccaccctccttacctgccgggaacgtacgagtgcgtcaccggccgctgcaccacacctaccgcctgaccgtaaaccagactttttccggacagacctcaataactctgtttaccagaacaggaggtgagcttagaaaacccttagggtattaggccaaaggcgcagctactgtggggtttatgaacaattcaagcaactctacgggctattctaattcaggtttctctagaatcggggttggggttattctctgtcttgtgattctctttattcttatactaacgcttctctgcctaaggctcgccgcctgctgtgtgcacatttgcatttattgtcagctttttaaacgctggggtcgccacccaagatgattaggtacataatcctaggtttactcacccttgcgtcagcccacggtaccacccaaaaggtggattttaaggagccagcctgtaatgttacattcgcagctgaagctaatgagtgcaccactcttataaaatgcaccacagaacatgaaaagctgcttattcgccacaaaaacaaaattggcaagtatgctgtttatgctatttggcagccaggtgacactacagagtataatgttacagttttccagggtaaaagtcataaaacttttatgtatacttttccattttatgaaatgtgcgacattaccatgtacatgagcaaacagtataagttgtggcccccacaaaattgtgtggaaaacactggcactttctgctgcactgctatgctaattacagtgctcgctttggtctgtaccctactctatattaaatacaaaagcagacgcagctttattgaggaaaagaaaatgccttaatttactaagttacaaagctaatgtcaccactaactgctttactcgctgcttgcaaaacaaattcaaaaagttagcattataattagaataggatttaaaccccccggtcatttcctgctcaataccattcccctgaacaattgactctatgtgggatatgctccagcgctacaaccttgaagtcaggcttcctggatgtcagcatctgactttggccagcacctgtcccgcggatttgttccagtccaactacagcgacccaccctaacagagatgaccaacacaaccaacgcggccgccgctaccggacttacatctaccacaaatacaccccaagtttctgcctttgtcaataactgggataacttgggcatgtggtggttctccatagcgcttatgtttgtatgccttattattatgtggctcatctgctgcctaaagcgcaaacgcgcccgaccacccatctatagtcccatcattgtgctacacccaaacaatgatggaatccatagattggacggactgaaacacatgttcttttctcttacagtatgattaaatgagacatgattcctcgagtttttatattactgacccttgttgcgcttttttgtgcgtgctccacattggctgcggtttctcacatcgaagtagactgcattccagccttcacagtctatttgctttacggatttgtcaccctcacgctcatctgcagcctcatcactgtggtcatcgcctttatccagtgcattgactgggtctgtgtgcgctttgcatatctcagacaccatccccagtacagggacaggactatagctgagcttcttagaattctttaattatgaaatttactgtgacttttctgctgattatttgcaccctatctgcgttttgttccccgacctccaagcctcaaagacatatatcatgcagattcactcgtatatggaatattccaagttgctacaatgaaaaaagcgatctttccgaagcctggttatatgcaatcatctctgttatggtgttctgcagtaccatcttagccctagctatatatccctaccttgacattggctggaaacgaatagatgccatgaaccacccaactttccccgcgcccgctatgcttccactgcaacaagttgttgccggcggctttgtcccagccaatcagcctcgccccacttctcccacccccactgaaatcagctactttaatctaacaggaggagatgactgacaccctagatctagaaatggacggaattattacagagcagcgcctgctagaaagacgcagggcagcggccgagcaacagcgcatgaatcaagagctccaagacatggttaacttgcaccagtgcaaaaggggtatcttttgtctggtaaagcaggccaaagtcacctacgacagtaataccaccggacaccgccttagctacaagttgccaaccaagcgtcagaaattggtggtcatggtgggagaaaagcccattaccataactcagcactcggtagaaaccgaaggctgcattcactcaccttgtcaaggacctgaggatctctgcacccttattaagaccctgtgcggtctcaaagatcttattccctttaactaataaaaaaaaataataaagcatcacttacttaaaatcagttagcaaatttctgtccagtttattcagcagcacctccttgccctcctcccagctctggtattgcagcttcctcctggctgcaaactttctccacaatctaaatggaatgtcagtttcctcctgttcctgtccatccgcacccactatcttcatgttgttgcagatgaagcgcgcaagaccgtctgaagataccttcaaccccgtgtatccatatgacacggaaaccggtcctccaactgtgccttttcttactcctccctttgtatcccccaatgggtttcaagagagtccccctggggtactctctttgcgcctatccgaacctctagttacctccaatggcatgcttgcgctcaaaatgggcaacggcctctctctggacgaggccggcaaccttacctcccaaaatgtaaccactgtgagcccacctctccgaggagacaagtcaaacataaacctggaaatatctgcacccctcacagttacctcagaagccctaactgtggctgccgccgcacctctaatggtcgcgggcaacacactcaccatgcaatcacaggccccgctaaccgtgcacgactccaaacttagcattgccacccaaggacccctcacagtgtcagaaggaaagctagccctgcaaacatcaggccccctcaccaccaccgatagcagtacccttactatcactgcctcaccccctctaactactgccactggtagcttgggcattgacttgaaagagcccatttatacacaaaatggaaaactaggactaaagtacggggctcctttgcatgtaacagacgacctaaacactttgaccgtagcaactggtccaggtgtgactattaataatacttccttgcaaactaaagttactggagccttgggttttgattcacaaggcaatatgcaacttaatgtagcaggaggactaaggattgattctcaaaacagacgccttatacttgatgttagttatccgtttgatgctcaaaaccaactaaatctaagactaggacagggccctctttttataaactcagcccacaacttggatattaactacaacaaaggcctttacttgtttacagcttcaaacaattccaaaaagcttgaggttaacctaagcactgccaaggggttgatgtttgacgctacagccatagccattaatgcaggagatgggcttgaatttggttcacctaatgcaccaaacacaaatcccctcaaaacaaaaattggccatggcctagaatttgattcaaacaaggctatggttcctaaactaggaactggccttagttttgacagcacaggtgccattacagtaggaaacaaaaataatgataagctaactttgtggaccacaccagctccatctcctaactgtagactaaatgcagagaaagatgctaaactcactttggtcttaacaaaatgtggcagtcaaatacttgctacagtttcagttttggctgttaaaggcagtttggctccaatatctggaacagttcaaagtgctcatcttattataagatttgacgaaaatggagtgctactaaacaattccttcctggacccagaatattggaactttagaaatggagatcttactgaaggcacagcctatacaaacgctgttggatttatgcctaacctatcagcttatccaaaatctcacggtaaaactgccaaaagtaacattgtcagtcaagtttacttaaacggagacaaaactaaacctgtaacactaaccattacactaaacggtacacaggaaacaggagacacaactccaagtgcatactctatgtcattttcatgggactggtctggccacaactacattaatgaaatatttgccacatcctcttacactttttcatacattgcccaagaataaagaatcgtttgtgttatgtttcaacgtgtttatttttcaattgcagaaaatttcaagtcatttttcattcagtagtatagccccaccaccacatagcttatacagatcaccgtaccttaatcaaactcacagaaccctagtattcaacctgccacctccctcccaacacacagagtacacagtcctttctccccggctggccttaaaaagcatcatatcatgggtaacagacatattcttaggtgttatattccacacggtttcctgtcgagccaaacgctcatcagtgatattaataaactccccgggcagctcacttaagttcatgtcgctgtccagctgctgagccacaggctgctgtccaacttgcggttgcttaacgggcggcgaaggagaagtccacgcctacatgggggtagagtcataatcgtgcatcaggatagggcggtggtgctgcagcagcgcgcgaataaactgctgccgccgccgctccgtcctgcaggaatacaacatggcagtggtctcctcagcgatgattcgcaccgcccgcagcataaggcgccttgtcctccgggcacagcagcgcaccctgatctcacttaaatcagcacagtaactgcagcacagcaccacaatattgttcaaaatcccacagtgcaaggcgctgtatccaaagctcatggcggggaccacagaacccacgtggccatcataccacaagcgcaggtagattaagtggcgacccctcataaacacgctggacataaacattacctcttttggcatgttgtaattcaccacctcccggtaccatataaacctctgattaaacatggcgccatccaccaccatcctaaaccagctggccaaaacctgcccgccggctatacactgcagggaaccgggactggaacaatgacagtggagagcccaggactcgtaaccatggatcatcatgctcgtcatgatatcaatgttggcacaacacaggcacacgtgcatacacttcctcaggattacaagctcctcccgcgttagaaccatatcccagggaacaacccattcctgaatcagcgtaaatcccacactgcagggaagacctcgcacgtaactcacgttgtgcattgtcaaagtgttacattcgggcagcagcggatgatcctccagtatggtagcgcgggtttctgtctcaaaaggaggtagacgatccctactgtacggagtgcgccgagacaaccgagatcgtgttggtcgtagtgtcatgccaaatggaacgccggacgtagtcatatttcctgaagcaaaaccaggtgcgggcgtgacaaacagatctgcgtctccggtctcgccgcttagatcgctctgtgtagtagttgtagtatatccactctctcaaagcatccaggcgccccctggcttcgggttctatgtaaactccttcatgcgccgctgccctgataacatccaccaccgcagaataagccacacccagccaacctacacattcgttctgcgagtcacacacgggaggagcgggaagagctggaagaaccatgtttttttttttattccaaaagattatccaaaacctcaaaatgaagatctattaagtgaacgcgctcccctccggtggcgtggtcaaactctacagccaaagaacagataatggcatttgtaagatgttgcacaatggcttccaaaaggcaaacggccctcacgtccaagtggacgtaaaggctaaacccttcagggtgaatctcctctataaacattccagcaccttcaaccatgcccaaataattctcatctcgccaccttctcaatatatctctaagcaaatcccgaatattaagtccggccattgtaaaaatctgctccagagcgccctccaccttcagcctcaagcagcgaatcatgattgcaaaaattcaggttcctcacagacctgtataagattcaaaagcggaacattaacaaaaataccgcgatcccgtaggtcccttcgcagggccagctgaacataatcgtgcaggtctgcacggaccagcgcggccacttccccgccaggaaccatgacaaaagaacccacactgattatgacacgcatactcggagctatgctaaccagcgtagccccgatgtaagcttgttgcatgggcggcgatataaaatgcaaggtgctgctcaaaaaatcaggcaaagcctcgcgcaaaaaagaaagcacatcgtagtcatgctcatgcagataaaggcaggtaagctccggaaccaccacagaaaaagacaccatttttctctcaaacatgtctgcgggtttctgcataaacacaaaataaaataacaaaaaaacatttaaacattagaagcctgtcttacaacaggaaaaacaacccttataagcataagacggactacggccatgccggcgtgaccgtaaaaaaactggtcaccgtgattaaaaagcaccaccgacagctcctcggtcatgtccggagtcataatgtaagactcggtaaacacatcaggttgattcacatcggtcagtgctaaaaagcgaccgaaatagcccgggggaatacatacccgcaggcgtagagacaacattacagcccccataggaggtataacaaaattaataggagagaaaaacacataaacacctgaaaaaccctcctgcctaggcaaaatagcaccctcccgctccagaacaacatacagcgcttccacagcggcagccataacagtcagccttaccagtaaaaaagaaaacctattaaaaaaacaccactcgacacggcaccagctcaatcagtcacagtgtaaaaaagggccaagtgcagagcgagtatatataggactaaaaaatgacgtaacggttaaagtccacaaaaaacacccagaaaaccgcacgcgaacctacgcccagaaacgaaagccaaaaaacccacaacttcctcaaatcgtcacttccgttttcccacgttacgtcacttcccattttaagaaaactacaattcccaacacatactagttactccgccctaaaacctacgtcacccgccccgttcccacgccccgcgccacgtcacaaactccaccccctcattatcatattggcttcaatccaaaataaggtatattattgatgatgt

SEQ ID NO: 5 - DNA, 36090 bp, Artificial Sequence
  ICOVIR15K-QD
catcatcaataatataccttattttggattgaagccaatatgataatgagggggtggagtttgtgacgtggcgcggggcgtgggaacggggcgggtgacgtagtagtgtggcggaagtgtgatgttgcaagtgtggcggaacacatgtaagcgacggatgtggcaaaagtgacgtttttggtgtgcgccggtgtacacaggaagtgacaattttcgcgcggttttaggcggatgttgtagtaaatttgggcgtaaccgagtaagatttggccattttcgcgggaaaactgaataagaggaagtgaaatctgaataattttgtgttactcatagcgcgtaatatttgtctagggccgcggggactttgaccgtttacgtggagactcgcccaggtgtttttctcaggtgttttccgcgtacgtcggcggctcgtggctctttcgcggcaaaaaggatttggcgcgtaaaagtggttcgagtacgtcggcggctcgtggctctttcgcggcaaaaaggatttggcgcgtaaaagtggttcgaagtacgtcgaccacaaaccccgcccagcgtcttgtcattggcgtcgacgctgtacggggtcaaagttggcgttttattattatagtcagctgacgtgtagtgtatttatacccggtgagttcctcaagaggccactcttgagtgccagcgagtagagttttctcctccgagccgctccgacaccgggactgaaaatgagacatattatctgccacggaggtgttattaccgaagaaatggccgccagtcttttggaccagctgatcgaagaggtactggctgataatcttccacctcctagccattttgaaccacctacccttcacgaactgtatgatttagacgtgacggcccccgaagatcccaacgaggaggcggtttcgcagatttttcccgactctgtaatgttggcggtgcaggaagggattgacttactcacttttccgccggcgcccggttctccggagccgcctcacctttcccggcagcccgagcagccggagcagagagccttgggtccggtttctatgccaaaccttgtaccggaggtgatcgatccacccagtgacgacgaggatgaagagggtgaggagtttgtgttagattatgtggagcaccccgggcacggttgcaggtcttgtcattatcaccggaggaatacgggggacccagatattatgtgttcgctttgctatatgaggacctgtggcatgtttgtctacagtaagtgaaaattatgggcagtgggtgatagagtggtgggtttggtgtggtaattttttttttaatttttacagttttgtggtttaaagaattttgtattgtgatttttttaaaaggtcctgtgtctgaacctgagcctgagcccgagccagaaccggagcctgcaagacctacccgccgtcctaaaatggcgcctgctatcctgagacgcccgacatcacctgtgtccagagaatgcaatagtagtacggatagctgtgactccggtccttctaacacacctcctgagatacacccggtggtcccgctgtgccccattaaaccagttgccgtgagagttggtgggcgtcgccaggctgtggaatgtatcgaggacttgcttaacgagcctgggcaacctttggacttgagctgtaaacgccccaggccataaggtgtaaacctgtgattgcgtgtgtggttaacgcctttgtttgctgaatgagttgatgtaagtttaataaagggtgagataatgtttaacttgcatggcgtgttaaatggggcggggcttaaagggtatataatgcgccgtgggctaatcttggttacatctgacctcatggaggcttgggagtgtttggaagatttttctgctgtgcgtaacttgctggaacagagctctaacagtacctcttggttttggaggtttctgtggggctcatcccaggcaaagttagtctgcagaattaaggaggattacaagtgggaatttgaagagcttttgaaatcctgtggtgagctgtttgattctttgaatctgggtcaccaggcgcttttccaagagaaggtcatcaagactttggatttttccacaccggggcgcgctgcggctgctgttgcttttttgagttttataaaggataaatggagcgaagaaacccatctgagcggggggtacctgctggattttctggccatgcatctgtggagagcggttgtgagacacaagaatcgcctgctactgttgtcttccgtccgcccggcgataataccgacggaggagcagcagcagcagcaggaggaagccaggcggcggcggcaggagcagagcccatggaacccgagagccggcctggaccctcgggaatgaatgttgtacaggtggctgaactgtatccagaactgagacgcattttgacaattacagaggatgggcaggggctaaagggggtaaagagggagcggggggcttgtgaggctacagaggaggctaggaatctagcttttagcttaatgaccagacaccgtcctgagtgtattacttttcaacagatcaaggataattgcgctaatgagcttgatctgctggcgcagaagtattccatagagcagctgaccacttactggctgcagccaggggatgattttgaggaggctattagggtatatgcaaaggtggcacttaggccagattgcaagtacaagatcagcaaacttgtaaatatcaggaattgttgctacatttctgggaacggggccgaggtggagatagatacggaggatagggtggcctttagatgtagcatgataaatatgtggccgggggtgcttggcatggacggggtggttattatgaatgtaaggtttactggccccaattttagcggtacggttttcctggccaataccaaccttatcctacacggtgtaagcttctatgggtttaacaatacctgtgtggaagcctggaccgatgtaagggttcggggctgtgccttttactgctgctggaagggggtggtgtgtcgccccaaaagcagggcttcaattaagaaatgcctctttgaaaggtgtaccttgggtatcctgtctgagggtaactccagggtgcgccacaatgtggcctccgactgtggttgcttcatgctagtgaaaagcgtggctgtgattaagcataacatggtatgtggcaactgcgaggacagggcctctcagatgctgacctgctcggacggcaactgtcacctgctgaagaccattcacgtagccagccactctcgcaaggcctggccagtgtttgagcataacatactgacccgctgttccttgcatttgggtaacaggaggggggtgttcctaccttaccaatgcaatttgagtcacactaagatattgcttgagcccgagagcatgtccaaggtgaacctgaacggggtgtttgacatgaccatgaagatctggaaggtgctgaggtacgatgagacccgcaccaggtgcagaccctgcgagtgtggcggtaaacatattaggaaccagcctgtgatgctggatgtgaccgaggagctgaggcccgatcacttggtgctggcctgcacccgcgctgagtttggctctagcgatgaagatacagattgaggtactgaaatgtgtgggcgtggcttaagggtgggaaagaatatataaggtgggggtcttatgtagttttgtatctgttttgcagcagccgccgccgccatgagcaccaactcgtttgatggaagcattgtgagctcatatttgacaacgcgcatgcccccatgggccggggtgcgtcagaatgtgatgggctccagcattgatggtcgccccgtcctgcccgcaaactctactaccttgacctacgagaccgtgtctggaacgccgttggagactgcagcctccgccgccgcttcagccgctgcagccaccgcccgcgggattgtgactgactttgctttcctgagcccgcttgcaagcagtgcagcttcccgttcatccgcccgcgatgacaagttgacggctcttttggcacaattggattctttgacccgggaacttaatgtcgtttctcagcagctgttggatctgcgccagcaggtttctgccctgaaggcttcctcccctcccaatgcggtttaaaacataaataaaaaaccagactctgtttggatttggatcaagcaagtgtcttgctgtctttatttaggggttttgcgcgcgcggtaggcccgggaccagcggtctcggtcgttgagggtcctgtgtattttttccaggacgtggtaaaggtgactctggatgttcagatacatgggcataagcccgtctctggggtggaggtagcaccactgcagagcttcatgctgcggggtggtgttgtagatgatccagtcgtagcaggagcgctgggcgtggtgcctaaaaatgtctttcagtagcaagctgattgccaggggcaggcccttggtgtaagtgtttacaaagcggttaagctgggatgggtgcatacgtggggatatgagatgcatcttggactgtatttttaggttggctatgttcccagccatatccctccggggattcatgttgtgcagaaccaccagcacagtgtatccggtgcacttgggaaatttgtcatgtagcttagaaggaaatgcgtggaagaacttggagacgcccttgtgacctccaagattttccatgcattcgtccataatgatggcaatgggcccacgggcggcggcctgggcgaagatatttctgggatcactaacgtcatagttgtgttccaggatgagatcgtcataggccatttttacaaagcgcgggcggagggtgccagactgcggtataatggttccatccggcccaggggcgtagttaccctcacagatttgcatttcccacgctttgagttcagatggggggatcatgtctacctgcggggcgatgaagaaaacggtttccggggtaggggagatcagctgggaagaaagcaggttcctgagcagctgcgacttaccgcagccggtgggcccgtaaatcacacctattaccgggtgcaactggtagttaagagagctgcagctgccgtcatccctgagcaggggggccacttcgttaagcatgtccctgactcgcatgttttccctgaccaaatccgccagaaggcgctcgccgcccagcgatagcagttcttgcaaggaagcaaagtttttcaacggtttgagaccgtccgccgtaggcatgcttttgagcgtttgaccaagcagttccaggcggtcccacagctcggtcacctgctctacggcatctcgatccagcatatctcctcgtttcgcgggttggggcggctttcgctgtacggcagtagtcggtgctcgtccagacgggccagggtcatgtctttccacgggcgcagggtcctcgtcagcgtagtctgggtcacggtgaaggggtgcgctccgggctgcgcgctggccagggtgcgcttgaggctggtcctgctggtgctgaagcgctgccggtcttcgccctgcgcgtcggccaggtagcatttgaccatggtgtcatagtccagcccctccgcggcgtggcccttggcgcgcagcttgcccttggaggaggcgccgcacgaggggcagtgcagacttttgagggcgtagagcttgggcgcgagaaataccgattccggggagtaggcatccgcgccgcaggccccgcagacggtctcgcattccacgagccaggtgagctctggccgttcggggtcaaaaaccaggtttcccccatgctttttgatgcgtttcttacctctggtttccatgagccggtgtccacgctcggtgacgaaaaggctgtccgtgtccccgtatacagacttgagaggcctgtcctcgagcggtgttccgcggtcctcctcgtatagaaactcggaccactctgagacaaaggctcgcgtccaggccagcacgaaggaggctaagtgggaggggtagcggtcgttgtccactagggggtccactcgctccagggtgtgaagacacatgtcgccctcttcggcatcaaggaaggtgattggtttgtaggtgtaggccacgtgaccgggtgttcctgaaggggggctataaaagggggtgggggcgcgttcgtcctcactctcttccgcatcgctgtctgcgagggccagctgttggggtgagtactccctctgaaaagcgggcatgacttctgcgctaagattgtcagtttccaaaaacgaggaggatttgatattcacctggcccgcggtgatgcctttgagggtggccgcatccatctggtcagaaaagacaatctttttgttgtcaagcttggtggcaaacgacccgtagagggcgttggacagcaacttggcgatggagcgcagggtttggtttttgtcgcgatcggcgcgctccttggccgcgatgtttagctgcacgtattcgcgcgcaacgcaccgccattcgggaaagacggtggtgcgctcgtcgggcaccaggtgcacgcgccaaccgcggttgtgcagggtgacaaggtcaacgctggtggctacctctccgcgtaggcgctcgttggtccagcagaggcggccgcccttgcgcgagcagaatggcggtagggggtctagctgcgtctcgtccggggggtctgcgtccacggtaaagaccccgggcagcaggcgcgcgtcgaagtagtctatcttgcatccttgcaagtctagcgcctgctgccatgcgcgggcggcaagcgcgcgctcgtatgggttgagtgggggaccccatggcatggggtgggtgagcgcggaggcgtacatgccgcaaatgtcgtaaacgtagaggggctctctgagtattccaagatatgtagggtagcatcttccaccgcggatgctggcgcgcacgtaatcgtatagttcgtgcgagggagcgaggaggtcgggaccgaggttgctacgggcgggctgctctgctcggaagactatctgcctgaagatggcatgtgagttggatgatatggttggacgctggaagacgttgaagctggcgtctgtgagacctaccgcgtcacgcacgaaggaggcgtaggagtcgcgcagcttgttgaccagctcggcggtgacctgcacgtctagggcgcagtagtccagggtttccttgatgatgtcatacttatcctgtcccttttttttccacagctcgcggttgaggacaaactcttcgcggtctttccagtactcttggatcggaaacccgtcggcctccgaacggtaagagcctagcatgtagaactggttgacggcctggtaggcgcagcatcccttttctacgggtagcgcgtatgcctgcgcggccttccggagcgaggtgtgggtgagcgcaaaggtgtccctgaccatgactttgaggtactggtatttgaagtcagtgtcgtcgcatccgccctgctcccagagcaaaaagtccgtgcgctttttggaacgcggatttggcagggcgaaggtgacatcgttgaagagtatctttcccgcgcgaggcataaagttgcgtgtgatgcggaagggtcccggcacctcggaacggttgttaattacctgggcggcgagcacgatctcgtcaaagccgttgatgttgtggcccacaatgtaaagttccaagaagcgcgggatgcccttgatggaaggcaattttttaagttcctcgtaggtgagctcttcaggggagctgagcccgtgctctgaaagggcccagtctgcaagatgagggttggaagcgacgaatgagctccacaggtcacgggccattagcatttgcaggtggtcgcgaaaggtcctaaactggcgacctatggccattttttctggggtgatgcagtagaaggtaagcgggtcttgttcccagcggtcccatccaaggttcgcggctaggtctcgcgcggcagtcactagaggctcatctccgccgaacttcatgaccagcatgaagggcacgagctgcttcccaaaggcccccatccaagtataggtctctacatcgtaggtgacaaagagacgctcggtgcgaggatgcgagccgatcgggaagaactggatctcccgccaccaattggaggagtggctattgatgtggtgaaagtagaagtccctgcgacgggccgaacactcgtgctggcttttgtaaaaacgtgcgcagtactggcagcggtgcacgggctgtacatcctgcacgaggttgacctgacgaccgcgcacaaggaagcagagtgggaatttgagcccctcgcctggcgggtttggctggtggtcttctacttcggctgcttgtccttgaccgtctggctgctcgaggggagttacggtggatcggaccaccacgccgcgcgagcccaaagtccagatgtccgcgcgcggcggtcggagcttgatgacaacatcgcgcagatgggagctgtccatggtctggagctcccgcggcgtcaggtcaggcgggagctcctgcaggtttacctcgcatagacgggtcagggcgcgggctagatccaggtgatacctaatttccaggggctggttggtggcggcgtcgatggcttgcaagaggccgcatccccgcggcgcgactacggtaccgcgcggcgggcggtgggccgcgggggtgtccttggatgatgcatctaaaagcggtgacgcgggcgagcccccggaggtagggggggctccggacccgccgggagagggggcaggggcacgtcggcgccgcgcgcgggcaggagctggtgctgcgcgcgtaggttgctggcgaacgcgacgacgcggcggttgatctcctgaatctggcgcctctgcgtgaagacgacgggcccggtgagcttgagcctgaaagagagttcgacagaatcaatttcggtgtcgttgacggcggcctggcgcaaaatctcctgcacgtctcctgagttgtcttgataggcgatctcggccatgaactgctcgatctcttcctcctggagatctccgcgtccggctcgctccacggtggcggcgaggtcgttggaaatgcgggccatgagctgcgagaaggcgttgaggcctccctcgttccagacgcggctgtagaccacgcccccttcggcatcgcgggcgcgcatgaccacctgcgcgagattgagctccacgtgccgggcgaagacggcgtagtttcgcaggcgctgaaagaggtagttgagggtggtggcggtgtgttctgccacgaagaagtacataacccagcgtcgcaacgtggattcgttgatatcccccaaggcctcaaggcgctccatggcctcgtagaagtccacggcgaagttgaaaaactgggagttgcgcgccgacacggttaactcctcctccagaagacggatgagctcggcgacagtgtcgcgcacctcgcgctcaaaggctacaggggcctcttcttcttcttcaatctcctcttccataagggcctccccttcttcttcttctggcggcggtgggggaggggggacacggcggcgacgacggcgcaccgggaggcggtcgacaaagcgctcgatcatctccccgcggcgacggcgcatggtctcggtgacggcgcggccgttctcgcgggggcgcagttggaagacgccgcccgtcatgtcccggttatgggttggcggggggctgccatgcggcagggatacggcgctaacgatgcatctcaacaattgttgtgtaggtactccgccgccgagggacctgagcgagtccgcatcgaccggatcggaaaacctctcgagaaaggcgtctaaccagtcacagtcgcaaggtaggctgagcaccgtggcgggcggcagcgggcggcggtcggggttgtttctggcggaggtgctgctgatgatgtaattaaagtaggcggtcttgagacggcggatggtcgacagaagcaccatgtccttgggtccggcctgctgaatgcgcaggcggtcggccatgccccaggcttcgttttgacatcggcgcaggtctttgtagtagtcttgcatgagcctttctaccggcacttcttcttctccttcctcttgtcctgcatctcttgcatctatcgctgcggcggcggcggagtttggccgtaggtggcgccctcttcctcccatgcgtgtgaccccgaagcccctcatcggctgaagcagggctaggtcggcgacaacgcgctcggctaatatggcctgctgcacctgcgtgagggtagactggaagtcatccatgtccacaaagcggtggtatgcgcccgtgttgatggtgtaagtgcagttggccataacggaccagttaacggtctggtgacccggctgcgagagctcggtgtacctgagacgcgagtaagccctcgagtcaaatacgtagtcgttgcaagtccgcaccaggtactggtatcccaccaaaaagtgcggcggcggctggcggtagaggggccagcgtagggtggccggggctccgggggcgagatcttccaacataaggcgatgatatccgtagatgtacctggacatccaggtgatgccggcggcggtggtggaggcgcgcggaaagtcgcggacgcggttccagatgttgcgcagcggcaaaaagtgctccatggtcgggacgctctggccggtcaggcgcgcgcaatcgttgacgctctagaccgtgcaaaaggagagcctgtaagcgggcactcttccgtggtctggtggataaattcgcaagggtatcatggcggacgaccggggttcgagccccgtatccggccgtccgccgtgatccatgcggttaccgcccgcgtgtcgaacccaggtgtgcgacgtcagacaacgggggagtgctccttttggcttccttccaggcgcggcggctgctgcgctagcttttttggccactggccgcgcgcagcgtaagcggttaggctggaaagcgaaagcattaagtggctcgctccctgtagccggagggttattttccaagggttgagtcgcgggacccccggttcgagtctcggaccggccggactgcggcgaacgggggtttgcctccccgtcatgcaagaccccgcttgcaaattcctccggaaacagggacgagccccttttttgcttttcccagatgcatccggtgctgcggcagatgcgcccccctcctcagcagcggcaagagcaagagcagcggcagacatgcagggcaccctcccctcctcctaccgcgtcaggaggggcgacatccgcggttgacgcggcagcagatggtgattacgaacccccgcggcgccgggcccggcactacctggacttggaggagggcgagggcctggcgcggctaggagcgccctctcctgagcggtacccaagggtgcagctgaagcgtgatacgcgtgaggcgtacgtgccgcggcagaacctgtttcgcgaccgcgagggagaggagcccgaggagatgcgggatcgaaagttccacgcagggcgcgagctgcggcatggcctgaatcgcgagcggttgctgcgcgaggaggactttgagcccgacgcgcgaaccgggattagtcccgcgcgcgcacacgtggcggccgccgacctggtaaccgcatacgagcagacggtgaaccaggagattaactttcaaaaaagctttaacaaccacgtgcgtacgcttgtggcgcgcgaggaggtggctataggactgatgcatctgtgggactttgtaagcgcgctggagcaaaacccaaatagcaagccgctcatggcgcagctgttccttatagtgcagcacagcagggacaacgaggcattcagggatgcgctgctaaacatagtagagcccgagggccgctggctgctcgatttgataaacatcctgcagagcatagtggtgcaggagcgcagcttgagcctggctgacaaggtggccgccatcaactattccatgcttagcctgggcaagttttacgcccgcaagatataccataccccttacgttcccatagacaaggaggtaaagatcgaggggttctacatgcgcatggcgctgaaggtgcttaccttgagcgacgacctgggcgtttatcgcaacgagcgcatccacaaggccgtgagcgtgagccggcggcgcgagctcagcgaccgcgagctgatgcacagcctgcaaagggccctggctggcacgggcagcggcgatagagaggccgagtcctactttgacgcgggcgctgacctgcgctgggccccaagccgacgcgccctggaggcagctggggccggacctgggctggcggtggcacccgcgcgcgctggcaacgtcggcggcgtggaggaatatgacgaggacgatgagtacgagccagaggacggcgagtactaagcggtgatgtttctgatcagatgatgcaagacgcaacggacccggcggtgcgggcggcgctgcagagccagccgtccggccttaactccacggacgactggcgccaggtcatggaccgcatcatgtcgctgactgcgcgcaatcctgacgcgttccggcagcagccgcaggccaaccggctctccgcaattctggaagcggtggtcccggcgcgcgcaaaccccacgcacgagaaggtgctggcgatcgtaaacgcgctggccgaaaacagggccatccggcccgacgaggccggcctggtctacgacgcgctgcttcagcgcgtggctcgttacaacagcggcaacgtgcagaccaacctggaccggctggtgggggatgtgcgcgaggccgtggcgcagcgtgagcgcgcgcagcagcagggcaacctgggctccatggttgcactaaacgccttcctgagtacacagcccgccaacgtgccgcggggacaggaggactacaccaactttgtgagcgcactgcggctaatggtgactgagacaccgcaaagtgaggtgtaccagtctgggccagactattttttccagaccagtagacaaggcctgcagaccgtaaacctgagccaggctttcaaaaacttgcaggggctgtggggggtgcgggctcccacaggcgaccgcgcgaccgtgtctagcttgctgacgcccaactcgcgcctgttgctgctgctaatagcgcccttcacggacagtggcagcgtgtcccgggacacatacctaggtcacttgctgacactgtaccgcgaggccataggtcaggcgcatgtggacgagcatactttccaggagattacaagtgtcagccgcgcgctggggcaggaggacacgggcagcctggaggcaaccctaaactacctgctgaccaaccggcggcagaagatcccctcgttgcacagtttaaacagcgaggaggagcgcattttgcgctacgtgcagcagagcgtgagccttaacctgatgcgcgacggggtaacgcccagcgtggcgctggacatgaccgcgcgcaacatggaaccgggcatgtatgcctcaaaccggccgtttatcaaccgcctaatggactacttgcatcgcgcggccgccgtgaaccccgagtatttcaccaatgccatcttgaacccgcactggctaccgccccctggtttctacaccgggggattcgaggtgcccgagggtaacgatggattcctctgggacgacatagacgacagcgtgttttccccgcaaccgcagaccctgctagagttgcaacagcgcgagcaggcagaggcggcgctgcgaaaggaaagcttccgcaggccaagcagcttgtccgatctaggcgctgcggccccgcggtcagatgctagtagcccatttccaagcttgatagggtctcttaccagcactcgcaccacccgcccgcgcctgctgggcgaggaggagtacctaaacaactcgctgctgcagccgcagcgcgaaaaaaacctgcctccggcatttcccaacaacgggatagagagcctagtggacaagatgagtagatggaagacgtacgcgcaggagcacagggacgtgccaggcccgcgcccgcccacccgtcgtcaaaggcacgaccgtcagcggggtctggtgtgggaggacgatgactcggcagacgacagcagcgtcctggatttgggagggagtggcaacccgtttgcgcaccttcgccccaggctggggagaatgttttaaaaaaaaaaaagcatgatgcaaaataaaaaactcaccaaggccatggcaccgagcgttggttttcttgtattccccttagtatgcggcgcgcggcgatgtatgaggaaggtcctcctccctcctacgagagtgtggtgagcgcggcgccagtggcggcggcgctgggttctcccttcgatgctcccctggacccgccgtttgtgcctccgcggtacctgcggcctaccggggggagaaacagcatccgttactctgagttggcacccctattcgacaccacccgtgtgtacctggtggacaacaagtcaacggatgtggcatccctgaactaccagaacgaccacagcaactttctgaccacggtcattcaaaacaatgactacagcccgggggaggcaagcacacagaccatcaatcttgacgaccggtcgcactggggcggcgacctgaaaaccatcctgcataccaacatgccaaatgtgaacgagttcatgtttaccaataagtttaaggcgcgggtgatggtgtcgcgcttgcctactaaggacaatcaggtggagctgaaatacgagtgggtggagttcacgctgcccgagggcaactactccgagaccatgaccatagaccttatgaacaacgcgatcgtggagcactacttgaaagtgggcagacagaacggggttctggaaagcgacatcggggtaaagtttgacacccgcaacttcagactggggtttgaccccgtcactggtcttgtcatgcctggggtatatacaaacgaagccttccatccagacatcattttgctgccaggatgcggggtggacttcacccacagccgcctgagcaacttgttgggcatccgcaagcggcaacccttccaggagggctttaggatcacctacgatgatctggagggtggtaacattcccgcactgttggatgtggacgcctaccaggcgagcttgaaagatgacaccgaacagggcgggggtggcgcaggcggcagcaacagcagtggcagcggcgcggaagagaactccaacgcggcagccgcggcaatgcagccggtggaggacatgaacgatcatgccattcgcggcgacacctttgccacacgggctgaggagaagcgcgctgaggccgaagcagcggccgaagctgccgcccccgctgcgcaacccgaggtcgagaagcctcagaagaaaccggtgatcaaacccctgacagaggacagcaagaaacgcagttacaacctaataagcaatgacagcaccttcacccagtaccgcagctggtaccttgcatacaactacggcgaccctcagaccggaatccgctcatggaccctgctttgcactcctgacgtaacctgcggctcggagcaggtctactggtcgttgccagacatgatgcaagaccccgtgaccttccgctccacgcgccagatcagcaactttccggtggtgggcgccgagctgttgcccgtgcactccaagagcttctacaacgaccaggccgtctactcccaactcatccgccagtttacctctctgacccacgtgttcaatcgctttcccgagaaccagattttggcgcgcccgccagcccccaccatcaccaccgtcagtgaaaacgttcctgctctcacagatcacgggacgctaccgctgcgcaacagcatcggaggagtccagcgagtgaccattactgacgccagacgccgcacctgcccctacgtttacaaggccctgggcatagtctcgccgcgcgtcctatcgagccgcactttttgagcaagcatgtccatccttatatcgcccagcaataacacaggctggggcctgcgcttcccaagcaagatgtttggcggggccaagaagcgctccgaccaacacccagtgcgcgtgcgcgggcactaccgcgcgccctggggcgcgcacaaacgcggccgcactgggcgcaccaccgtcgatgacgccatcgacgcggtggtggaggaggcgcgcaactacacgcccacgccgccaccagtgtccacagtggacgcggccattcagaccgtggtgcgcggagcccggcgctatgctaaaatgaagagacggcggaggcgcgtagcacgtcgccaccgccgccgacccggcactgccgcccaacgcgcggcggcggccctgcttaaccgcgcacgtcgcaccggccgacgggcggccatgcgggccgctcgaaggctggccgcgggtattgtcactgtgccccccaggtccaggcgacgagcggccgccgcagcagccgcggccattagtgctatgactcagggtcgcaggggcaacgtgtattgggtgcgcgactcggttagcggcctgcgcgtgcccgtgcgcacccgccccccgcgcaactagattgcaagaaaaaactacttagactcgtactgttgtatgtatccagcggcggcggcgcgcaacgaagctatgtccaagcgcaaaatcaaagaagagatgctccaggtcatcgcgccggagatctatggccccccgaagaaggaagagcaggattacaagccccgaaagctaaagcgggtcaaaaagaaaaagaaagatgatgatgatgaacttgacgacgaggtggaactgctgcacgctaccgcgcccaggcgacgggtacagtggaaaggtcgacgcgtaaaacgtgttttgcgacccggcaccaccgtagtctttacgcccggtgagcgctccacccgcacctacaagcgcgtgtatgatgaggtgtacggcgacgaggacctgcttgagcaggccaacgagcgcctcggggagtttgcctacggaaagcggcataaggacatgctggcgttgccgctggacgagggcaacccaacacctagcctaaagcccgtaacactgcagcaggtgctgcccgcgcttgcaccgtccgaagaaaagcgcggcctaaagcgcgagtctggtgacttggcacccaccgtgcagctgatggtacccaagcgccagcgactggaagatgtcttggaaaaaatgaccgtggaacctgggctggagcccgaggtccgcgtgcggccaatcaagcaggtggcgccgggactgggcgtgcagaccgtggacgttcagatacccactaccagtagcaccagtattgccaccgccacagagggcatggagacacaaacgtccccggttgcctcagcggtggcggatgccgcggtgcaggcggtcgctgcggccgcgtccaagacctctacggaggtgcaaacggacccgtggatgtttcgcgtttcagccccccggcgcccgcgcggttcgaggaagtacggcgccgccagcgcgctactgcccgaatatgccctacatccttccattgcgcctacccccggctatcgtggctacacctaccgccccagaagacgagcaactacccgacgccgaaccaccactggaacccgccgccgccgtcgccgtcgccagcccgtgctggccccgatttccgtgcgcagggtggctcgcgaaggaggcaggaccctggtgctgccaacagcgcgctaccaccccagcatcgtttaaaagccggtctttgtggttcttgcagatatggccctcacctgccgcctccgtttcccggtgccgggattccgaggaagaatgcaccgtaggaggggcatggccggccacggcctgacgggcggcatgcgtcgtgcgcaccaccggcggcggcgcgcgtcgcaccgtcgcatgcgcggcggtatcctgcccctccttattccactgatcgccgcggcgattggcgccgtgcccggaattgcatccgtggccttgcaggcgcagagacactgattaaaaacaagttgcatgtggaaaaatcaaaataaaaagtctggactctcacgctcgcttggtcctgtaactattttgtagaatggaagacatcaactttgcgtctctggccccgcgacacggctcgcgcccgttcatgggaaactggcaagatatcggcaccagcaatatgagcggtggcgccttcagctggggctcgctgtggagcggcattaaaaatttcggttccaccgttaagaactatggcagcaaggcctggaacagcagcacaggccagatgctgagggataagttgaaagagcaaaatttccaacaaaaggtggtagatggcctggcctctggcattagcggggtggtggacctggccaaccaggcagtgcaaaataagattaacagtaagcttgatccccgccctcccgtagaggagcctccaccggccgtggagacagtgtctccagaggggcgtggcgaaaagcgtccgcgccccgacagggaagaaactctggtgacgcaaatagacgagcctccctcgtacgaggaggcactaaagcaaggcctgcccaccacccgtcccatcgcgcccatggctaccggagtgctgggccagcacacacccgtaacgctggacctgcctccccccgccgacacccagcagaaacctgtgctgccaggcccgaccgccgttgttgtaacccgtcctagccgcgcgtccctgcgccgcgccgccagcggtccgcgatcgttgcggcccgtagccagtggcaactggcaaagcacactgaacagcatcgtgggtctgggggtgcaatccctgaagcgccgacgatgcttctgaatagctaacgtgtcgtatgtgtgtcatgtatgcgtccatgtcgccgccagaggagctgctgagccgccgcgcgcccgctttccaagatggctaccccttcgatgatgccgcagtggtcttacatgcacatctcgggccaggacgcctcggagtacctgagccccgggctggtgcagtttgcccgcgccaccgagacgtacttcagcctgaataacaagtttagaaaccccacggtggcgcctacgcacgacgtgaccacagaccggtcccagcgtttgacgctgcggttcatccctgtggaccgtgaggatactgcgtactcgtacaaggcgcggttcaccctagctgtgggtgataaccgtgtgctggacatggcttccacgtactttgacatccgcggcgtgctggacaggggccctacttttaagccctactctggcactgcctacaacgccctggctcccaagggtgccccaaatccttgcgaatgggatgaagctgctactgctcttgaaataaacctagaagaagaggacgatgacaacgaagacgaagtagacgagcaagctgagcagcaaaaaactcacgtatttgggcaggcgccttattctggtataaatattacaaaggagggtattcaaataggtgtcgaaggtcaaacacctaaatatgccgataaaacatttcaacctgaacctcaaataggagaatctcagtggtacgaaactgaaattaatcatgcagctgggagagtccttaaaaagactaccccaatgaaaccatgttacggttcatatgcaaaacccacaaatgaaaatggagggcaaggcattcttgtaaagcaacaaaatggaaagctagaaagtcaagtggaaatgcaatttttctcaactactgaggcgaccgcaggcaatggtgataacttgactcctaaagtggtattgtacagtgaagatgtagatatagaaaccccagacactcatatttcttacatgcccactattaaggaaggtaactcacgagaactaatgggccaacaatctatgcccaacaggcctaattacattgcttttagggacaattttattggtctaatgtattacaacagcacgggtaatatgggtgttctggcgggccaagcatcgcagttgaatgctgttgtagatttgcaagacagaaacacagagctttcataccagcttttgcttgattccattggtgatagaaccaggtacttttctatgtggaatcaggctgttgacagctatgatccagatgttagaattattgaaaatcatggaactgaagatgaacttccaaattactgctttccactgggaggtgtgattaatacagagactcttaccaaggtaaaacctaaaacaggtcaggaaaatggatgggaaaaagatgctacagaattttcagataaaaatgaaataagagttggaaataattttgccatggaaatcaatctaaatgccaacctgtggagaaatttcctgtactccaacatagcgctgtatttgcccgacaagctaaagtacagtccttccaacgtaaaaatttctgataacccaaacacctacgactacatgaacaagcgagtggtggctcccgggttagtggactgctacattaaccccggagcacgctggtcccttgactatatggacaacgtcaacccatttaaccaccaccgcaatgctggcctgcgctaccgctcaatgttgctgggcaatggtcgctatgtgcccttccacatccaggtgcctcagaagttctttgccattaaaaacctccttctcctgccgggctcatacacctacgagtggaacttcaggaaggatgttaacatggttctgcagagctccctaggaaatgacctaagggttgacggagccagcattaagtttgatagcatttgcctttacgccaccttcttccccatggcccacaacaccgcctccacgcttgaggccatgcttagaaacgacaccaacgaccagtcctttaacgactatctctccgccgccaacatgctctaccctatacccgccaacgctaccaacgtgcccatatccatcccctcccgcaactgggcggctttccgcggctgggccttcacgcgccttaagactaaggaaaccccatcactgggctcgggctacgacccttattacacctactctggctctataccctacctagatggaaccttttacctcaaccacacctttaagaaggctgccattacctttgactcttctgtcagctggcctggcaatgaccgcctgcttacccccaacgagtttgaaattaagcgctcagttgacggggagggttacaacgttgcccagtgtaacatgaccaaagactggttcctggtacaaatgctagctaactataacattggctaccagggcttctatatcccagagagctacaaggaccgcatgtactccttctttagaaacttccagcccatgagccgtcaggtggtggatgatactaaatacaaggactaccaacaggtgggcatcctacaccaacacaacaactctggatttgttggctaccttgcccccaccatgcgcgaaggacaggcctaccctgctaacttcccctatccgcttataggcaagaccgcagttgacagcattacccagaaaaagtttctttgcgatcgcaccctttggcgcatcccattctccagtaactttatgtccatgggcgcactcacagacctgggccaaaaccttctctacgccaactccgcccactccctagacatgacttttgaggtggatcccatggacgagcccacccttctttatgttttgtttgaagtctttgacaaggtccgtgtgcaccagccgcaccgcggcgtcatcgaaaccgtgtacctgcgcacgcccttctcggccggcaacgccacaacataaagaagcaagcaacatcaacaacagctgccgccatgggctccagtgagcaggaactgaaagccattgtcaaagatcttggttgtgggccatattttttgggcacctatgacaagcgctttccaggctttgtttctccacacaagctcgcctgcgccatagtcaatacggccggtcgcgagactgggggcgtacactggatggcctttgcctggaacccgcactcaaaaacatgctacctctttgagccctttggcttttctgaccagcgactcaagcaggtttaccagtttgagtacgagtcactcctgcgccgtagcgccattgcttcttcccccgaccgctgtataacgctggaaaagtccacccaaagcgtacaggggcccaactcggccgcctgtggactattctgctgcatgtttctccacgcctttgccaactggccccaaactcccatggatcacaaccccaccatgaaccttattaccggggtacccaactccatgctcaacagtccccaggtacagcccaccctgcgtcgcaaccaggaacagctctacagcttcctggagcgccactcgccctacttccgcagccacagtgcgcagattaggagcgccacttctttttgtcacttgaaaaacatgtaaaaataatgtactagagacactttcaataaaggcaaatgcttttatttgtacactctcgggtgattatttacccccacccttgccgtctgcgccgtttaaaaatcaaaggggttctgccgcgcatcgctatgcgccactggcagggacacgttgcgatactggtgtttagtgctccacttaaactcaggcacaaccatccgcggcagctcggtgaagttttcactccacaggctgcgcaccatcaccaacgcgtttagcaggtcgggcgccgatatcttgaagtcgcagttggggcctccgccctgcgcgcgcgagttgcgatacacagggttgcagcactggaacactatcagcgccgggtggtgcacgctggccagcacgctcttgtcggagatcagatccgcgtccaggtcctccgcgttgctcagggcgaacggagtcaactttggtagctgccttcccaaaaagggcgcgtgcccaggctttgagttgcactcgcaccgtagtggcatcaaaaggtgaccgtgcccggtctgggcgttaggatacagcgcctgcataaaagccttgatctgcttaaaagccacctgagcctttgcgccttcagagaagaacatgccgcaagacttgccggaaaactgattggccggacaggccgcgtcgtgcacgcagcaccttgcgtcggtgttggagatctgcaccacatttcggccccaccggttcttcacgatcttggccttgctagactgctccttcagcgcgcgctgcccgttttcgctcgtcacatccatttcaatcacgtgctccttatttatcataatgcttccgtgtagacacttaagctcgccttcgatctcagcgcagcggtgcagccacaacgcgcagcccgtgggctcgtgatgcttgtaggtcacctctgcaaacgactgcaggtacgcctgcaggaatcgccccatcatcgtcacaaaggtcttgttgctggtgaaggtcagctgcaacccgcggtgctcctcgttcagccaggtcttgcatacggccgccagagcttccacttggtcaggcagtagtttgaagttcgcctttagatcgttatccacgtggtacttgtccatcagcgcgcgcgcagcctccatgcccttctcccacgcagacacgatcggcacactcagcgggttcatcaccgtaatttcactttccgcttcgctgggctcttcctcttcctcttgcgtccgcataccacgcgccactgggtcgtcttcattcagccgccgcactgtgcgcttacctcctttgccatgcttgattagcaccggtgggttgctgaaacccaccatttgtagcgccacatcttctctttcttcctcgctgtccacgattacctctggtgatggcgggcgctcgggcttgggagaagggcgcttctttttcttcttgggcgcaatggccaaatccgccgccgaggtcgatggccgcgggctgggtgtgcgcggcaccagcgcgtcttgtgatgagtcttcctcgtcctcggactcgatacgccgcctcatccgcttttttgggggcgcccggggaggcggcggcgacggggacggggacgacacgtcctccatggttgggggacgtcgcgccgcaccgcgtccgcgctcgggggtggtttcgcgctgctcctcttcccgactggccatttccttctcctataggcagaaaaagatcatggagtcagtcgagaagaaggacagcctaaccgccccctctgagttcgccaccaccgcctccaccgatgccgccaacgcgcctaccaccttccccgtcgaggcacccccgcttgaggaggaggaagtgattatcgagcaggacccaggttttgtaagcgaagacgacgaggaccgctcagtaccaacagaggataaaaagcaagaccaggacaacgcagaggcaaacgaggaacaagtcgggcggggggacgaaaggcatggcgactacctagatgtgggagacgacgtgctgttgaagcatctgcagcgccagtgcgccattatctgcgacgcgttgcaagagcgcagcgatgtgcccctcgccatagcggatgtcagccttgcctacgaacgccacctattctcaccgcgcgtaccccccaaacgccaagaaaacggcacatgcgagcccaacccgcgcctcaacttctaccccgtatttgccgtgccagaggtgcttgccacctatcacatctttttccaaaactgcaagatacccctatcctgccgtgccaaccgcagccgagcggacaagcagctggccttgcggcagggcgctgtcatacctgatatcgcctcgctcaacgaagtgccaaaaatctttgagggtcttggacgcgacgagaagcgcgcggcaaacgctctgcaacaggaaaacagcgaaaatgaaagtcactctggagtgttggtggaactcgagggtgacaacgcgcgcctagccgtactaaaacgcagcatcgaggtcacccactttgcctacccggcacttaacctaccccccaaggtcatgagcacagtcatgagtgagctgatcgtgcgccgtgcgcagcccctggagagggatgcaaatttgcaagaacaaacagaggagggcctacccgcagttggcgacgagcagctagcgcgctggcttcaaacgcgcgagcctgccgacttggaggagcgacgcaaactaatgatggccgcagtgctcgttaccgtggagcttgagtgcatgcagcggttctttgctgacccggagatgcagcgcaagctagaggaaacattgcactacacctttcgacagggctacgtacgccaggcctgcaagatctccaacgtggagctctgcaacctggtctcctaccttggaattttgcacgaaaaccgccttgggcaaaacgtgcttcattccacgctcaagggcgaggcgcgccgcgactacgtccgcgactgcgtttacttatttctatgctacacctggcagacggccatgggcgtttggcagcagtgcttggaggagtgcaacctcaaggagctgcagaaactgctaaagcaaaacttgaaggacctatggacggccttcaacgagcgctccgtggccgcgcacctggcggacatcattttccccgaacgcctgcttaaaaccctgcaacagggtctgccagacttcaccagtcaaagcatgttgcagaactttaggaactttatcctagagcgctcaggaatcttgcccgccacctgctgtgcacttcctagcgactttgtgcccattaagtaccgcgaatgccctccgccgctttggggccactgctaccttctgcagctagccaactaccttgcctaccactctgacataatggaagacgtgagcggtgacggtctactggagtgtcactgtcgctgcaacctatgcaccccgcaccgctccctggtttgcaattcgcagctgcttaacgaaagtcaaattatcggtacctttgagctgcagggtccctcgcctgacgaaaagtccgcggctccggggttgaaactcactccggggctgtggacgtcggcttaccttcgcaaatttgtacctgaggactaccacgcccacgagattaggttctacgaagaccaatcccgcccgccaaatgcggagcttaccgcctgcgtcattacccagggccacattcttggccaattgcaagccatcaacaaagcccgccaagagtttctgctacgaaagggacggggggtttacttggacccccagtccggcgaggagctcaacccaatccccccgccgccgcagccctatcagcagcagccgcgggcccttgcttcccaggatggcacccaaaaagaagctgcagctgccgccgccacccacggacgaggaggaatactgggacagtcaggcagaggaggttttggacgaggaggaggaggacatgatggaagactgggagagcctagacgaggaagcttccgaggtcgaagaggtgtcagacgaaacaccgtcaccctcggtcgcattcccctcgccggcgccccagaaatcggcaaccggttccagcatggctacaacctccgctcctcaggcgccgccggcactgcccgttcgccgacccaaccgtagatgggacaccactggaaccagggccggtaagtccaagcagccgccgccgttagcccaagagcaacaacagcgccaaggctaccgctcatggcgcgggcacaagaacgccatagttgcttgcttgcaagactgtgggggcaacatctccttcgcccgccgctttcttctctaccatcacggcgtggccttcccccgtaacatcctgcattactaccgtcatctctacagcccatactgcaccggcggcagcggcagcggcagcaacagcagcggccacacagaagcaaaggcgaccggatagcaagactctgacaaagcccaagaaatccacagcggcggcagcagcaggaggaggagcgctgcgtctggcgcccaacgaacccgtatcgacccgcgagcttagaaacaggatttttcccactctgtatgctatatttcaacagagcaggggccaagaacaagagctgaaaataaaaaacaggtctctgcgatccctcacccgcagctgcctgtatcacaaaagcgaagatcagcttcggcgcacgctggaagacgcggaggctctcttcagtaaatactgcgcgctgactcttaaggactagtttcgcgccctttctcaaatttaagcgcgaaaactacgtcatctccagcggccacacccggcgccagcacctgtcgtcagcgccattatgagcaaggaaattcccacgccctacatgtggagttaccagccacaaatgggacttgcggctggagctgcccaagactactcaacccgaataaactacatgagcgcgggaccccacatgatatcccgggtcaacggaatccgcgcccaccgaaaccgaattctcttggaacaggcggctattaccaccacacctcgtaataaccttaatccccgtagttggcccgctgccctggtgtaccaggaaagtcccgctcccaccactgtggtacttcccagagacgcccaggccgaagttcagatgactaactcaggggcgcagcttgcgggcggctttcgtcacagggtgcggtcgcccgggcagggtataactcacctgacaatcagagggcgaggtattcagctcaacgacgagtcggtgagctcctcgcttggtctccgtccggacgggacatttcagatcggcggcgccggccgtccttcattcacgcctcgtcaggcaatcctaactctgcagacctcgtcctctgagccgcgctctggaggcattggaactctgcaatttattgaggagtttgtgccatcggtctactttaaccccttctcgggacctcccggccactatccggatcaatttattcctaactttgacgcggtaaaggactcggcggacggctacgactgaatgttaagtggagaggcagagcaactgcgcctgaaacacctggtccactgtcgccgccacaagtgctttgcccgcgactccggtgagttttgctactttgaattgcccgaggatcatatcgagggcccggcgcacggcgtccggcttaccgcccagggagagcttgcccgtagcctgattcgggagtttacccagcgccccctgctagttgagcgggacaggggaccctgtgttctcactgtgatttgcaactgtcctaaccttggattacatcaagatctttgttgccatctctgtgctgagtataataaatacagaaattaaaatatactggggctcctatcgccatcctgtaaacgccaccgtcttcacccgcccaagcaaaccaaggcgaaccttacctggtacttttaacatctctccctctgtgatttacaacagtttcaacccagacggagtgagtctacgagagaacctctccgagctcagctactccatcagaaaaaacaccaccctccttacctgccgggaacgtacgagtgcgtcaccggccgctgcaccacacctaccgcctgaccgtaaaccagactttttccggacagacctcaataactctgtttaccagaacaggaggtgagcttagaaaacccttagggtattaggccaaaggcgcagctactgtggggtttatgaacaattcaagcaactctacgggctattctaattcaggtttctctagaatcggggttggggttattctctgtcttgtgattctctttattcttatactaacgcttctctgcctaaggctcgccgcctgctgtgtgcacatttgcatttattgtcagctttttaaacgctggggtcgccacccaagatgattaggtacataatcctaggtttactcacccttgcgtcagcccacggtaccacccaaaaggtggattttaaggagccagcctgtaatgttacattcgcagctgaagctaatgagtgcaccactcttataaaatgcaccacagaacatgaaaagctgcttattcgccacaaaaacaaaattggcaagtatgctgtttatgctatttggcagccaggtgacactacagagtataatgttacagttttccagggtaaaagtcataaaacttttatgtatacttttccattttatgaaatgtgcgacattaccatgtacatgagcaaacagtataagttgtggcccccacaaaattgtgtggaaaacactggcactttctgctgcactgctatgctaattacagtgctcgctttggtctgtaccctactctatattaaatacaaaagcagacgcagctttattgaggaaaagaaaatgccttaatttactaagttacaaagctaatgtcaccactaactgctttactcgctgcttgcaaaacaaattcaaaaagttagcattataattagaataggatttaaaccccccggtcatttcctgctcaataccattcccctgaacaattgactctatgtgggatatgctccagcgctacaaccttgaagtcaggcttcctggatgtcagcatctgactttggccagcacctgtcccgcggatttgttccagtccaactacagcgacccaccctaacagagatgaccaacacaaccaacgcggccgccgctaccggacttacatctaccacaaatacaccccaagtttctgcctttgtcaataactgggataacttgggcatgtggtggttctccatagcgcttatgtttgtatgccttattattatgtggctcatctgctgcctaaagcgcaaacgcgcccgaccacccatctatagtcccatcattgtgctacacccaaacaatgatggaatccatagattggacggactgaaacacatgttcttttctcttacagtatgattaaatgagacatgattcctcgagtttttatattactgacccttgttgcgcttttttgtgcgtgctccacattggctgcggtttctcacatcgaagtagactgcattccagccttcacagtctatttgctttacggatttgtcaccctcacgctcatctgcagcctcatcactgtggtcatcgcctttatccagtgcattgactgggtctgtgtgcgctttgcatatctcagacaccatccccagtacagggacaggactatagctgagcttcttagaattctttaattatgaaatttactgtgacttttctgctgattatttgcaccctatctgcgttttgttccccgacctccaagcctcaaagacatatatcatgcagattcactcgtatatggaatattccaagttgctacaatgaaaaaagcgatctttccgaagcctggttatatgcaatcatctctgttatggtgttctgcagtaccatcttagccctagctatatatccctaccttgacattggctggaaacgaatagatgccatgaaccacccaactttccccgcgcccgctatgcttccactgcaacaagttgttgccggcggctttgtcccagccaatcagcctcgccccacttctcccacccccactgaaatcagctactttaatctaacaggaggagatgactgacaccctagatctagaaatggacggaattattacagagcagcgcctgctagaaagacgcagggcagcggccgagcaacagcgcatgaatcaagagctccaagacatggttaacttgcaccagtgcaaaaggggtatcttttgtctggtaaagcaggccaaagtcacctacgacagtaataccaccggacaccgccttagctacaagttgccaaccaagcgtcagaaattggtggtcatggtgggagaaaagcccattaccataactcagcactcggtagaaaccgaaggctgcattcactcaccttgtcaaggacctgaggatctctgcacccttattaagaccctgtgcggtctcaaagatcttattccctttaactaataaaaaaaaataataaagcatcacttacttaaaatcagttagcaaatttctgtccagtttattcagcagcacctccttgccctcctcccagctctggtattgcagcttcctcctggctgcaaactttctccacaatctaaatggaatgtcagtttcctcctgttcctgtccatccgcacccactatcttcatgttgttgcagatgaagcgcgcaagaccgtctgaagataccttcaaccccgtgtatccatatgacacggaaaccggtcctccaactgtgccttttcttactcctccctttgtatcccccaatgggtttcaagagagtccccctggggtactctctttgcgcctatccgaacctctagttacctccaatggcatgcttgcgctcaaaatgggcaacggcctctctctggacgaggccggcaaccttacctcccaaaatgtaaccactgtgagcccacctctccgaggagacaagtcaaacataaacctggaaatatctgcacccctcacagttacctcagaagccctaactgtggctgccgccgcacctctaatggtcgcgggcaacacactcaccatgcaatcacaggccccgctaaccgtgcacgactccaaacttagcattgccacccaaggacccctcacagtgtcagaaggaaagctagccctgcaaacatcaggccccctcaccaccaccgatagcagtacccttactatcactgcctcaccccctctaactactgccactggtagcttgggcattgacttgaaagagcccatttatacacaaaatggaaaactaggactaaagtacggggctcctttgcatgtaacagacgacctaaacactttgaccgtagcaactggtccaggtgtgactattaataatacttccttgcaaactaaagttactggagccttgggttttgattcacaaggcaatatgcaacttaatgtagcaggaggactaaggattgattctcaaaacagacgccttatacttgatgttagttatccgtttgatgctcaaaaccaactaaatctaagactaggacagggccctctttttataaactcagcccacaacttggatattaactacaacaaaggcctttacttgtttacagcttcaaacaattccaaaaagcttgaggttaacctaagcactgccaaggggttgatgtttgacgctacagccatagccattaatgcaggagatgggcttgaatttggttcacctaatgcaccaaacacaaatcccctcaaaacaaaaattggccatggcctagaatttgattcaaacaaggctatggttcctaaactaggaactggccttagttttgacagcacaggtgccattacagtaggaaacaaaaataatgataagctaactttgtggaccacaccagctccatctcctaactgtagactaaatgcagagaaagatgctaaactcactttggtcttaacaaaatgtggcagtcaaatacttgctacagtttcagttttggctgttaaaggcagtttggctccaatatctggaacagttcaaagtgctcatcttattataagatttgacgaaaatggagtgctactaaacaattccttcctggacccagaatattggaactttagaaatggagatcttactgaaggcacagcctatacaaacgctgttggatttatgcctaacctatcagcttatccaaaatctcacggtaaaactgccaaaagtaacattgtcagtcaagtttacttaaacggagacaaaactaaacctgtaacactaaccattacactaaacggtacacaggaaacaggagacacaactccaagtgcatactctatgtcattttcatgggactggtctggccacaactacattaatgaaatatttgccacatcctcttacactttttcatacattgcccaagaataaagaatcgtttgtgttatgtttcaacgtgtttatttttcaattgcagaaaatttcaagtcatttttcattcagtagtatagccccaccaccacatagcttatacagatcaccgtaccttaatcaaactcacagaaccctagtattcaacctgccacctccctcccaacacacagagtacacagtcctttctccccggctggccttaaaaagcatcatatcatgggtaacagacatattcttaggtgttatattccacacggtttcctgtcgagccaaacgctcatcagtgatattaataaactccccgggcagctcacttaagttcatgtcgctgtccagctgctgagccacaggctgctgtccaacttgcggttgcttaacgggcggcgaaggagaagtccacgcctacatgggggtagagtcataatcgtgcatcaggatagggcggtggtgctgcagcagcgcgcgaataaactgctgccgccgccgctccgtcctgcaggaatacaacatggcagtggtctcctcagcgatgattcgcaccgcccgcagcataaggcgccttgtcctccgggcacagcagcgcaccctgatctcacttaaatcagcacagtaactgcagcacagcaccacaatattgttcaaaatcccacagtgcaaggcgctgtatccaaagctcatggcggggaccacagaacccacgtggccatcataccacaagcgcaggtagattaagtggcgacccctcataaacacgctggacataaacattacctcttttggcatgttgtaattcaccacctcccggtaccatataaacctctgattaaacatggcgccatccaccaccatcctaaaccagctggccaaaacctgcccgccggctatacactgcagggaaccgggactggaacaatgacagtggagagcccaggactcgtaaccatggatcatcatgctcgtcatgatatcaatgttggcacaacacaggcacacgtgcatacacttcctcaggattacaagctcctcccgcgttagaaccatatcccagggaacaacccattcctgaatcagcgtaaatcccacactgcagggaagacctcgcacgtaactcacgttgtgcattgtcaaagtgttacattcgggcagcagcggatgatcctccagtatggtagcgcgggtttctgtctcaaaaggaggtagacgatccctactgtacggagtgcgccgagacaaccgagatcgtgttggtcgtagtgtcatgccaaatggaacgccggacgtagtcatatttcctgaagcaaaaccaggtgcgggcgtgacaaacagatctgcgtctccggtctcgccgcttagatcgctctgtgtagtagttgtagtatatccactctctcaaagcatccaggcgccccctggcttcgggttctatgtaaactccttcatgcgccgctgccctgataacatccaccaccgcagaataagccacacccagccaacctacacattcgttctgcgagtcacacacgggaggagcgggaagagctggaagaaccatgtttttttttttattccaaaagattatccaaaacctcaaaatgaagatctattaagtgaacgcgctcccctccggtggcgtggtcaaactctacagccaaagaacagataatggcatttgtaagatgttgcacaatggcttccaaaaggcaaacggccctcacgtccaagtggacgtaaaggctaaacccttcagggtgaatctcctctataaacattccagcaccttcaaccatgcccaaataattctcatctcgccaccttctcaatatatctctaagcaaatcccgaatattaagtccggccattgtaaaaatctgctccagagcgccctccaccttcagcctcaagcagcgaatcatgattgcaaaaattcaggttcctcacagacctgtataagattcaaaagcggaacattaacaaaaataccgcgatcccgtaggtcccttcgcagggccagctgaacataatcgtgcaggtctgcacggaccagcgcggccacttccccgccaggaaccatgacaaaagaacccacactgattatgacacgcatactcggagctatgctaaccagcgtagccccgatgtaagcttgttgcatgggcggcgatataaaatgcaaggtgctgctcaaaaaatcaggcaaagcctcgcgcaaaaaagaaagcacatcgtagtcatgctcatgcagataaaggcaggtaagctccggaaccaccacagaaaaagacaccatttttctctcaaacatgtctgcgggtttctgcataaacacaaaataaaataacaaaaaaacatttaaacattagaagcctgtcttacaacaggaaaaacaacccttataagcataagacggactacggccatgccggcgtgaccgtaaaaaaactggtcaccgtgattaaaaagcaccaccgacagctcctcggtcatgtccggagtcataatgtaagactcggtaaacacatcaggttgattcacatcggtcagtgctaaaaagcgaccgaaatagcccgggggaatacatacccgcaggcgtagagacaacattacagcccccataggaggtataacaaaattaataggagagaaaaacacataaacacctgaaaaaccctcctgcctaggcaaaatagcaccctcccgctccagaacaacatacagcgcttccacagcggcagccataacagtcagccttaccagtaaaaaagaaaacctattaaaaaaacaccactcgacacggcaccagctcaatcagtcacagtgtaaaaaagggccaagtgcagagcgagtatatataggactaaaaaatgacgtaacggttaaagtccacaaaaaacacccagaaaaccgcacgcgaacctacgcccagaaacgaaagccaaaaaacccacaacttcctcaaatcgtcacttccgttttcccacgttacgtcacttcccattttaagaaaactacaattcccaacacatactagttactccgccctaaaacctacgtcacccgccccgttcccacgccccgcgccacgtcacaaactccaccccctcattatcatattggcttcaatccaaaataaggtatattattgatgatgt

SEQ ID NO: 6 - DNA, 102 bp, Artificial Sequence
  gp100-tyr insertion with linkers
ggaagcggttctcgctacctggagcctggcccagtgactgccgctggttccggaagcagatacatggacggaacaatgtcccaggttgccggttctggctcc

SEQ ID NO: 7 - protein, 34 aa, Artificial Sequence
  gp100-tyr insertion with linkers
GSGSRYLEPGPVTAAGSGSRYMDGTMSQVAGSGS

SEQ ID NO: 8 - DNA, 2859 bp, Artificial Sequence
  wt Hexon
atggctaccccttcgatgatgccgcagtggtcttacatgcacatctcgggccaggacgcctcggagtacctgagccccgggctggtgcagtttgcccgcgccaccgagacgtacttcagcctgaataacaagtttagaaaccccacggtggcgcctacgcacgacgtgaccacagaccggtcccagcgtttgacgctgcggttcatccctgtggaccgtgaggatactgcgtactcgtacaaggcgcggttcaccctagctgtgggtgataaccgtgtgctggacatggcttccacgtactttgacatccgcggcgtgctggacaggggccctacttttaagccctactctggcactgcctacaacgccctggctcccaagggtgccccaaatccttgcgaatgggatgaagctgctactgctcttgaaataaacctagaagaagaggacgatgacaacgaagacgaagtagacgagcaagctgagcagcaaaaaactcacgtatttgggcaggcgccttattctggtataaatattacaaaggagggtattcaaataggtgtcgaaggtcaaacacctaaatatgccgataaaacatttcaacctgaacctcaaataggagaatctcagtggtacgaaactgaaattaatcatgcagctgggagagtccttaaaaagactaccccaatgaaaccatgttacggttcatatgcaaaacccacaaatgaaaatggagggcaaggcattcttgtaaagcaacaaaatggaaagctagaaagtcaagtggaaatgcaatttttctcaactactgaggcgaccgcaggcaatggtgataacttgactcctaaagtggtattgtacagtgaagatgtagatatagaaaccccagacactcatatttcttacatgcccactattaaggaaggtaactcacgagaactaatgggccaacaatctatgcccaacaggcctaattacattgcttttagggacaattttattggtctaatgtattacaacagcacgggtaatatgggtgttctggcgggccaagcatcgcagttgaatgctgttgtagatttgcaagacagaaacacagagctttcataccagcttttgcttgattccattggtgatagaaccaggtacttttctatgtggaatcaggctgttgacagctatgatccagatgttagaattattgaaaatcatggaactgaagatgaacttccaaattactgctttccactgggaggtgtgattaatacagagactcttaccaaggtaaaacctaaaacaggtcaggaaaatggatgggaaaaagatgctacagaattttcagataaaaatgaaataagagttggaaataattttgccatggaaatcaatctaaatgccaacctgtggagaaatttcctgtactccaacatagcgctgtatttgcccgacaagctaaagtacagtccttccaacgtaaaaatttctgataacccaaacacctacgactacatgaacaagcgagtggtggctcccgggttagtggactgctacattaaccttggagcacgctggtcccttgactatatggacaacgtcaacccatttaaccaccaccgcaatgctggcctgcgctaccgctcaatgttgctgggcaatggtcgctatgtgcccttccacatccaggtgcctcagaagttctttgccattaaaaacctccttctcctgccgggctcatacacctacgagtggaacttcaggaaggatgttaacatggttctgcagagctccctaggaaatgacctaagggttgacggagccagcattaagtttgatagcatttgcctttacgccaccttcttccccatggcccacaacaccgcctccacgcttgaggccatgcttagaaacgacaccaacgaccagtcctttaacgactatctctccgccgccaacatgctctaccctatacccgccaacgctaccaacgtgcccatatccatcccctcccgcaactgggcggctttccgcggctgggccttcacgcgccttaagactaaggaaaccccatcactgggctcgggctacgacccttattacacctactctggctctataccctacctagatggaaccttttacctcaaccacacctttaagaaggtggccattacctttgactcttctgtcagctggcctggcaatgaccgcctgcttacccccaacgagtttgaaattaagcgctcagttgacggggagggttacaacgttgcccagtgtaacatgaccaaagactggttcctggtacaaatgctagctaactacaacattggctaccagggcttctatatcccagagagctacaaggaccgcatgtactccttctttagaaacttccagcccatgagccgtcaggtggtggatgatactaaatacaaggactaccaacaggtgggcatcctacaccaacacaacaactctggatttgttggctaccttgcccccaccatgcgcgaaggacaggcctaccctgctaacttcccctatccgcttataggcaagaccgcagttgacagcattacccagaaaaagtttctttgcgatcgcaccctttggcgcatcccattctccagtaactttatgtccatgggcgcactcacagacctgggccaaaaccttctctacgccaactccgcccacgcgctagacatgacttttgaggtggatcccatggacgagcccacccttctttatgttttgtttgaagtctttgacgtggtccgtgtgcaccagccgcaccgcggcgtcatcgaaaccgtgtacctgcgcacgcccttctcggccggcaacgccacaacataa

SEQ ID NO: 9 - protein, 952 aa, Artificial Sequence
  wt Hexon
MATPSMMPQWSYMHISGQDASEYLSPGLVQFARATETYFSLNNKFRNPTVAPTHDVTTDRSQRLTLRFIPVDREDTAYSYKARFTLAVGDNRVLDMASTYFDIRGVLDRGPTFKPYSGTAYNALAPKGAPNPCEWDEAATALEINLEEEDDDNEDEVDEQAEQQKTHVFGQAPYSGINITKEGIQIGVEGQTPKYADKTFQPEPQIGESQWYETEINHAAGRVLKKTTPMKPCYGSYAKPTNENGGQGILVKQQNGKLESQVEMQFFSTTEATAGNGDNLTPKVVLYSEDVDIETPDTHISYMPTIKEGNSRELMGQQSMPNRPNYIAFRDNFIGLMYYNSTGNMGVLAGQASQLNAVVDLQDRNTELSYQLLLDSIGDRTRYFSMWNQAVDSYDPDVRIIENHGTEDELPNYCFPLGGVINTETLTKVKPKTGQENGWEKDATEFSDKNEIRVGNNFAMEINLNANLWRNFLYSNIALYLPDKLKYSPSNVKISDNPNTYDYMNKRVVAPGLVDCYINLGARWSLDYMDNVNPFNHHRNAGLRYRSMLLGNGRYVPFHIQVPQKFFAIKNLLLLPGSYTYEWNFRKDVNMVLQSSLGNDLRVDGASIKFDSICLYATFFPMAHNTASTLEAMLRNDTNDQSFNDYLSAANMLYPIPANATNVPISIPSRNWAAFRGWAFTRLKTKETPSLGSGYDPYYTYSGSIPYLDGTFYLNHTFKKVAITFDSSVSWPGNDRLLTPNEFEIKRSVDGEGYNVAQCNMTKDWFLVQMLANYNIGYQGFYIPESYKDRMYSFFRNFQPMSRQVVDDTKYKDYQQVGILHQHNNSGFVGYLAPTMREGQAYPANFPYPLIGKTAVDSITQKKFLCDRTLWRIPFSSNFMSMGALTDLGQNLLYANSAHALDMTFEVDPMDEPTLLYVLFEVFDVVRVHQPHRGVIETVYLRTPFSAGNATT

SEQ ID NO: 10 - DNA, 27 bp, Artificial Sequence
  Hex713 epitope
tacctcaaccacacctttaagaaggtg

SEQ ID NO: 11 - protein, 9 aa, Artificial Sequence
  Hex713 epitope
YLNHTFKKV

SEQ ID NO: 12 - DNA, 27 bp, Artificial Sequence
  V721A epitope
tacctcaaccacacctttaagaaggct

SEQ ID NO: 13 - protein, 9 aa, Artificial Sequence
  V721A epitope
YLNHTFKKA

SEQ ID NO: 14 - DNA, 27 bp, Artificial Sequence
  Hex892 epitope
cttctctacgccaactccgcccacgcg

SEQ ID NO: 15 - protein, 9 aa, Artificial Sequence
  Hex892 epitope
LLYANSAHA

SEQ ID NO: 16 - DNA, 27 bp, Artificial Sequence
  A900S epitope
cttctctacgccaactccgcccactcc

SEQ ID NO: 17 - protein, 9 aa, Artificial Sequence
  A900S epitope
LLYANSAHS

SEQ ID NO: 18 - DNA, 27 bp, Artificial Sequence
  Hex917 epitope
tatgttttgtttgaagtctttgacgtg

SEQ ID NO: 19 - protein, 9 aa, Artificial Sequence
  Hex917 epitope
YVLFEVFDV

SEQ ID NO: 20 - DNA, 27 bp, Artificial Sequence
  V925K epitope
tatgttttgtttgaagtctttgacaag

SEQ ID NO: 21 - protein, 9 aa, Artificial Sequence
  V925K epitope
YVLFEVFDK

SEQ ID NO: 22 - DNA, 27 bp, Artificial Sequence
  Hex512 epitope
gggttagtggactgctacattaacctt

SEQ ID NO: 23 - protein, 9 aa, Artificial Sequence
  Hex512 epitope
GLVDCYINL

SEQ ID NO: 24 - DNA, 27 bp, Artificial Sequence
  L520P epitope
gggttagtggactgctacattaacccc

SEQ ID NO: 25 - protein, 9 aa, Artificial Sequence
  L520P epitope
GLVDCYINP

SEQ ID NO: 26 - protein, 4 aa, Artificial Sequence
  heparin sulphate glycosaminoglycan (HSG)-binding site
KKTK

SEQ ID NO: 27 - protein, 4 aa, Artificial Sequence
  integrin-binding motif
RGDK

SEQ ID NO: 28 - protein, 5 aa, Artificial Sequence
  flexible linker
GSGSR

SEQ ID NO: 29 - protein, 6 aa, Artificial Sequence
  flexible linker
AGSGSR

SEQ ID NO: 30 - protein, 5 aa, Artificial Sequence
  flexible linker
AGSGS

SEQ ID NO: 31 - protein, 9 aa, Artificial Sequence
  gp100-280
YLEPGPVTA

SEQ ID NO: 32 - protein, 9 aa, Artificial Sequence
  Tyr369(3D)
YMDGTMSQV

SEQ ID NO: 33 - protein, 9 aa, Artificial Sequence
  E1A19
LLDQLIEEV

SEQ ID NO: 34 - protein, 9 aa, Artificial Sequence
  Hex63
RLTLRFIPV

SEQ ID NO: 35 - protein, 9 aa, Artificial Sequence
  Hex548
MLLGNGRYV

SEQ ID NO: 36 - protein, 9 aa, Artificial Sequence
  Hex652
MLYPIPANA

SEQ ID NO: 37 - protein, 9 aa, Artificial Sequence
  Hex914
TLLYVLFEV

SEQ ID NO: 38 - protein, 9 aa, Artificial Sequence
  gp100-209
IMDQVPFSV